European Patent Specification EP 3 984 537 B1, published March 20, 2024. Title: CANCER TREATMENTS USING COMBINATIONS OF TYPE 2 MEK AND ERK INHIBITORS. Applicant: BIOMED VALLEY DISCOVERIES, INC. The sequence listing filed with the application follows.

SEQUENCE LISTING (128 sequences)

SEQ ID NO: 1 - DNA, 1061 bp, Homo sapiens
tgccctgcgcccgcaacccgagccgcacccgccgcggacggagcccatgcgcggggcgaaccgcgcgcccccgcccccgccccgccccggcctcggccccggccctggccccgggggcagtcgcgcctgtgaacggtggggcaggagaccctgtaggaggaccccgggccgcaggcccctgaggagcgatgacggaatataagctggtggtggtgggcgccggcggtgtgggcaagagtgcgctgaccatccagctgatccagaaccattttgtggacgaatacgaccccactatagaggattcctaccggaagcaggtggtcattgatggggagacgtgcctgttggacatcctggataccgccggccaggaggagtacagcgccatgcgggaccagtacatgcgcaccggggagggcttcctgtgtgtgtttgccatcaacaacaccaagtcttttgaggacatccaccagtacagggagcagatcaaacgggtgaaggactcggatgacgtgcccatggtgctggtggggaacaagtgtgacctggctgcacgcactgtggaatctcggcaggctcaggacctcgcccgaagctacggcatcccctacatcgagacctcggccaagacccggcagggagtggaggatgccttctacacgttggtgcgtgagatccggcagcacaagctgcggaagctgaaccctcctgatgagagtggccccggctgcatgagctgcaagtgtgtgctctcctgacgcagcacaagctcaggacatggaggtgccggatgcaggaaggaggtgcagacggaaggaggaggaaggaaggacggaagcaaggaaggaaggaagggctgctggagcccagtcaccccgggaccgtgggccgaggtgactgcagaccctcccagggaggctgtgcacagactgtcttgaacatcccaaatgccaccggaaccccagcccttagctcccctcccaggcctctgtgggcccttgtcgggcacagatgggatcacagtaaattattggatggtcttgaaaaaaaaaaaaaaaaaa

SEQ ID NO: 2 - protein, 189 aa, Homo sapiens
MTEYKLVVVGAGGVGKSALTIQLIQNHFVDEYDPTIEDSYRKQVVIDGETCLLDILDTAGQEEYSAMRDQYMRTGEGFLCVFAINNTKSFEDIHQYREQIKRVKDSDDVPMVLVGNKCDLAARTVESRQAQDLARSYGIPYIETSAKTRQGVEDAFYTLVREIRQHKLRKLNPPDESGPGCMSCKCVLS

SEQ ID NO: 3 - DNA, 1251 bp, Homo sapiens
tgccctgcgcccgcaacccgagccgcacccgccgcggacggagcccatgcgcggggcgaaccgcgcgcccccgcccccgccccgccccggcctcggccccggccctggccccgggggcagtcgcgcctgtgaacggtggggcaggagaccctgtaggaggaccccgggccgcaggcccctgaggagcgatgacggaatataagctggtggtggtgggcgccggcggtgtgggcaagagtgcgctgaccatccagctgatccagaaccattttgtggacgaatacgaccccactatagaggattcctaccggaagcaggtggtcattgatggggagacgtgcctgttggacatcctggataccgccggccaggaggagtacagcgccatgcgggaccagtacatgcgcaccggggagggcttcctgtgtgtgtttgccatcaacaacaccaagtcttttgaggacatccaccagtacagggagcagatcaaacgggtgaaggactcggatgacgtgcccatggtgctggtggggaacaagtgtgacctggctgcacgcactgtggaatctcggcaggctcaggacctcgcccgaagctacggcatcccctacatcgagacctcggccaagacccggcagggcagccgctctggctctagctccagctccgggaccctctgggaccccccgggacccatgtgacccagcggcccctcgcgctggagtggaggatgccttctacacgttggtgcgtgagatccggcagcacaagctgcggaagctgaaccctcctgatgagagtggccccggctgcatgagctgcaagtgtgtgctctcctgacgcaggtgagggggactcccagggcggccgccacgcccaccggatgaccccggctccccgcccctgccggtctcctggcctgcggtcagcagcctcccttgtgccccgcccagcacaagctcaggacatggaggtgccggatgcaggaaggaggtgcagacggaaggaggaggaaggaaggacggaagcaaggaaggaaggaagggctgctggagcccagtcaccccgggaccgtgggccgaggtgactgcagaccctcccagggaggctgtgcacagactgtcttgaacatcccaaatgccaccggaaccccagcccttagctcccctcccaggcctctgtgggcccttgtcgggcacagatgggatcacagtaaattattggatggtcttgaaaaaaaaaaaaaaaaaa

SEQ ID NO: 4 - protein, 170 aa, Homo sapiens
MTEYKLVVVGAGGVGKSALTIQLIQNHFVDEYDPTIEDSYRKQVVIDGETCLLDILDTAGQEEYSAMRDQYMRTGEGFLCVFAINNTKSFEDIHQYREQIKRVKDSDDVPMVLVGNKCDLAARTVESRQAQDLARSYGIPYIETSAKTRQGSRSGSSSSSGTLWDPPGPM

SEQ ID NO: 5 - DNA, 1169 bp, Homo sapiens
tgccctgcgcccgcaacccgagccgcacccgccgcggacggagcccatgcgcggggcgaaccgcgcgcccccgcccccgccccgccccggcctcggccccggccctggccccgggggcagtcgcgcctgtgaacggtggggcaggagaccctgtaggaggaccccgggccgcaggcccctgaggagcgatgacggaatataagctggtggtggtgggcgccggcggtgtgggcaagagtgcgctgaccatccagctgatccagaaccattttgtggacgaatacgaccccactatagaggattcctaccggaagcaggtggtcattgatggggagacgtgcctgttggacatcctggataccgccggccaggaggagtacagcgccatgcgggaccagtacatgcgcaccggggagggcttcctgtgtgtgtttgccatcaacaacaccaagtcttttgaggacatccaccagtacagggagcagatcaaacgggtgaaggactcggatgacgtgcccatggtgctggtggggaacaagtgtgacctggctgcacgcactgtggaatctcggcaggctcaggacctcgcccgaagctacggcatcccctacatcgagacctcggccaagacccggcagggagtggaggatgccttctacacgttggtgcgtgagatccggcagcacaagctgcggaagctgaaccctcctgatgagagtggccccggctgcatgagctgcaagtgtgtgctctcctgacgcaggtgagggggactcccagggcggccgccacgcccaccggatgaccccggctccccgcccctgccggtctcctggcctgcggtcagcagcctcccttgtgccccgcccagcacaagctcaggacatggaggtgccggatgcaggaaggaggtgcagacggaaggaggaggaaggaaggacggaagcaaggaaggaaggaagggctgctggagcccagtcaccccgggaccgtgggccgaggtgactgcagaccctcccagggaggctgtgcacagactgtcttgaacatcccaaatgccaccggaaccccagcccttagctcccctcccaggcctctgtgggcccttgtcgggcacagatgggatcacagtaaattattggatggtcttgaaaaaaaaaaaaaaaaaa

SEQ ID NO: 6 - protein, 189 aa, Homo sapiens; identical to SEQ ID NO: 2

SEQ ID NO: 7 - DNA, 1246 bp, Rattus norvegicus
gcccggcgcccgcagcccgagccgcacccgccgcggacggagcccatgcgcgggcccagtcggcgcccgtccgcgcccccgccctgccccggccccggccccgggggcagtcgcgccagcaagcggtggggcaggagctcctggtttggcagcccctgtagaagcgatgacagaatacaagcttgtggtggtgggcgctggaggcgtgggaaagagtgccctgaccatccagctgatccagaaccattttgtggacgagtatgatcccactatagaggactcctaccggaaacaggtagtcattgatggggagacgtgtttactggacatcttagacacagcaggtcaagaagagtatagtgccatgcgggaccagtacatgcgcacaggggagggcttcctctgtgtatttgccatcaacaacaccaagtcctttgaagacatccatcagtacagggagcagatcaagcgggtgaaagattcagatgatgtgccaatggtgctggtgggcaacaagtgtgacctggccgctcgcactgttgagtctcggcaggcccaggaccttgctcgcagctatggcatcccctacattgaaacatcagccaagacccggcagggtgtggaggatgccttctacacactagtacgtgagattcggcagcataaactgcggaaactgaacccgcctgatgagagtggccctggctgcatgagctgcaagtgtgtgctgtcctgacaccaggctcaggacgaggaggtgccggatgcagggaggaggtgctgtcggaaggaaggaaagaggagggaaggaaggaaacgatgctggagccagtccagtccagggatggtggacagatgtgaccaagaccttcgcatggacaatttgaacagactgtcatgaactatccctgttgccactggcacccaagtcctccgcccctctcagctcccttgggcgcctatgagggcacatgttgaatcacagtaaattatttgatggtcttgacttgtctctggctggaagtaggaggtgtagtgcctgtggcctcacagaagatactggggacctgggatctatcatctgccttgttcctgtttctagaagaggctggggaggctggcctgggacctgggactgtgcagcccttctcttctgcctgcctcaactgtcttgtgtttcctgcagaaagttataaataacacaagaatagtcaggtgatatgaaaaaaaaaaaaaaaaaaaaaaa

SEQ ID NO: 8 - protein, 189 aa, Rattus norvegicus; identical to SEQ ID NO: 2

SEQ ID NO: 9 - DNA, 1392 bp, Rattus norvegicus
gcccggcgcccgcagcccgagccgcacccgccgcggacggagcccatgcgcgggcccagtcggcgcccgtccgcgcccccgccctgccccggccccggccccgggggcagtcgcgccagcaagcggtggggcaggagctcctggtttggcagcccctgtagaagcgatgacagaatacaagcttgtggtggtgggcgctggaggcgtgggaaagagtgccctgaccatccagctgatccagaaccattttgtggacgagtatgatcccactatagaggactcctaccggaaacaggtagtcattgatggggagacgtgtttactggacatcttagacacagcaggtcaagaagagtatagtgccatgcgggaccagtacatgcgcacaggggagggcttcctctgtgtatttgccatcaacaacaccaagtcctttgaagacatccatcagtacagggagcagatcaagcgggtgaaagattcagatgatgtgccaatggtgctggtgggcaacaagtgtgacctggccgctcgcactgttgagtctcggcaggcccaggaccttgctcgcagctatggcatcccctacattgaaacatcagccaagacccggcagggtgtggaggatgccttctacacactagtacgtgagattcggcagcataaactgcggaaactgaacccgcctgatgagagtggccctggctgcatgagctgcaagtgtgtgctgtcctgacaccaggtgaggcagggaccagcaagacatctggggcagtgacctcagctagccagatgaacttcatatccactttgatgtccctgctcccccaattctgccaatccccctgcctgcagtcagtcatgtcctttgtgcccgtcccggcacaggctcaggacgaggaggtgccggatgcagggaggaggtgctgtcggaaggaaggaaagaggagggaaggaaggaaacgatgctggagccagtccagtccagggatggtggacagatgtgaccaagaccttcgcatggacaatttgaacagactgtcatgaactatccctgttgccactggcacccaagtcctccgcccctctcagctcccttgggcgcctatgagggcacatgttgaatcacagtaaattatttgatggtcttgacttgtctctggctggaagtaggaggtgtagtgcctgtggcctcacagaagatactggggacctgggatctatcatctgccttgttcctgtttctagaagaggctggggaggctggcctgggacctgggactgtgcagcccttctcttctgcctgcctcaactgtcttgtgtttcctgcagaaagttataaataacacaagaatagtcaggtgatatgaaaaaaaaaaaaaaaaaaaaaaa

SEQ ID NO: 10 - protein, 189 aa, Rattus norvegicus; identical to SEQ ID NO: 2

SEQ ID NO: 11 - DNA, 504 bp, Mus musculus
atggcggtaaatgattgcttcagtctgacctatcctcacaacccacacccaggagacttgattgaagtgttccgtccttgctatcagcactgggcactgtacttgggtgatggctacgtgatcaacattgcacctatagatggcattcgctcatcatttacaagtgctaagtccgtgttcagcacaaaggccttggtgaaaatgcagcttttgaaggatgttgtgggaaatgacacatacagaataaataacaagtacgacacaacataccctcctcttcctgtggaggaggtgatacaacggtcagagttccctattgggcaggaagtagcctatgacttgctggtcaacaactgtgagcattttgtaaccttgctgcgctatggagaaggagtgtcagagcaggccaaccgagcaatcggcaccatcggattggtggcagctggtattgatatcttcacattcctcggcttgtttcccaaaagacaaagaacgaaatattag

SEQ ID NO: 12 - protein, 167 aa, Mus musculus
MAVNDCFSLTYPHNPHPGDLIEVFRPCYQHWALYLGDGYVINIAPIDGIRSSFTSAKSVFSTKALVKMQLLKDVVGNDTYRINNKYDTTYPPLPVEEVIQRSEFPIGQEVAYDLLVNNCEHFVTLLRYGEGVSEQANRAIGTIGLVAAGIDIFTFLGLFPKRQRTKY

SEQ ID NO: 13 - DNA, 1455 bp, Cavia porcellus
cgggctctgcggcggggcagctgcgccctgcgcgcgtgccgcgcttcccggggccccagctgtggccgggcgctcagcgaggcgccgcccgggctcggggacgcgggcccgcggccatgtcgctcggtgcgggacgccgcgcgtctctgtccagctccgcttccctgtcgcccgcgctccccggccgcccgcgctcccccgctgtcccctgcgccctggacccctagccgctgctccgtggaccgcttgggacgtgtcggccggggccgcgtctccccgccgcccttcccccgcgccgcgtgcagccggcgcctgtggacgcacacgggcctgcgccgctgtaggcgcggctgtcgggacgctgcctgcctcgacacgcccgccggcgggcaaggacctgttcgggcggccccgccagcaggtggggcaagagcccccgagtgccctgagcgtcagtccctggaggagccatgacggagtacaagcttgtggtggtgggtgcaggaggtgtggggaagagcgccctgactatccagctgatccagaaccattttgtggacgaatatgaccccaccatagaggattcataccggaagcaggtggtcattgatggggagacctgtctgctggatatcttggacacagctggccaagaggagtatagtgccatgcgggaccaatacatgcgcactggggagggcttcctttgtgtgttcgccatcaacaataccaaatctttcgaggacatccatcagtacagggagcagatcaagcgggtgaaggactcagatgatgtgcccatggtgctggtgggaaacaaatgtgacctggctacacgcaccgtggagtctcggcaggcccaagaccttgcccgcagttacggcattccctacattgagacatcagccaagacccgccagggagtagaagacgccttctatacactagttcgagagatccggcagcacaaactgcggaagctgaatccaccagatgagagtgggccagggtgcatgagctgcaaatgtgtgctatcctgatccaggtgagcagggcccagctggctccccgagccacagccctagccggccagccagctaagctgcacatctactctgatgttcctgggcttcctgaacctgctggtccccttgtctacgatcagtggcgtccttcatgctccatcctggcccaggctcaggacacagaggtaccagatgtggggaagaggtacagaaggaaggaaggaaggaaggaaggaagtgccactggagtccagccagcccagggatggtggatagaggcgactgcagaccctcctgtggatgctttgcaagctgtcatgaactgtcccaaacaccactggcctcccagccctaactcccctcccagtttttccagcctctgacaggtgcaggttgatttgcagtaaattatttgatggtcttgactcca

SEQ ID NO: 14 - protein, 189 aa, Cavia porcellus
MTEYKLVVVGAGGVGKSALTIQLIQNHFVDEYDPTIEDSYRKQVVIDGETCLLDILDTAGQEEYSAMRDQYMRTGEGFLCVFAINNTKSFEDIHQYREQIKRVKDSDDVPMVLVGNKCDLATRTVESRQAQDLARSYGIPYIETSAKTRQGVEDAFYTLVREIRQHKLRKLNPPDESGPGCMSCKCVLS

SEQ ID NO: 15 - DNA, 1694 bp, Cavia porcellus
cgggctctgcggcggggcagctgcgccctgcgcgcgtgccgcgcttcccggggccccagctgtggccgggcgctcagcgaggcgccgcccgggctcggggacgcgggcccgcggccatgtcgctcggtgcgggacgccgcgcgtctctgtccagctccgcttccctgtcgcccgcgctccccggccgcccgcgctcccccgctgtcccctgcgccctggacccctagccgctgctccgtggaccgcttgggacgtgtcggccggggccgcgtctccccgccgcccttcccccgcgccgcgtgcagccggcgcctgtggacgcacacgggcctgcgccgctgtaggcgcggctgtcgggacgctgcctgcctcgacacgcccgccggcgggcaaggacctgttcgggcggccccgccagcaggtgcctatgacctaggctttttgcctacccagcaacttctaatttgggtgcctggttgggagcggctcagctgtcaccctgcctcggcgccggcccctgcttccttacaggccacgaggtgcagcggggtgcggtgagaccctcagcccgctggaggtgccacaggtgccgccatcctggctggcgcccttccagccactccgctgggtggcgcttggctgagctggtcctcctcacaggtggggcaagagcccccgagtgccctgagcgtcagtccctggaggagccatgacggagtacaagcttgtggtggtgggtgcaggaggtgtggggaagagcgccctgactatccagctgatccagaaccattttgtggacgaatatgaccccaccatagaggattcataccggaagcaggtggtcattgatggggagacctgtctgctggatatcttggacacagctggccaagaggagtatagtgccatgcgggaccaatacatgcgcactggggagggcttcctttgtgtgttcgccatcaacaataccaaatctttcgaggacatccatcagtacagggagcagatcaagcgggtgaaggactcagatgatgtgcccatggtgctggtgggaaacaaatgtgacctggctacacgcaccgtggagtctcggcaggcccaagaccttgcccgcagttacggcattccctacattgagacatcagccaagacccgccagggagtagaagacgccttctatacactagttcgagagatccggcagcacaaactgcggaagctgaatccaccagatgagagtgggccagggtgcatgagctgcaaatgtgtgctatcctgatccaggtgagcagggcccagctggctccccgagccacagccctagccggccagccagctaagctgcacatctactctgatgttcctgggcttcctgaacctgctggtccccttgtctacgatcagtggcgtccttcatgctccatcctggcccaggctcaggacacagaggtaccagatgtggggaagaggtacagaaggaaggaaggaaggaaggaaggaagtgccactggagtccagccagcccagggatggtggatagaggcgactgcagaccctcctgtggatgctttgcaagctgtcatgaactgtcccaaacaccactggcctcccagccctaactcccctcccagtttttccagcctctgacaggtgcaggttgatttgcagtaaattatttgatggtcttgactcca

SEQ ID NO: 16 - protein, 189 aa, Cavia porcellus; identical to SEQ ID NO: 14

SEQ ID NO: 17 - DNA, 1180 bp, Cavia porcellus
actgggcctacagtccccaccgcccgcgccgcgagcccgcagcccgagccgcacccgctgcggacggagcccatgcgcgggcccagccagcgcccgcccgcgcccccgccccgccccggccccgggggcagttgcaccagcgagtggtggggcaagagcccccgagtgccctgagcgtcagtccctggaggagccatgacggagtacaagcttgtggtggtgggtgcaggaggtgtggggaagagcgccctgactatccagctgatccagaaccattttgtggacgaatatgaccccaccatagaggattcataccggaagcaggtggtcattgatggggagacctgtctgctggatatcttggacacagctggccaagaggagtatagtgccatgcgggaccaatacatgcgcactggggagggcttcctttgtgtgttcgccatcaacaataccaaatctttcgaggacatccatcagtacagggagcagatcaagcgggtgaaggactcagatgatgtgcccatggtgctggtgggaaacaaatgtgacctggctacacgcaccgtggagtctcggcaggcccaagaccttgcccgcagttacggcattccctacattgagacatcagccaagacccgccagggagtagaagacgccttctatacactagttcgagagatccggcagcacaaactgcggaagctgaatccaccagatgagagtgggccagggtgcatgagctgcaaatgtgtgctatcctgatccaggtgagcagggcccagctggctccccgagccacagccctagccggccagccagctaagctgcacatctactctgatgttcctgggcttcctgaacctgctggtccccttgtctacgatcagtggcgtccttcatgctccatcctggcccaggctcaggacacagaggtaccagatgtggggaagaggtacagaaggaaggaaggaaggaaggaaggaagtgccactggagtccagccagcccagggatggtggatagaggcgactgcagaccctcctgtggatgctttgcaagctgtcatgaactgtcccaaacaccactggcctcccagccctaactcccctcccagtttttccagcctctgacaggtgcaggttgatttgcagtaaattatttgatggtcttgactcca

SEQ ID NO: 18 - protein, 189 aa, Cavia porcellus; identical to SEQ ID NO: 14

SEQ ID NO: 19 - DNA, 1270 bp, Cavia porcellus
cgggctctgcggcggggcagctgcgccctgcgcgcgtgccgcgcttcccggggccccagctgtggccgggcgctcagcgaggcgccgcccgggctcggggacgcgggcccgcggccatgtcgctcggtgcgggacgccgcgcgtctctgtccagctccgcttccctgtcgcccgcgctccccggccgcccgcgctcccccgctgtcccctgcgccctggacccctagccgctgctccgtggaccgcttgggacgtgtcggccggggccgcgtctccccgccgcccttcccccgcgccgcgtgcagccggcgcctgtggacgcacacgggcctgcgccgctgtaggcgcggctgtcgggacgctgcctgcctcgacacgcccgccggcgggcaaggacctgttcgggcggccccgccagcaggtgcctatgacctaggctttttgcctacccagcaacttctaatttgggtgcctggttgggagcggctcagctgtcaccctgcctcggcgccggcccctgcttccttacaggccacgaggtgcagcggggtgcggtgagaccctcagcccgctggaggtgccacaggtgccgccatcctggctggcgcccttccagccactccgctgggtggcgcttggctgagctggtcctcctcacaggtggggcaagagcccccgagtgccctgagcgtcagtccctggaggagccatgacggagtacaagcttgtggtggtgggtgcaggaggtgtggggaagagcgccctgactatccagctgatccagaaccattttgtggacgaatatgaccccaccatagaggattcataccggaagcaggtggtcattgatggggagacctgtctgctggatatcttggacacagctggccaagaggagtatagtgccatgcgggaccaatacatgcgcactggggagggcttcctttgtgtgttcgccatcaacaataccaaatctttcgaggacatccatcagtacagggagcagatcaagcgggtgaaggactcagatgatgtgcccatggtgctggtgggaaacaaatgtgacctggctacacgcaccgtggagtctcggcaggcccaagaccttgcccgcagttacggcattccctacattgagacatcagccaagacccgccagggcagccgctctggctctggcttcagctccgggacccactgggaacccctgggatccatgtgacccatcggcccccatgctggagtagaagacgccttctatacactagtt

SEQ ID NO: 20 - protein, 170 aa, Cavia porcellus
MTEYKLVVVGAGGVGKSALTIQLIQNHFVDEYDPTIEDSYRKQVVIDGETCLLDILDTAGQEEYSAMRDQYMRTGEGFLCVFAINNTKSFEDIHQYREQIKRVKDSDDVPMVLVGNKCDLATRTVESRQAQDLARSYGIPYIETSAKTRQGSRSGSGFSSGTHWEPLGSM

SEQ ID NO: 21 - DNA, 696 bp, Canis lupus
ggctgagagcagcttcctcagcaggtgggacaggagacctcgttggcgtcctgtgctgcgtcccgtgaggagccatgacggagtataagctggtggtggtgggcgctggaggcgtgggcaagagcgccctgaccatccagctcatccagaaccacttcgtggatgagtacgaccccaccatcgaggactcctatcggaagcaagtggtcatcgacggggagacgtgcctgctggacatcctggacacagcgggccaggaggagtacagcgccatgcgggaccagtacatgcgcacgggggagggctttctctgtgtatttgccatcaacaacaccaagtcctttgaggacatccaccagtacagggagcagatcaagcgagtgaaggactctgacgacgtgcccatggtgctggtggggaacaagtgtgacctggctgctcgcaccgtggagtcccggcaggcgcaggacctcgcccgcagctacggcatcccctacatcgagacgtcagccaagacgcgccagggcagccggtctggctctggctccagctccgggaccctctgggaccctccgggacccccgtgacccagcggcccctagcgctggcgtggaggatgccttctacacgctggtgcgagagattcgacagcacaaggtgcgcaagctgagcccgcccgacgagggaggcccaggc

SEQ ID NO: 22 - protein, 170 aa, Canis lupus
MTEYKLVVVGAGGVGKSALTIQLIQNHFVDEYDPTIEDSYRKQVVIDGETCLLDILDTAGQEEYSAMRDQYMRTGEGFLCVFAINNTKSFEDIHQYREQIKRVKDSDDVPMVLVGNKCDLAARTVESRQAQDLARSYGIPYIETSAKTRQGSRSGSGSSSGTLWDPPGPP

SEQ ID NO: 23 - DNA, 956 bp, Canis lupus
gctgagagcagcttcctcagcaggtgggacaggagacctcgttggcgtcctgtgctgcgtcccgtgaggagccatgacggagtataagctggtggtggtgggcgctggaggcgtgggcaagagcgccctgaccatccagctcatccagaaccacttcgtggatgagtacgaccccaccatcgaggactcctatcggaagcaagtggtcatcgacggggagacgtgcctgctggacatcctggacacagcgggccaggaggagtacagcgccatgcgggaccagtacatgcgcacgggggagggctttctctgtgtatttgccatcaacaacaccaagtcctttgaggacatccaccagtacagggagcagatcaagcgagtgaaggactctgacgacgtgcccatggtgctggtggggaacaagtgtgacctggctgctcgcaccgtggagtcccggcaggcgcaggacctcgcccgcagctacggcatcccctacatcgagacgtcagccaagacgcgccagggcgtggaggatgccttctacacgctggtgcgagagattcgacagcacaaggtgcgcaagctgagcccgcccgacgagggaggcccaggctgcatgagctgcaagtgcctgctgtcctgacgtcccctccagggccacgttggcagccccgctggtcctctgtgccccaggcgcacaggctcggggcgaggaggtgccggaagctgggaggaggcgcggaaggaggaaggaggagggcgaggaaggaaggaagcgcccccggggcccggccagcccaggccccctggacagggggagcacggacctcccagggcgctttgcacagactgtcgtgaactgaggccacgggcccccccggctgtcactctcccccagtcccgtccttgcccgcggggcaaaggctgagtcgcagtaaattatttgatggtcttga

SEQ ID NO: 24 - protein, 189 aa, Canis lupus
MTEYKLVVVGAGGVGKSALTIQLIQNHFVDEYDPTIEDSYRKQVVIDGETCLLDILDTAGQEEYSAMRDQYMRTGEGFLCVFAINNTKSFEDIHQYREQIKRVKDSDDVPMVLVGNKCDLAARTVESRQAQDLARSYGIPYIETSAKTRQGVEDAFYTLVREIRQHKVRKLSPPDEGGPGCMSCKCLLS

SEQ ID NO: 25 - DNA, 593 bp, Felis catus
gccgcgatcccctgaggaacgatgacggaatataagctcgtggtggtgggcgctggaggtgtggggaagagtgccctgaccatccagctcatccagaaccacttcgtggatgagtatgaccccaccatcgaggactcctatcggaagcaagtggttattgatggcgagacgtgcctactggacattttggacacggcgggccaggaggagtatagcgccatgcgggaccagtacatgcgcactggagaaggcttcctctgtgtgtttgccatcaacaataccaagtcctttgaggacatccaccagtacagggagcaaatcaagcgagtgaaggactccgatgacgtgcccatggtgttggtggggaacaagtgcgacctggccgcgcgcaccgtggagtcccggcaggcgcaggacctcgcccgcagctacggcatcccgtacatcgagacgtcggccaagactcgccagggtgtggaggacgctttctacacgctggtccgagagatccggcaacacaaggtgcggaagctgagcccgcccgacgagggtggccccggctgcatgagctgcaagtgcctgctctcctgacg

SEQ ID NO: 26 - protein, 189 aa, Felis catus; identical to SEQ ID NO: 24

SEQ ID NO: 27 - DNA, 675 bp, Felis catus
gccgcgatcccctgaggaacgatgacggaatataagctcgtggtggtgggcgctggaggtgtggggaagagtgccctgaccatccagctcatccagaaccacttcgtggatgagtatgaccccaccatcgaggactcctatcggaagcaagtggttattgatggcgagacgtgcctactggacattttggacacggcgggccaggaggagtatagcgccatgcgggaccagtacatgcgcactggagaaggcttcctctgtgtgtttgccatcaacaataccaagtcctttgaggacatccaccagtacagggagcaaatcaagcgagtgaaggactccgatgacgtgcccatggtgttggtggggaacaagtgcgacctggccgcgcgcaccgtggagtcccggcaggcgcaggacctcgcccgcagctacggcatcccgtacatcgagacgtcggccaagactcgccagggcagccgctctggctctggctccagctccgggaccctctgggaccctccgggacccccgtgacccagcggcccctagcgctggtgtggaggacgctttctacacgctggtccgagagatccggcaacacaaggtgcggaagctgagcccgcccgacgagggtggccccggctgcatgagctgcaagtgcctgctctcctgacg

SEQ ID NO: 28 - protein, 170 aa, Felis catus; identical to SEQ ID NO: 22

SEQ ID NO: 29 - DNA, 978 bp, Bos taurus
ccgccgcggacgggacccatgcgtcgggcgagccctgcgccccggccccggcccctgccgccgcccccgctccggccccggcccggggggcagtcgagccagtgagcggtgggaccggcgaccactgcagcgcctcgtgctgcggtctcttgaggagcaatgacggagtataagctcgtggtggtgggcgccggtggcgtggggaagagcgccctgactatccagctcattcagaatcacttcgtggacgagtacgaccccaccatcgaggactcctaccggaagcaagtggtcatcgatggggagacgtgcctgctggacatcctggacacagcgggccaggaggaatacagcgccatgcgagaccagtacatgcgcaccggggagggctttctctgcgtgtttgctatcaaccacgtcaagtccttcgaggacatccaccagtaccgggagcagatcaagcgggtgaaggactcggatgacgtgcccatggtgttggttgggaacaagtgcgacctggccgcgcgcaccgtggagtctcggcaggcccaggacctcgcccgcagctacggcatcccgtacatcgagacctccgccaagacccgccagggcgtggaggatgctttctacaccctggtgcgcgagatccggcagcacaaggtgcgcaagctgagcccgccggacgagggcggccccggctgcctgagctgcaggtgcctgctctcctgacggcagcgtgggcgcggagcgctgggtgccatgcaggaggcggcgcagcaggggtggagggaggtgccgccagagcccagccccccaggccagtgggcagtgcccgcgggcctcccgggacgcttcgcacagactctggtgaactgatgctgctggcccccagcctcgctctcctccagccctgtcctggcccagcgggcgcaggccgagtcgcagtaaattatttcatggtcttgaaaaaaaaaaaaa

SEQ ID NO: 30 - protein, 189 aa, Bos taurus
MTEYKLVVVGAGGVGKSALTIQLIQNHFVDEYDPTIEDSYRKQVVIDGETCLLDILDTAGQEEYSAMRDQYMRTGEGFLCVFAINHVKSFEDIHQYREQIKRVKDSDDVPMVLVGNKCDLAARTVESRQAQDLARSYGIPYIETSAKTRQGVEDAFYTLVREIRQHKVRKLSPPDEGGPGCLSCRCLLS

SEQ ID NO: 31 - DNA, 1060 bp, Bos taurus
ccgccgcggacgggacccatgcgtcgggcgagccctgcgccccggccccggcccctgccgccgcccccgctccggccccggcccggggggcagtcgagccagtgagcggtgggaccggcgaccactgcagcgcctcgtgctgcggtctcttgaggagcaatgacggagtataagctcgtggtggtgggcgccggtggcgtggggaagagcgccctgactatccagctcattcagaatcacttcgtggacgagtacgaccccaccatcgaggactcctaccggaagcaagtggtcatcgatggggagacgtgcctgctggacatcctggacacagcgggccaggaggaatacagcgccatgcgagaccagtacatgcgcaccggggagggctttctctgcgtgtttgctatcaaccacgtcaagtccttcgaggacatccaccagtaccgggagcagatcaagcgggtgaaggactcggatgacgtgcccatggtgttggttgggaacaagtgcgacctggccgcgcgcaccgtggagtctcggcaggcccaggacctcgcccgcagctacggcatcccgtacatcgagacctccgccaagacccgccagggcagccgctctggctctggctccagctccgggaccctctgggaccctccgggacccccgtgacccagccgcccctctcgctggcgtggaggatgctttctacaccctggtgcgcgagatccggcagcacaaggtgcgcaagctgagcccgccggacgagggcggccccggctgcctgagctgcaggtgcctgctctcctgacggcagcgtgggcgcggagcgctgggtgccatgcaggaggcggcgcagcaggggtggagggaggtgccgccagagcccagccccccaggccagtgggcagtgcccgcgggcctcccgggacgcttcgcacagactctggtgaactgatgctgctggcccccagcctcgctctcctccagccctgtcctggcccagcgggcgcaggccgagtcgcagtaaattatttcatggtcttgaaaaaaaaaaaaa

SEQ ID NO: 32 - protein, 170 aa, Bos taurus
MTEYKLVVVGAGGVGKSALTIQLIQNHFVDEYDPTIEDSYRKQVVIDGETCLLDILDTAGQEEYSAMRDQYMRTGEGFLCVFAINHVKSFEDIHQYREQIKRVKDSDDVPMVLVGNKCDLAARTVESRQAQDLARSYGIPYIETSAKTRQGSRSGSGSSSGTLWDPPGPP

SEQ ID NO: 33 - DNA, 1531 bp, Bos taurus
cccatttaaaacatcgggagaactttctagatttgcagctggcctcctgctgcctcaggacagctgtctagctgcataaaacactccgtttgctcaaaatcgcaaataaactctgatattacttcagcatcgtcctttccagcccgaccaatttccagtggaaacctggctggcagaagacacacagagtgaacttctggtggtgggtagagaggtgcccagcaagatgtggggagaatgaaccggccacggctcactgcgtttgatgaggccctgcaggaggcaaacttcagctggaatggggagagcccaggcgttctgagacctgtggctcgaaaaatacaacggcttctcaactcaaatcagtgacaagaaaaatgaagaaaggcgtggagttagaaagaccccatgagattcggcctcggggagaaaccggttgccaggcacttgctgcccttgggtggtgctaggaggaccaaggcctgagacccccggttccagtgattgagtctgcagagacagaaatgctgcagcagctgccagtggagtggctttgcatggttggcactggatacaagtgtgctaggaagcacgcccgccgagggccacggcctggaccgaggttgaccgtggtcatcagagaccaggagtccgggcttctctcacacaggcagtgggaccggcgaccactgcagcgcctcgtgctgcggtctcttgaggagcaatgacggagtataagctcgtggtggtgggcgccggtggcgtggggaagagcgccctgactatccagctcattcagaatcacttcgtggacgagtacgaccccaccatcgaggactcctaccggaagcaagtggtcatcgatggggagacgtgcctgctggacatcctggacacagcgggccaggaggaatacagcgccatgcgagaccagtacatgcgcaccggggagggctttctctgcgtgtttgctatcaaccacgtcaagtccttcgaggacatccaccagtaccgggagcagatcaagcgggtgaaggactcggatgacgtgcccatggtgttggttgggaacaagtgcgacctggccgcgcgcaccgtggagtctcggcaggcccaggacctcgcccgcagctacggcatcccgtacatcgagacctccgccaagacccgccagggcgtggaggatgctttctacaccctggtgcgcgagatccggcagcacaaggtgcgcaagctgagcccgccggacgagggcggccccggctgcctgagctgcaggtgcctgctctcctgacggcagcgtgggcgcggagcgctgggtgccatgcaggaggcggcgcagcaggggtggagggaggtgccgccagagcccagccccccaggccagtgggcagtgcccgcgggcctcccgggacgcttcgcacagactctggtgaactgatgctgctggcccccagcctcgctctcctccagccctgtcctggcccagcgggcgcaggccgagtcgcagtaaattatttcatggtcttga

SEQ ID NO: 34 - protein, 189 aa, Bos taurus; identical to SEQ ID NO: 30

SEQ ID NO: 35 - DNA, 962 bp, Gallus gallus
gggttgatggccggaccgtcgattccctgacgactacgagcacctacacctgaggtggtggtgctcctggaggccctgagctggggtcagctggaagatgaccgagtacaagctggtggtagtgggagctggaggtgtcgggaagagcgctttgacgatacagctcattcagaaccattttgttgatgagtacgaccccacaatagaggattcctacagaaagcaagtcgtcatcgatggagagacctgtttgctggacatcctggatacggcggggcaggaggagtacagtgccatgcgagaccagtacatgagaacgggggaaggattcctgtgcgtctttgccattaacaacaccaagtcctttgaggacatccaccagtacagggagcagatcaagagggtgaaagactcagatgatgtccccatggtgctggtgggaaataaatgtgatctgccagcacggacagtggagacccggcaagcgcaggacctggcccggagttacgggatcccctacatagaaacgtcggccaaaaccagacagggcgtcgaagatgccttctataccttagtgcgggagatccgtcagcataaactgcgcaagctgaacccaccagatgagagtggccctggctgcatgaactgtaaatgcgtgatatcgtgactgtgctgactggaccctgacttggagaggtgtccgctgtgcagagcacaaggaaagaggtgatgcgaaggaagaaacaaatggattcaggggaggagtggagggggagggagagaggaagaagaggacgggaggagtgccagcccctccaaggactatctcgcacttcacccaggccggcagcagatgacttttggttctttccccatcccctcctcctttggcctcctccaccccggcaactgtacaaagccacagattgaatcacagtaaattattatttgatggtctcgac

SEQ ID NO: 36 - protein, 189 aa, Gallus gallus
MTEYKLVVVGAGGVGKSALTIQLIQNHFVDEYDPTIEDSYRKQVVIDGETCLLDILDTAGQEEYSAMRDQYMRTGEGFLCVFAINNTKSFEDIHQYREQIKRVKDSDDVPMVLVGNKCDLPARTVETRQAQDLARSYGIPYIETSAKTRQGVEDAFYTLVREIRQHKLRKLNPPDESGPGCMNCKCVIS

SEQ ID NO: 37 - DNA, 5436 bp, Homo sapiens
ggccgcggcggcggaggcagcagcggcggcggcagtggcggcggcgaaggtggcggcggctcggccagtactcccggcccccgccatttcggactgggagcgagcgcggcgcaggcactgaaggcggcggcggggccagaggctcagcggctcccaggtgcgggagagaggcctgctgaaaatgactgaatataaacttgtggtagttggagctggtggcgtaggcaagagtgccttgacgatacagctaattcagaatcattttgtggacgaatatgatccaacaatagaggattcctacaggaagcaagtagtaattgatggagaaacctgtctcttggatattctcgacacagcaggtcaagaggagtacagtgcaatgagggaccagtacatgaggactggggagggctttctttgtgtatttgccataaataatactaaatcatttgaagatattcaccattatagagaacaaattaaaagagttaaggactctgaagatgtacctatggtcctagtaggaaataaatgtgatttgccttctagaacagtagacacaaaacaggctcaggacttagcaagaagttatggaattccttttattgaaacatcagcaaagacaagacagagagtggaggatgctttttatacattggtgagggagatccgacaatacagattgaaaaaaatcagcaaagaagaaaagactcctggctgtgtgaaaattaaaaaatgcattataatgtaatctgggtgttgatgatgccttctatacattagttcgagaaattcgaaaacataaagaaaagatgagcaaagatggtaaaaagaagaaaaagaagtcaaagacaaagtgtgtaattatgtaaatacaatttgtacttttttcttaaggcatactagtacaagtggtaatttttgtacattacactaaattattagcatttgttttagcattacctaatttttttcctgctccatgcagactgttagcttttaccttaaatgcttattttaaaatgacagtggaagtttttttttcctctaagtgccagtattcccagagttttggtttttgaactagcaatgcctgtgaaaaagaaactgaatacctaagatttctgtcttggggtttttggtgcatgcagttgattacttcttatttttcttaccaattgtgaatgttggtgtgaaacaaattaatgaagcttttgaatcatccctattctgtgttttatctagtcacataaatggattaattactaatttcagttgagaccttctaattggtttttactgaaacattgagggaacacaaatttatgggcttcctgatgatgattcttctaggcatcatgtcctatagtttgtcatccctgatgaatgtaaagttacactgttcacaaaggttttgtctcctttccactgctattagtcatggtcactctccccaaaatattatattttttctataaaaagaaaaaaatggaaaaaaattacaaggcaatggaaactattataaggccatttccttttcacattagataaattactataaagactcctaatagcttttcctgttaaggcagacccagtatgaaatggggattattatagcaaccattttggggctatatttacatgctactaaatttttataataattgaaaagattttaacaagtataaaaaattctcataggaattaaatgtagtctccctgtgtcagactgctctttcatagtataactttaaatcttttcttcaacttgagtctttgaagatagttttaattctgcttgtgacattaaaagattatttgggccagttatagcttattaggtgttgaagagaccaaggttgcaaggccaggccctgtgtgaacctttgagctttcatagagagtttcacagcatggactgtgtccccacggtcatccagtgttgtcatgcattggttagtcaaaatggggagggactagggcagtttggatagctcaacaagatacaatctcactctgtggtggtcctgctgacaaatcaagagcattgcttttgtttcttaagaaaacaaactcttttttaaaaattacttttaaatattaactcaaaagttgagattttggggtggtggtgtgccaagacattaattttttttttaaacaatgaagtgaaaaagttttacaatctctaggtttggctagttctcttaacactggttaaattaacattgcataaacacttttcaagtctgatccatatttaataatgctttaaaataaaaataaaaacaatccttttgataaatttaaaatgttacttattttaaaataaatgaagtgagatggcatggtgaggtgaaagtatcactggactaggaagaaggtgacttaggttctagataggtgtcttttaggactctgattttgaggacatcacttactatccatttcttcatgttaaaagaagtcatctcaaactcttagttttttttttttacaactatgtaatttatattccatttacataaggatacacttatttgtcaagctcagcacaatctgtaaatttttaacctatgttacaccatcttcagtgccagtcttgggcaaaattgtgcaagaggtgaagtttatatttgaatatccattctcgttttaggactcttcttccatattagtgtcatcttgcctccctaccttccacatgccccatgacttgatgcagttttaatacttgtaattcccctaaccataagatttactgctgctgtggatatctccatgaagttttcccactgagtcacatcagaaatgccctacatcttatttcctcagggctcaagagaatctgacagataccataaagggatttgacctaatcactaattttcaggtggtggctgatgctttgaacatctctttgctgcccaatccattagcgacagtaggatttttcaaacctggtatgaatagacagaaccctatccagtggaaggagaatttaataaagatagtgctgaaagaattccttaggtaatctataactaggactactcctggtaacagtaatacattccattgttttagtaaccagaaatcttcatgcaatgaaaaatactttaattcatgaagcttactttttttttttggtgtcagagtctcgctcttgtcacccaggctggaatgcagtggcgccatctcagctcactgcaacctccatctcccaggttcaagcgattctcgtgcctcggcctcctgagtagctgggattacaggcgtgtgccactacactcaactaatttttgtatttttaggagagacggggtttcaccctgttggccaggctggtctcgaactcctgacctcaagtgattcacccaccttggcctcataaacctgttttgcagaactcatttattcagcaaatatttattgagtgcctaccagatgccagtcaccgcacaaggcactgggtatatggtatccccaaacaagagacataatcccggtccttaggtagtgctagtgtggtctgtaatatcttactaaggcctttggtatacgacccagagataacacgatgcgtattttagttttgcaaagaaggggtttggtctctgtgccagctctataattgttttgctacgattccactgaaactcttcgatcaagctactttatgtaaatcacttcattgttttaaaggaataaacttgattatattgtttttttatttggcataactgtgattcttttaggacaattactgtacacattaaggtgtatgtcagatattcatattgacccaaatgtgtaatattccagttttctctgcataagtaattaaaatatacttaaaaattaatagttttatctgggtacaaataaacaggtgcctgaactagttcacagacaaggaaacttctatgtaaaaatcactatgatttctgaattgctatgtgaaactacagatctttggaacactgtttaggtagggtgttaagacttacacagtacctcgtttctacacagagaaagaaatggccatacttcaggaactgcagtgcttatgaggggatatttaggcctcttgaatttttgatgtagatgggcatttttttaaggtagtggttaattacctttatgtgaactttgaatggtttaacaaaagatttgtttttgtagagattttaaagggggagaattctagaaataaatgttacctaattattacagccttaaagacaaaaatccttgttgaagtttttttaaaaaaagctaaattacatagacttaggcattaacatgtttgtggaagaatatagcagacgtatattgtatcatttgagtgaatgttcccaagtaggcattctaggctctatttaactgagtcacactgcataggaatttagaacctaacttttataggttatcaaaactgttgtcaccattgcacaattttgtcctaatatatacatagaaactttgtggggcatgttaagttacagtttgcacaagttcatctcatttgtattccattgattttttttttcttctaaacattttttcttcaaacagtatataactttttttaggggatttttttttagacagcaaaaactatctgaagatttccatttgtcaaaaagtaatgatttcttgataattgtgtagtaatgttttttagaacccagcagttaccttaaagctgaatttatatttagtaacttctgtgttaatactggatagcatgaattctgcattgagaaactgaatagctgtcataaaatgaaactttctttctaaagaaagatactcacatgagttcttgaagaatagtcataactagattaagatctgtgttttagtttaatagtttgaagtgcctgtttgggataatgataggtaatttagatgaatttaggggaaaaaaaagttatctgcagatatgttgagggcccatctctccccccacacccccacagagctaactgggttacagtgttttatccgaaagtttccaattccactgtcttgtgttttcatgttgaaaatacttttgcatttttcctttgagtgccaatttcttactagtactatttcttaatgtaacatgtttacctggaatgtattttaactatttttgtatagtgtaaactgaaacatgcacattttgtacattgtgctttcttttgtgggacatatgcagtgtgatccagttgttttccatcatttggttgcgctgacctaggaatgttggtcatatcaaacattaaaaatgaccactcttttaattgaaattaacttttaaatgtttataggagtatgtgctgtgaagtgatctaaaatttgtaatatttttgtcatgaactgtactactcctaattattgtaatgtaataaaaatagttacagtgacaaaaaaaaaaaaaaa

SEQ ID NO: 38 - protein, 189 aa, Homo sapiens [sequence omitted]

SEQ ID NO: 39 - DNA, 5312 bp, Homo sapiens
ggccgcggcggcggaggcagcagcggcggcggcagtggcggcggcgaaggtggcggcggctcggccagtactcccggcccccgccatttcggactgggagcgagcgcggcgcaggcactgaaggcggcggcggggccagaggctcagcggctcccaggtgcgggagagaggcctgctgaaaatgactgaatataaacttgtggtagttggagctggtggcgtaggcaagagtgccttgacgatacagctaattcagaatcattttgtggacgaatatgatccaacaatagaggattcctacaggaagcaagtagtaattgatggagaaacctgtctcttggatattctcgacacagcaggtcaagaggagtacagtgcaatgagggaccagtacatgaggactggggagggctttctttgtgtatttgccataaataatactaaatcatttgaagatattcaccattatagagaacaaattaaaagagttaaggactctgaagatgtacctatggtcctagtaggaaataaatgtgatttgccttctagaacagtagacacaaaacaggctcaggacttagcaagaagttatggaattccttttattgaaacatcagcaaagacaagacagggtgttgatgatgccttctatacattagttcgagaaattcgaaaacataaagaaaagatgagcaaagatggtaaaaagaagaaaaagaagtcaaagacaaagtgtgtaattatgtaaatacaatttgtacttttttcttaaggcatactagtacaagtggtaatttttgtacattacactaaattattagcatttgttttagcattacctaatttttttcctgctccatgcagactgttagcttttaccttaaatgcttattttaaaatgacagtggaagtttttttttcctctaagtgccagtattcccagagttttggtttttgaactagcaatgcctgtgaaaaagaaactgaatacctaagatttctgtcttggggtttttggtgcatgcagttgattacttcttatttttcttaccaattgtgaatgttggtgtgaaacaaattaatgaagcttttgaatcatccctattctgtgttttatctagtcacataaatggattaattactaatttcagttgagaccttctaattggtttttactgaaacattgagggaacacaaatttatgggcttcctgatgatgattcttctaggcatcatgtcctatagtttgtcatccctgatgaatgtaaagttacactgttcacaaaggttttgtctcctttccactgctattagtcatggtcactctccccaaaatattatattttttctataaaaagaaaaaaatggaaaaaaattacaaggcaatggaaactattataaggccatttccttttcacattagataaattactataaagactcctaatagcttttcctgttaaggcagacccagtatgaaatggggattattatagcaaccattttggggctatatttacatgctactaaatttttataataattgaaaagattttaacaagtataaaaaattctcataggaattaaatgtagtctccctgtgtcagactgctctttcatagtataactttaaatcttttcttcaacttgagtctttgaagatagttttaattctgcttgtgacattaaaagattatttgggccagttatagcttattaggtgttgaagagaccaaggttgcaaggccaggccctgtgtgaacctttgagctttcatagagagtttcacagcatggactgtgtccccacggtcatccagtgttgtcatgcattggttagtcaaaatggggagggactagggcagtttggatagctcaacaagatacaatctcactctgtggtggtcctgctgacaaatcaagagcattgcttttgtttcttaagaaaacaaactcttttttaaaaattacttttaaatattaactcaaaagttgagattttggggtggtggtgtgccaagacattaattttttttttaaacaatgaagtgaaaaagttttacaatctctaggtttggctagttctcttaacactggttaaattaacattgcataaacacttttcaagtctgatccatatttaataatgctttaaaataaaaataaaaacaatccttttgataaatttaaaatgttacttattttaaaataaatgaagtgagatggcatggtgaggtgaaagtatcactggactaggaagaaggtgacttaggttctagataggtgtcttttaggactctgattttgaggacatcacttactatccatttcttcatgttaaaagaagtcatctcaaactcttagttttttttttttacaactatgtaatttatattccatttacataaggatacacttatttgtcaagctcagcacaatctgtaaatttttaacctatgttacaccatcttcagtgccagtcttgggcaaaattgtgcaagaggtgaagtttatatttgaatatccattctcgttttaggactcttcttccatattagtgtcatcttgcctccctaccttccacatgccccatgacttgatgcagttttaatacttgtaattcccctaaccataagatttactgctgctgtggatatctccatgaagttttcccactgagtcacatcagaaatgccctacatcttatttcctcagggctcaagagaatctgacagataccataaagggatttgacctaatcactaattttcaggtggtggctgatgctttgaacatctctttgctgcccaatccattagcgacagtaggatttttcaaacctggtatgaatagacagaaccctatccagtggaaggagaatttaataaagatagtgctgaaagaattccttaggtaatctataactaggactactcctggtaacagtaatacattccattgttttagtaaccagaaatcttcatgcaatgaaaaatactttaattcatgaagcttactttttttttttggtgtcagagtctcgctcttgtcacccaggctggaatgcagtggcgccatctcagctcactgcaacctccatctcccaggttcaagcgattctcgtgcctcggcctcctgagtagctgggattacaggcgtgtgccactacactcaactaatttttgtatttttaggagagacggggtttcaccctgttggccaggctggtctcgaactcctgacctcaagtgattcacccaccttggcctcataaacctgttttgcagaactcatttattcagcaaatatttattgagtgcctaccagatgccagtcaccgcacaaggcactgggtatatggtatccccaaacaagagacataatcccggtccttaggtagtgctagtgtggtctgtaatatcttactaaggcctttggtatacgacccagagataacacgatgcgtattttagttttgcaaagaaggggtttggtctctgtgccagctctataattgttttgctacgattccactgaaactcttcgatcaagctactttatgtaaatcacttcattgttttaaaggaataaacttgattatattgtttttttatttggcataactgtgattcttttaggacaattactgtacacattaaggtgtatgtcagatattcatattgacccaaatgtgtaatattccagttttctctgcataagtaattaaaatatacttaaaaattaatagttttatctgggtacaaataaacaggtgcctgaactagttcacagacaaggaaacttctatgtaaaaatcactatgatttctgaattgctatgtgaaactacagatctttggaacactgtttaggtagggtgttaagacttacacagtacctcgtttctacacagagaaagaaatggccatacttcaggaactgcagtgcttatgaggggatatttaggcctcttgaatttttgatgtagatgggcatttttttaaggtagtggttaattacctttatgtgaactttgaatggtttaacaaaagatttgtttttgtagagattttaaagggggagaattctagaaataaatgttacctaattattacagccttaaagacaaaaatccttgttgaagtttttttaaaaaaagctaaattacatagacttaggcattaacatgtttgtggaagaatatagcagacgtatattgtatcatttgagtgaatgttcccaagtaggcattctaggctctatttaactgagtcacactgcataggaatttagaacctaacttttataggttatcaaaactgttgtcaccattgcacaattttgtcctaatatatacatagaaactttgtggggcatgttaagttacagtttgcacaagttcatctcatttgtattccattgattttttttttcttctaaacattttttcttcaaacagtatataactttttttaggggatttttttttagacagcaaaaactatctgaagatttccatttgtcaaaaagtaatgatttcttgataattgtgtagtaatgttttttagaacccagcagttaccttaaagctgaatttatatttagtaacttctgtgttaatactggatagcatgaattctgcattgagaaactgaatagctgtcataaaatgaaactttctttctaaagaaagatactcacatgagttcttgaagaatagtcataactagattaagatctgtgttttagtttaatagtttgaagtgcctgtttgggataatgataggtaatttagatgaatttaggggaaaaaaaagttatctgcagatatgttgagggcccatctctccccccacacccccacagagctaactgggttacagtgttttatccgaaagtttccaattccactgtcttgtgttttcatgttgaaaatacttttgcatttttcctttgagtgccaatttcttactagtactatttcttaatgtaacatgtttacctggaatgtattttaactatttttgtatagtgtaaactgaaacatgcacattttgtacattgtgctttcttttgtgggacatatgcagtgtgatccagttgttttccatcatttggttgcgctgacctaggaatgttggtcatatcaaacattaaaaatgaccactcttttaattgaaattaacttttaaatgtttataggagtatgtgctgtgaagtgatctaaaatttgtaatatttttgtcatgaactgtactactcctaattattgtaatgtaataaaaatagttacagtgacaaaaaaaaaaaaaaa

SEQ ID NO: 40 - protein, 188 aa, Homo sapiens [sequence omitted]

SEQ ID NO: 41 - DNA, 661 bp, Rattus norvegicus
atgactgagtataaacttgtggtagttggagctggtggcgtaggcaagagtgccttgacgatacagctaattcagaatcactttgtggatgaatatgatcctacgatagaggactcctacaggaaacaagtagtaattgatggagaaacctgtctcttggatattctcgacacagcaggtcaagaggagtacagtgcaatgagggaccagtacatgagaactggggagggctttctttgtgtatttgccataaataatactaaatcatttgaagatattcaccattatagagaacaaattaaaagagtaaaggactctgaagatgtgcctatggtcctagtagggaataagtgtgacttgccttctagaacagtagacacgaaacaggctcaggagttagcaaggagttatgggattccattcattgagacctcagcgaagacaagacagggtgttgacgatgccttctatacattagtccgagaaattcgaaaacataaagaaaagatgagcaaagatgggaaaaagaagaagaagaagtcaaggacaaggtgtatagtcatgtgaatagtttgtactctttcttaaggcacacttaagtaaagtgtgatttttgtacattacactaaattattagcatttgttttagcattacctaatc

SEQ ID NO: 42 - protein, 188 aa, Rattus norvegicus
MTEYKLVVVGAGGVGKSALTIQLIQNHFVDEYDPTIEDSYRKQVVIDGETCLLDILDTAGQEEYSAMRDQYMRTGEGFLCVFAINNTKSFEDIHHYREQIKRVKDSEDVPMVLVGNKCDLPSRTVDTKQAQELARSYGIPFIETSAKTRQGVDDAFYTLVREIRKHKEKMSKDGKKKKKKSRTRCIVM

SEQ ID NO: 43 - DNA, 4670 bp, Mus musculus
aggcggcggccgcggcggctgaggcggcagcgctgtggcggcggctgagacggcaggggaaggcggcggcggctcggcccggagtcccgctcccgcgccatttcggacccggagcgagcgcggcgcgggcctgaaggcggcggcgggagcctgaggcgcggcggctccgcggcgcggagagaggcctgctgaaaatgactgagtataaacttgtggtggttggagctggtggcgtaggcaagagcgccttgacgatacagctaattcagaatcactttgtggatgagtatgaccctacgatagaggactcctacaggaaacaagtagtaattgatggagaaacctgtctcttggatattctcgacacagcaggtcaagaggagtacagtgcaatgagggaccagtacatgagaactggggagggctttctttgtgtatttgccataaataatactaaatcatttgaagatattcaccattatagagaacaaattaaaagagtaaaggactctgaagatgtgcctatggtcctggtagggaataagtgtgatttgccttctagaacagtagacacgaaacaggctcaggagttagcaaggagttacgggattccgttcattgagacctcagcaaagacaagacagggtgttgacgatgccttctatacattagtccgagaaattcgaaaacataaagaaaagatgagcaaagatgggaagaagaagaagaagaagtcaaggacaaggtgtacagttatgtgaatactttgtactctttcttaaggcacacttaagtaaaagtgtgatttttgtacattacactaaattattagcatttgttttagcattacctaatctttttttttcttctgttcgtgcaaactgtcagcttttatctcaaatgcttattttaaaagaacagtggaaaccttcttttttctaagtgccagtattccctgggttttggacttaaactagcaatgcctgtggaagagactaaagacctgagactctgtcttgggatttggtgcatgcagttgattccttgctagttctcttaccaactgtgaacactgatgggaagcaggataatgaagcttccggaccatccctgctctgtgtccatctactcatccaatggagtcattagcagtcaatcgccgcttcactggacactgaggggtcacagacttaggctccctttgagtcgcgtccagcgtgtcctagactttatcatctttcagaggcgtaggcagactgttcacaaaggctttctgtagctttccactgcaattaatcttggtcactccctcaaatagtatattttttctagaaaaggggaaaaatggaaaaaaaaaggcaatggaaaatgttgaaatccattcagtttccatgttagctaaattactgtaagattcctataatagcttttcctggtaaggcagacccagtatgaaatagtaataaccatttgggctatatttacatgctactaaatttttgtaataattcaaacaactttagcatatataaaaagttctcataagaattaagtacaattcccctttgtcagattgttcttatcctaactttcaagtcttttttgaatttctgttgttgaaagtagttttaatggttgtgaagctgaagatgatctgagacagttatagcttggcaggtgttgaggagaccagagttgcagggttgggccttacgtgaacctgtgacgaacgctactgggttttgcagcactgctgcattcaatgttggcgacgcattgtttggtcaacataggggataaggagactttgatggcttagtataatgcattctcaccatgtaacagtcctactgacaaatcaagaaatttgtttataataataaaaaatttttaaaaatttcgatgttcgcttcaaggttgagattttggggtaggaggctacaacaagagtaaatcttaaagcaaggttttaagaaggtttgaaaatgcaggtttgactagtctctcaactctagctaaacaaacattcccaagtacttcccaaatctgataggtatttaaaattatctaatgctttaagaatagttaacaggaaaaaaatctcctcagtgcacttaaagcaacccttcacatcatttgaaatgagatggaaatatcactggactatgaggactggatgtctgtctgattttaagcaaatcactgtctgcttggttttgaatcatctcaaagacattaacctcccagccgtgtaacatagtttacatgttgacacacctagttatcaagctcagcacaatctgtaactgttttacatggattaacatcttcactgccagtcttgggcaaattgtgcaagaggtaaaatttatatttcagtatccattctcccatttcaggactcccctccaacattatgctggctttcagcctgtctctcacctgcccatcacttagtgtagttttaataatttcccccacttcaaactttgtttccactatggacaacttcatgaactttgcccactaaggtaggtacatcaaagctgccctatggctttcttccccgggactgaaaataacagacaccatagtgggatttaaactaatagatggttttcagggccactacaacaattcaatctcaatcctttggacttcattcctgctgcccaggccactggtgcctcagtaggaattttcaaaattagtgtgaacagacagagcacagtccagtggaaggtgagcttaatcttcatctagccatcatcatggtaagtgatagattctattgttttaataaatacagtctaacaatgaaaaacacttcgaagtttcaatcataaagctgtctttttaaaaattttatttactcaacatttattcagtgcttgtcatattctgggaattacactaggcactcagggtgcggtgtcctcaatccttggccagtggtatgtagcatgatctgtaataccactaaataaggcatatagcatatgacttagacataatgaaatacatgatttgagttttgcagagaggagtttgggtttgtacattcccttcccccccagtttagcaagaattgtttgctgtgaatccaatgcaacttttaaatcaaactactttatataattatttcatttttctaaaggaacagaagtaccctaaactatttttttgaaatgttctaaactgtacatattcatagaacattctttgggtgaattttaagtcttaaaatgcaattagtaatacttctcatttctattcagaggaacaggtgtacttcaaaagctgcagtgtataatcagatatttttaatggacaatgtgttaaagaagtggtaattaccactatgtaaatttgaattgtgttacactttggttaacaaaaggggaaagaatcctagaaacaaatatgttatctagttactgcagccttaaagtccttgttgaagttaaaaagcaatgctaagttacagtcataggcattaacatgtttatgggaaggatatagtaggcaaatacaatttgagtaaatattttcagtagggaattttaggctctactgactgagtcacactgcataggaatttagatcttaacttttataggttatcgacctttgccaccattgcacaattttgtcctaacataaatacaagttctgtgaggcatgtcaaaagttacagtttgcataaattcatctcattttgtattccactgattttacattttcctcaaacatacatacatacatacatacaacacacacacactcacacatgaagggttttttttttgtaggcaataaaaatttaactaatttccatttgttaaaaagtagtgatttattgagaattatgcagtcattttttaaacccaaaagttatttaaaggtgaatttatactcaataacttctgtgtaatactgggtagcatgaattctgcattgaaaaattgaacagataataccaatagctgtaaattctgtcaaaacatgaaaattatttctaaagaagtacattagttttcaaagaacagttattagaatcagatctgtggtttagttcaataatttgaagtgcctgtttgggatggtggtaggcattttagatgaatttgggaaaaataaagttctgcagaaatgccagtttcagaccccgctaacccgctgagtgggctgtgtgctgtgttagctccagtgccccaatcccgtttcatgtcttcatgttgaaacacttctgcatttttatttgagtgccaatttcttactagtgctatttcttagtgtaacatgtttacctgggatgtattttaactatttttgtatagtgtaaactgaaacatgcacattttgtacattgtgctttccttctttccattccttttctttctgttttgtttgtttgtttgtttgtttgtttgttatgggacatatgcagtgtgatccagttgttttccatcctttggttgcgctgacctagggaatgttggtcatatcaaacattaaatttaaaagtgaccactcttaattaaaattaacttttaaatgtttataggagtacgtgctgtgaagtgatctgaaatttgtaatatttttgtcatgaaccgtactgctcctaatcattgtaatgtaataaaaatagttatggtgactatgaa

SEQ ID NO: 44 - protein, 188 aa, Mus musculus
MTEYKLVVVGAGGVGKSALTIQLIQNHFVDEYDPTIEDSYRKQVVIDGETCLLDILDTAGQEEYSAMRDQYMRTGEGFLCVFAINNTKSFEDIHHYREQIKRVKDSEDVPMVLVGNKCDLPSRTVDTKQAQELARSYGIPFIETSAKTRQGVDDAFYTLVREIRKHKEKMSKDGKKKKKKSRTRCTVM

SEQ ID NO: 45 - DNA, 2068 bp, Oryctolagus cuniculus
acacacgcgcccacccagccacccggccaccagccgccatgggcaaggacaggcagccccgcgggcagcagaggcagggggacgccgccgggcccgacgacccggggccgaagaaaggcgccgggacccgcgagcagcgcggggaggaggaggcccagacgtgctgcggctgccgcttcccgctgctgctcgcgctgctgcagctggccctgggcgtcgccgtgaccgtggtgggcttcctcatggcgagcgtcagctcctccctgctagtcagagccactccatattgggctgggatcattgtctgcgtggtggcctatcttggcttgtttatgctttgtgtctcgtaccaagttgatgaacggacgtgtatccagttttctatgaaactgctgtacttcgtgctgagcgccctggggctggtggtgtgcgtgctggccgtggccttcgccgcccaccactactcgctgctcacgcacctgacctgtgagaacgcccccgactcctgccagtgcaagctgccgtcctcggagccgctgagccggaccttcgtgtaccgggatgtgactgactgtaccagcatcacgggcaccttccaggtgttcctgctcgtccagatggttctgaacttggtctgtggccttgtgtgcttggtggcctgctttgtgatgtggaaacacaggtatcaggtcttttatgtgggggtcaggatgtgccccctgtcggcttccgaaggccagcagcagaaggtgtaggaatcttgctcagaattgggagagaaaatggcacactggctagctgaggttaaaaagaaaaattatttttaaggagaaagagagaaaacttttgccaatatttactgctctaaatgaatattttttatatttttcaagaaacaaaagagcatttcttcaggtttctattgtatttttaaacattcgtataggttcaacaagatacacattgatttgcgggatattcaaagtcaaaagcacaccaaactgggaagcaatggcacagaactgtcctcacagtctggggtttactcttcatgctcactttcgccaccactgacgtacggctttctggttaatacggtctaaggtttgtagtggctgccccaggtccttcccgcctcctaccacaatcccccactgcgtcttagagaaaggcaaggtgtggagaagtcactgggcaaccaggtggaatctcttcatttcccctactgcggatgttgtcaaggcccaaaacatgagcgaacttcaaaaacctcatgggaagtggagttcgaagtttattttgctgccaaaaaattaagatccacacatatatagggatcttcagaaagttcacagaaaatgcataatatgggaaaaaaaaagattcacggatttcagaattttgtttggaccaaactaaagttatcttttaatgccatttctgaagtgccctcatagcttggaaagccaagcagaaaagaggctttgcaaaaatacaagtaattataaacacctgggccagggcggctgtctcagctgccttcgcttggctctgtacgtagatcactcgcgcggggcttggcagggctctctgcttctcaataattgaaatatggtggtagttgtattcttaatgatgtagaaggtttaaaaataattacattacgcttccattctatcatctacaacaaatcattcaacctaatttctagctaattgttaattataattatgctcagaagtctatttaatgagctctggctgtacttaggcagctctgccagtgtaaagagaaattattctcgtaagagaagaggcctaaagattctttcttctgaaagtcaagcgttataagggaaaacttttttttaattaatagctcaggataaaaacaccaatttaaacaaaaacaagagcatttataataggaagtacttgtacaaatagcacgtttgtggcacattgcagagtgtctctctttgcagctaaatagctttgaagaaggctggcgagtgcagatgtattctgtgcacaaaactgtatttggctcataaccctattattgattc

SEQ ID NO: 46 - protein, 238 aa, Oryctolagus cuniculus
MGKDRQPRGQQRQGDAAGPDDPGPKKGAGTREQRGEEEAQTCCGCRFPLLLALLQLALGVAVTVVGFLMASVSSSLLVRATPYWAGIIVCVVAYLGLFMLCVSYQVDERTCIQFSMKLLYFVLSALGLVVCVLAVAFAAHHYSLLTHLTCENAPDSCQCKLPSSEPLSRTFVYRDVTDCTSITGTFQVFLLVQMVLNLVCGLVCLVACFVMWKHRYQVFYVGVRMCPLSASEGQQQKV

SEQ ID NO: 47 - DNA, 1039 bp, Cavia porcellus
ggtggcttctcggccagacctcccggcccccgccatttcggaccgggagccagcgcgacgcgggcactgagggcggcggcgggggccacaggctcggcggctcccaggtgcgggagagaggcctgctgaaaatgactgaatataaacttgtggtagttggagctggtggcgtaggcaagagtgccttgacgatacagctaattcagaatcactttgtggatgaatatgatcctacaatagaggattcctacaggaaacaagtagtaattgatggagaaacctgtctcttggatattctcgacacagcaggtcaagaggagtacagtgcaatgagggaccagtacatgaggactggggagggctttctttgtgtatttgccataaataatactaaatcttttgaagatattcaccattatagagaacaaattaaaagagttaaagactctgaagatgtacctatggtcctagtaggaaataaatgtgatttgccttctagaacagtagacacaaaacaagctcaggacttagcaagaagttatggaattccttttattgaaacatcagcaaagacaagacagagagtggaggatgctttttatacattggtgagagagattcgacaatacagattgaaaaaaatcagcaaagaagaaaagactcctggctgtgtgaaaattaaaaaatgcattataatgggtgttgatgatgccttctatacgttagttcgagaaattcgaaaacataaagaaaagatgagcaaagatggtaaaaagaagaaaaagaagtcgaagacaaagtgtataattatgtaaatacaatttgtacttttttcttaaggcatacttaagtaaaagtggtaatttttgtacattacactaaattattagcttttgttttagcattacttaattcttttcctatttcatgcaaactgttagcttttatcttaaatgctcattttaaaatgacagtggaaaccttttatttcctcttaagtgccagtattccctgcattttggtttttgaactagcaatg

SEQ ID NO: 48 - protein, 227 aa, Cavia porcellus
MTEYKLVVVGAGGVGKSALTIQLIQNHFVDEYDPTIEDSYRKQVVIDGETCLLDILDTAGQEEYSAMRDQYMRTGEGFLCVFAINNTKSFEDIHHYREQIKRVKDSEDVPMVLVGNKCDLPSRTVDTKQAQDLARSYGIPFIETSAKTRQRVEDAFYTLVREIRQYRLKKISKEEKTPGCVKIKKCIIMGVDDAFYTLVREIRKHKEKMSKDGKKKKKKSKTKCIIM

SEQ ID NO: 49 - DNA, 835 bp, Cavia porcellus
acaggctcggcggctcccaggtgcgggagagaggcctgctgaaaatgactgaatataaacttgtggtagttggagctggtggcgtaggcaagagtgccttgacgatacagctaattcagaatcactttgtggatgaatatgatcctacaatagaggattcctacaggaaacaagtagtaattgatggagaaacctgtctcttggatattctcgacacagcaggtcaagaggagtacagtgcaatgagggaccagtacatgaggactggggagggctttctttgtgtatttgccataaataatactaaatcttttgaagatattcaccattatagagaacaaattaaaagagttaaagactctgaagatgtacctatggtcctagtaggaaataaatgtgatttgccttctagaacagtagacacaaaacaagctcaggacttagcaagaagttatggaattccttttattgaaacatcagcaaagacaagacagggtgttgatgatgccttctatacgttagttcgagaaattcgaaaacataaagaaaagatgagcaaagatggtaaaaagaagaaaaagaagtcgaagacaaagtgtataattatgtaaatacaatttgtacttttttcttaaggcatacttaagtaaaagtggtaatttttgtacattacactaaattattagcttttgttttagcattacttaattcttttcctatttcatgcaaactgttagcttttatcttaaatgctcattttaaaatgacagtggaaaccttttatttcctcttaagtgccagtattccctgcattttggtttttgaactagcaatg

SEQ ID NO: 50 - protein, 188 aa, Cavia porcellus
MTEYKLVVVGAGGVGKSALTIQLIQNHFVDEYDPTIEDSYRKQVVIDGETCLLDILDTAGQEEYSAMRDQYMRTGEGFLCVFAINNTKSFEDIHHYREQIKRVKDSEDVPMVLVGNKCDLPSRTVDTKQAQDLARSYGIPFIETSAKTRQGVDDAFYTLVREIRKHKEKMSKDGKKKKKKSKTKCIIM

SEQ ID NO: 51 - DNA, 4993 bp, Canis lupus
gctgaaaatgactgaatataaacttgtggtagttggagctggtggcgtaggcaagagtgccttgacgatacagctaattcagaatcactttgtggatgaatatgatcctacaatagaggattcctacaggaaacaagtagtaattgatggagaaacctgtctcttggatattctcgacacagcaggtcaagaggagtacagtgcaatgagggaccagtacatgaggactggggagggctttctttgtgtatttgccataaataatactaaatcatttgaagatattcaccattatagagaacaaattaaaagagttaaagactctgaagatgtacctatggtcctagtaggaaataaatgtgatttgccttctagaacagtagacacaaaacaggctcaggacttagcaagaagttatggaattccttttattgaaacatcagcaaagacaagacagagagtggaggatgctttttatacattggtgagagagatccgacaatacagattgaaaaaaatcaacaaagaagaaaagactcctggctgtgtgaaaattaaaaaatgcattgtaatgggtgttgacgatgccttctatacattagttcgagaaattcgaaaacataaagaaaagatgagcaaagatggtaaaaagaagaaaaagaagtcaaagacaaagtgtataattatgtaaatacaatttgtacttttttcttaaggcatacttaagtaaaagtggtaatttttgtacattacactaaattattagcatttgttttagcattacctaattttctgctccatccaaactgttagcttttatcttgaatgcttattttaaaatgacagtggaaactttttcctctaagtgccagtattccctgagttttggttttgaactagcaatgcctgtgaaaaagaaactgaatacctgagatttctgtcttggggtttttggtgcatgcagttgattacttcctatttttcttaccaattgtgaactttggtgtgaaacaaattaatgaagctttcgaatcatccctattctgtgttttacctagtcacatacatggattaattactaattataacttcagttgatatttcatgattggttttactgaaacattgagggaacatgaatttatgggctgcttcttataggtataatgtcctatagtttcagtcacccttaatgaatgtaaagctacactgttcacaaaggttttctccatcttttcactgctatttgtcatagccacgctcccaaaaatattatattttttctataaaaaagggaaaaaatagaaaaaaatacaaggcaatggaaaatattaaaaggcatttactttccatattagataaattcctataatactctgaatagcttttcctgttaaggcagacccagtatgtaatgaggattatagcaaccattttggggctatatttacatgctactaaatttttgtattaattgaaaaagttttaacatgtataaaaaattcccataggaattaaatatagtctccctgtgtcagattgctctttcttagcataactttaaatcttttcttgatcttcaatcttagaaaatagttttaattcttgtagtgatgttaaagattatttgggccagttagtttttaatagatgttaaagagaccacagttccaaggccaggccttgtgtgaacctttaagcttcattaagagtttcatagtacagactgcatccctgtggtctcccagggtcatcatgcattgattgggtggtcaaaagtggggacaaagagtgtttagataagatgcatcctcactgtatggtggtcctgctgacagatcaggaccatcacttttgttttttaaaaaaccaacagagctttttaaaaacattatttaaaatgagatttttgggggcagggggtggcaagacttgaattttttttaaacaatgaagtaaaaaggtttcaaaatctctagtgttggctagttctcaacattggctaaagtaacatttcataaacactttacaagtattggtccatatttaagaatatctaatgcttaaataatagattaataacaattctttcagtgcatttaaaatgtatttttaaatatctgaagtgagatggtgtgttgaggtgaaaatatcactggactaggaggaaggtgacttagattctagttacgtgtcttttacaacttcagttttgggcaaatcactcactatccatttcttcatgttaagtcatctcaaaggctatatctagcatcaactatgtgatttacattcagtttacataaggatatacctatttgtcaatctcagcacaatctgtaactttttacctatgttctcttcagcgccagtcttaggcaaagttgtgcaagaggtgaggtttatttttgagaatctgatctccggtagcaggtactcctctcccatgttagtgtcatcttgcctgcctaccttctacatgccccatgacttgatgctttctaattccccgaacctcaagatgtagtgctgctttggatatctccatgaggtaataagtcacattagtcaggctcaacataatctgacagatactgtagtgggatttgatctaatagctaattttcaggtggtaactgtatcaatttaattttgatcttttgaacatcatctctgctacctggtccattagtgactaagtaggaaaagtaggaattttcatatctgtgatgtgtagacagaccctatccagtagaagaatttaataaatttaattaataaatactgaaagatttccttagataatccaaaactaggactagccctggtaacggtgatacattccattattttaataagtaaaatcttcttacaatgaaaaatactttaaaatttaattcataaagcttactttttagcagaattcatttattcaacaaatacttgagtgcctgctagatgccaggttctacacaaggcaccggggatattatggtattcccaacaagggacataatccctatccttaagtagtactgttattttagagtggtctgtagtatattagtgaggcatttggcacatgacccagagataatataatgcatattttagttttgcacagaagggatatggtctctaaggttttttccagctctaaaataattgttcgctctgattccaataaactgtttaatcaagctactttatataaatcactttacttcattattttaaagaagtaaacttgactatattgttttttatttgggataattatgtgattctgttgggatacttatatagtacacattaaattgtatgtcagatgataacattaaaattcccaagtgtaatattctacttggtctctgtgtatcataattaaaatagatttaaatattgagttcaaaaatagttttatttatctgggtgtgaataaacagatgcctgaactaattcacagaaaaggaaacttctgtgtaaaaagtcagtccaatttctgaaatgctatgctaaactacaggtttatggaacattagatagggtgttaagactttatatagtacttcctcttgtttctatacaagagaaagaaatggccatacttcaggaattgcagtgcataactgagggatttttaggactcttgaatttttgatgtagccgggcaactttttttaggcagtggtaattatcctttattatgtgaattttgaatggtttgacaaaacgtttgtttttgtagagattttaaaaggggagcgctaatcctagaaataaatattatgtaattattacggccttaaagataaaaatccttgttgaaagttgaaaaaaattgctaaattacatagtcttagacattaacatgtttgtggaagaatgtagcagaggtatgtagtataatttgagtgaatattcccaattaggaattctaggctctagtttaactgagtcacactgcataggaatttagaacctaacttctaggttatcaaaatctttgccaccattgcacaattttgtcctaatatatagagaaactttgtgaggcatgttcagttgcggtttgcacaagttcatctcatttgtattccagtgattttttttcttctaaccatttttttaaacaacatgtacacattgttttttttggtaggcaatgaaaactgtcatttccattgtcaaacagtaattcctcgataactgtattaatggtttttaaaaaaccatcagttactttaaaactgaatttatatttaataacttctgtattagtattgggtagcatgaaatctctattgagaaattgaacagcatacaactagtagctgtaaattccttcagaaagtgaaaattatttcttcctaaagatatcttgacatcagtgcttgaagaatagtcataactagattaataattgttttagttaaacagttttaagtgcctgtttcagatgatgataggcaatttagatgaatttaggaaaaatcaaagtttttacttgcagaaatgtccattatagggggcccccctcctcatagagctgaatgggttatgtaatgttttatccaaaagtttccaattccactgtcttgtgttttcatgttgaaaatacttttgcatttttcctttgagtgccaatttcttactagtactatttcttaatgtaacatgtttacctggaatgtattttaactatttttgtatagtgtaaactgaaacatgcacattttgtacattgtgcttttttttgtgggacatatgcagtgtgatccagttgttttccatcatttggttgcgctgacctaggaatgttggtcatatcaaacattaaatttaaaaatgaccactcttttaattaaaattaacttttaaatgtttataggagtatgtgctgtgaagtgatctgaaatttgtaatatttttgtcatgaactgtactgctcctaattattgtaatgtaataaaaatagttatggtgactatga

SEQ ID NO: 52 - protein, 4993 aa, Canis lupus
GCTGAAAATGACTGAATATAAACTTGTGGTAGTTGGAGCTGGTGGCGTAGGCAAGAGTGCCTTGACGATACAGCTAATTCAGAATCACTTTGTGGATGAATATGATCCTACAATAGAGGATTCCTACAGGAAACAAGTAGTAATTGATGGAGAAACCTGTCTCTTGGATATTCTCGACACAGCAGGTCAAGAGGAGTACAGTGCAATGAGGGACCAGTACATGAGGACTGGGGAGGGCTTTCTTTGTGTATTTGCCATAAATAATACTAAATCATTTGAAGATATTCACCATTATAGAGAACAAATTAAAAGAGTTAAAGACTCTGAAGATGTACCTATGGTCCTAGTAGGAAATAAATGTGATTTGCCTTCTAGAACAGTAGACACAAAACAGGCTCAGGACTTAGCAAGAAGTTATGGAATTCCTTTTATTGAAACATCAGCAAAGACAAGACAGAGAGTGGAGGATGCTTTTTATACATTGGTGAGAGAGATCCGACAATACAGATTGAAAAAAATCAACAAAGAAGAAAAGACTCCTGGCTGTGTGAAAATTAAAAAATGCATTGTAATGGGTGTTGACGATGCCTTCTATACATTAGTTCGAGAAATTCGAAAACATAAAGAAAAGATGAGCAAAGATGGTAAAAAGAAGAAAAAGAAGTCAAAGACAAAGTGTATAATTATGTAAATACAATTTGTACTTTTTTCTTAAGGCATACTTAAGTAAAAGTGGTAATTTTTGTACATTACACTAAATTATTAGCATTTGTTTTAGCATTACCTAATTTTCTGCTCCATCCAAACTGTTAGCTTTTATCTTGAATGCTTATTTTAAAATGACAGTGGAAACTTTTTCCTCTAAGTGCCAGTATTCCCTGAGTTTTGGTTTTGAACTAGCAATGCCTGTGAAAAAGAAACTGAATACCTGAGATTTCTGTCTTGGGGTTTTTGGTGCATGCAGTTGATTACTTCCTATTTTTCTTACCAATTGTGAACTTTGGTGTGAAACAAATTAATGAAGCTTTCGAATCATCCCTATTCTGTGTTTTACCTAGTCACATACATGGATTAATTACTAATTATAACTTCAGTTGATATTTCATGATTGGTTTTACTGAAACATTGAGGGAACATGAATTTATGGGCTGCTTCTTATAGGTATAATGTCCTATAGTTTCAGTCACCCTTAATGAATGTAAAGCTACACTGTTCACAAAGGTTTTCTCCATCTTTTCACTGCTATTTGTCATAGCCACGCTCCCAAAAATATTATATTTTTTCTATAAAAAAGGGAAAAAATAGAAAAAAATACAAGGCAATGGAAAATATTAAAAGGCATTTACTTTCCATATTAGATAAATTCCTATAATACTCTGAATAGCTTTTCCTGTTAAGGCAGACCCAGTATGTAATGAGGATTATAGCAACCATTTTGGGGCTATATTTACATGCTACTAAATTTTTGTATTAATTGAAAAAGTTTTAACATGTATAAAAAATTCCCATAGGAATTAAATATAGTCTCCCTGTGTCAGATTGCTCTTTCTTAGCATAACTTTAAATCTTTTCTTGATCTTCAATCTTAGAAAATAGTTTTAATTCTTGTAGTGATGTTAAAGATTATTTGGGCCAGTTAGTTTTTAATAGATGTTAAAGAGACCACAGTTCCAAGGCCAGGCCTTGTGTGAACCTTTAAGCTTCATTAAGAGTTTCATAGTACAGACTGCATCCCTGTGGTCTCCCAGGGTCATCATGCATTGATTGGGTGGTCAAAAGTGGGGACAAAGAGTGTTTAGATAAGATGCATCCTCACTGTATGGTGGTCCTGCTGACAGATCAGGACCATCACTTTTGTTTTTTAAAAAACCAACAGAGCTTTTTAAAAACATTATTTAAAATGAGATTTTTGGGGGCAGGGGGTGGCAAGACTTGAATTTTTTTTAAACAATGAAGTAAAAAGGTTTCAAAATCTCTAGTGTTGGCTAGTTCTCAACATTGGCTAAAGTAACATTTCATAAACACTTTACAAGTATTGGTCCATATTTAAGAATATCTAATGCTTAAATAATAGATTAATAACAATTCTTTCAGTGCATTTAAAATGTATTTTTAAATATCTGAAGTGAGATGGTGTGTTGAGGTGAAAATATCACTGGACTAGGAGGAAGGTGACTTAGATTCTAGTTACGTGTCTTTTACAACTTCAGTTTTGGGCAAATCACTCACTATCCATTTCTTCATGTTAAGTCATCTCAAAGGCTATATCTAGCATCAACTATGTGATTTACATTCAGTTTACATAAGGATATACCTATTTGTCAATCTCAGCACAATCTGTAACTTTTTACCTATGTTCTCTTCAGCGCCAGTCTTAGGCAAAGTTGTGCAAGAGGTGAGGTTTATTTTTGAGAATCTGATCTCCGGTAGCAGGTACTCCTCTCCCATGTTAGTGTCATCTTGCCTGCCTACCTTCTACATGCCCCATGACTTGATGCTTTCTAATTCCCCGAACCTCAAGATGTAGTGCTGCTTTGGATATCTCCATGAGGTAATAAGTCACATTAGTCAGGCTCAACATAATCTGACAGATACTGTAGTGGGATTTGATCTAATAGCTAATTTTCAGGTGGTAACTGTATCAATTTAATTTTGATCTTTTGAACATCATCTCTGCTACCTGGTCCATTAGTGACTAAGTAGGAAAAGTAGGAATTTTCATATCTGTGATGTGTAGACAGACCCTATCCAGTAGAAGAATTTAATAAATTTAATTAATAAATACTGAAAGATTTCCTTAGATAATCCAAAACTAGGACTAGCCCTGGTAACGGTGATACATTCCATTATTTTAATAAGTAAAATCTTCTTACAATGAAAAATACTTTAAAATTTAATTCATAAAGCTTACTTTTTAGCAGAATTCATTTATTCAACAAATACTTGAGTGCCTGCTAGATGCCAGGTTCTACACAAGGCACCGGGGATATTATGGTATTCCCAACAAGGGACATAATCCCTATCCTTAAGTAGTACTGTTATTTTAGAGTGGTCTGTAGTATATTAGTGAGGCATTTGGCACATGACCCAGAGATAATATAATGCATATTTTAGTTTTGCACAGAAGGGATATGGTCTCTAAGGTTTTTTCCAGCTCTAAAATAATTGTTCGCTCTGATTCCAATAAACTGTTTAATCAAGCTACTTTATATAAATCACTTTACTTCATTATTTTAAAGAAGTAAACTTGACTATATTGTTTTTTATTTGGGATAATTATGTGATTCTGTTGGGATACTTATATAGTACACATTAAATTGTATGTCAGATGATAACATTAAAATTCCCAAGTGTAATATTCTACTTGGTCTCTGTGTATCATAATTAAAATAGATTTAAATATTGAGTTCAAAAATAGTTTTATTTATCTGGGTGTGAATAAACAGATGCCTGAACTAATTCACAGAAAAGGAAACTTCTGTGTAAAAAGTCAGTCCAATTTCTGAAATGCTATGCTAAACTACAGGTTTATGGAACATTAGATAGGGTGTTAAGACTTTATATAGTACTTCCTCTTGTTTCTATACAAGAGAAAGAAATGGCCATACTTCAGGAATTGCAGTGCATAACTGAGGGATTTTTAGGACTCTTGAATTTTTGATGTAGCCGGGCAACTTTTTTTAGGCAGTGGTAATTATCCTTTATTATGTGAATTTTGAATGGTTTGACAAAACGTTTGTTTTTGTAGAGATTTTAAAAGGGGAGCGCTAATCCTAGAAATAAATATTATGTAATTATTACGGCCTTAAAGATAAAAATCCTTGTTGAAAGTTGAAAAAAATTGCTAAATTACATAGTCTTAGACATTAACATGTTTGTGGAAGAATGTAGCAGAGGTATGTAGTATAATTTGAGTGAATATTCCCAATTAGGAATTCTAGGCTCTAGTTTAACTGAGTCACACTGCATAGGAATTTAGAACCTAACTTCTAGGTTATCAAAATCTTTGCCACCATTGCACAATTTTGTCCTAATATATAGAGAAACTTTGTGAGGCATGTTCAGTTGCGGTTTGCACAAGTTCATCTCATTTGTATTCCAGTGATTTTTTTTCTTCTAACCATTTTTTTAAACAACATGTACACATTGTTTTTTTTGGTAGGCAATGAAAACTGTCATTTCCATTGTCAAACAGTAATTCCTCGATAACTGTATTAATGGTTTTTAAAAAACCATCAGTTACTTTAAAACTGAATTTATATTTAATAACTTCTGTATTAGTATTGGGTAGCATGAAATCTCTATTGAGAAATTGAACAGCATACAACTAGTAGCTGTAAATTCCTTCAGAAAGTGAAAATTATTTCTTCCTAAAGATATCTTGACATCAGTGCTTGAAGAATAGTCATAACTAGATTAATAATTGTTTTAGTTAAACAGTTTTAAGTGCCTGTTTCAGATGATGATAGGCAATTTAGATGAATTTAGGAAAAATCAAAGTTTTTACTTGCAGAAATGTCCATTATAGGGGGCCCCCCTCCTCATAGAGCTGAATGGGTTATGTAATGTTTTATCCAAAAGTTTCCAATTCCACTGTCTTGTGTTTTCATGTTGAAAATACTTTTGCATTTTTCCTTTGAGTGCCAATTTCTTACTAGTACTATTTCTTAATGTAACATGTTTACCTGGAATGTATTTTAACTATTTTTGTATAGTGTAAACTGAAACATGCACATTTTGTACATTGTGCTTTTTTTTGTGGGACATATGCAGTGTGATCCAGTTGTTTTCCATCATTTGGTTGCGCTGACCTAGGAATGTTGGTCATATCAAACATTAAATTTAAAAATGACCACTCTTTTAATTAAAATTAACTTTTAAATGTTTATAGGAGTATGTGCTGTGAAGTGATCTGAAATTTGTAATATTTTTGTCATGAACTGTACTGCTCCTAATTATTGTAATGTAATAAAAATAGTTATGGTGACTATGA

SEQ ID NO: 53 - DNA, 4876 bp, Canis lupus
gctgaaaatgactgaatataaacttgtggtagttggagctggtggcgtaggcaagagtgccttgacgatacagctaattcagaatcactttgtggatgaatatgatcctacaatagaggattcctacaggaaacaagtagtaattgatggagaaacctgtctcttggatattctcgacacagcaggtcaagaggagtacagtgcaatgagggaccagtacatgaggactggggagggctttctttgtgtatttgccataaataatactaaatcatttgaagatattcaccattatagagaacaaattaaaagagttaaagactctgaagatgtacctatggtcctagtaggaaataaatgtgatttgccttctagaacagtagacacaaaacaggctcaggacttagcaagaagttatggaattccttttattgaaacatcagcaaagacaagacagggtgttgacgatgccttctatacattagttcgagaaattcgaaaacataaagaaaagatgagcaaagatggtaaaaagaagaaaaagaagtcaaagacaaagtgtataattatgtaaatacaatttgtacttttttcttaaggcatacttaagtaaaagtggtaatttttgtacattacactaaattattagcatttgttttagcattacctaattttctgctccatccaaactgttagcttttatcttgaatgcttattttaaaatgacagtggaaactttttcctctaagtgccagtattccctgagttttggttttgaactagcaatgcctgtgaaaaagaaactgaatacctgagatttctgtcttggggtttttggtgcatgcagttgattacttcctatttttcttaccaattgtgaactttggtgtgaaacaaattaatgaagctttcgaatcatccctattctgtgttttacctagtcacatacatggattaattactaattataacttcagttgatatttcatgattggttttactgaaacattgagggaacatgaatttatgggctgcttcttataggtataatgtcctatagtttcagtcacccttaatgaatgtaaagctacactgttcacaaaggttttctccatcttttcactgctatttgtcatagccacgctcccaaaaatattatattttttctataaaaaagggaaaaaatagaaaaaaatacaaggcaatggaaaatattaaaaggcatttactttccatattagataaattcctataatactctgaatagcttttcctgttaaggcagacccagtatgtaatgaggattatagcaaccattttggggctatatttacatgctactaaatttttgtattaattgaaaaagttttaacatgtataaaaaattcccataggaattaaatatagtctccctgtgtcagattgctctttcttagcataactttaaatcttttcttgatcttcaatcttagaaaatagttttaattcttgtagtgatgttaaagattatttgggccagttagtttttaatagatgttaaagagaccacagttccaaggccaggccttgtgtgaacctttaagcttcattaagagtttcatagtacagactgcatccctgtggtctcccagggtcatcatgcattgattgggtggtcaaaagtggggacaaagagtgtttagataagatgcatcctcactgtatggtggtcctgctgacagatcaggaccatcacttttgttttttaaaaaaccaacagagctttttaaaaacattatttaaaatgagatttttgggggcagggggtggcaagacttgaattttttttaaacaatgaagtaaaaaggtttcaaaatctctagtgttggctagttctcaacattggctaaagtaacatttcataaacactttacaagtattggtccatatttaagaatatctaatgcttaaataatagattaataacaattctttcagtgcatttaaaatgtatttttaaatatctgaagtgagatggtgtgttgaggtgaaaatatcactggactaggaggaaggtgacttagattctagttacgtgtcttttacaacttcagttttgggcaaatcactcactatccatttcttcatgttaagtcatctcaaaggctatatctagcatcaactatgtgatttacattcagtttacataaggatatacctatttgtcaatctcagcacaatctgtaactttttacctatgttctcttcagcgccagtcttaggcaaagttgtgcaagaggtgaggtttatttttgagaatctgatctccggtagcaggtactcctctcccatgttagtgtcatcttgcctgcctaccttctacatgccccatgacttgatgctttctaattccccgaacctcaagatgtagtgctgctttggatatctccatgaggtaataagtcacattagtcaggctcaacataatctgacagatactgtagtgggatttgatctaatagctaattttcaggtggtaactgtatcaatttaattttgatcttttgaacatcatctctgctacctggtccattagtgactaagtaggaaaagtaggaattttcatatctgtgatgtgtagacagaccctatccagtagaagaatttaataaatttaattaataaatactgaaagatttccttagataatccaaaactaggactagccctggtaacggtgatacattccattattttaataagtaaaatcttcttacaatgaaaaatactttaaaatttaattcataaagcttactttttagcagaattcatttattcaacaaatacttgagtgcctgctagatgccaggttctacacaaggcaccggggatattatggtattcccaacaagggacataatccctatccttaagtagtactgttattttagagtggtctgtagtatattagtgaggcatttggcacatgacccagagataatataatgcatattttagttttgcacagaagggatatggtctctaaggttttttccagctctaaaataattgttcgctctgattccaataaactgtttaatcaagctactttatataaatcactttacttcattattttaaagaagtaaacttgactatattgttttttatttgggataattatgtgattctgttgggatacttatatagtacacattaaattgtatgtcagatgataacattaaaattcccaagtgtaatattctacttggtctctgtgtatcataattaaaatagatttaaatattgagttcaaaaatagttttatttatctgggtgtgaataaacagatgcctgaactaattcacagaaaaggaaacttctgtgtaaaaagtcagtccaatttctgaaatgctatgctaaactacaggtttatggaacattagatagggtgttaagactttatatagtacttcctcttgtttctatacaagagaaagaaatggccatacttcaggaattgcagtgcataactgagggatttttaggactcttgaatttttgatgtagccgggcaactttttttaggcagtggtaattatcctttattatgtgaattttgaatggtttgacaaaacgtttgtttttgtagagattttaaaaggggagcgctaatcctagaaataaatattatgtaattattacggccttaaagataaaaatccttgttgaaagttgaaaaaaattgctaaattacatagtcttagacattaacatgtttgtggaagaatgtagcagaggtatgtagtataatttgagtgaatattcccaattaggaattctaggctctagtttaactgagtcacactgcataggaatttagaacctaacttctaggttatcaaaatctttgccaccattgcacaattttgtcctaatatatagagaaactttgtgaggcatgttcagttgcggtttgcacaagttcatctcatttgtattccagtgattttttttcttctaaccatttttttaaacaacatgtacacattgttttttttggtaggcaatgaaaactgtcatttccattgtcaaacagtaattcctcgataactgtattaatggtttttaaaaaaccatcagttactttaaaactgaatttatatttaataacttctgtattagtattgggtagcatgaaatctctattgagaaattgaacagcatacaactagtagctgtaaattccttcagaaagtgaaaattatttcttcctaaagatatcttgacatcagtgcttgaagaatagtcataactagattaataattgttttagttaaacagttttaagtgcctgtttcagatgatgataggcaatttagatgaatttaggaaaaatcaaagtttttacttgcagaaatgtccattatagggggcccccctcctcatagagctgaatgggttatgtaatgttttatccaaaagtttccaattccactgtcttgtgttttcatgttgaaaatacttttgcatttttcctttgagtgccaatttcttactagtactatttcttaatgtaacatgtttacctggaatgtattttaactatttttgtatagtgtaaactgaaacatgcacattttgtacattgtgcttttttttgtgggacatatgcagtgtgatccagttgttttccatcatttggttgcgctgacctaggaatgttggtcatatcaaacattaaatttaaaaatgaccactcttttaattaaaattaacttttaaatgtttataggagtatgtgctgtgaagtgatctgaaatttgtaatatttttgtcatgaactgtactgctcctaattattgtaatgtaataaaaatagttatggtgactatga

SEQ ID NO: 54 - protein, 188 aa, Canis lupus; identical to SEQ ID NO: 50

SEQ ID NO: 55 - DNA, 1394 bp, Felis catus
gctgaaaatgactgaatataaacttgtggtagttggagctggtggcgtaggcaagagtgccttgacgatacagctaattcagaatcactttgtggatgaatatgatcctacaatagaggattcctacaggaaacaagtagtaattgatggagaaacctgtctcttggatattctcgacacagcaggtcaagaggagtacagtgcaatgagggaccagtacatgaggactggggagggctttctttgcgtatttgccataaataatactaaatcatttgaagatattcaccactatagagaacaaataaaaagagttaaagactctgaagatgtacctatggtcctagtaggaaataaatgtgatttgccttctagaacagtagatacaaaacaggctcaggacttagcaagaagttatggaattccttttattgaaacatcagcaaagacaagacagggtgttgacgatgccttctatacattagttcgagaaattcgaaaacataaagaaaagatgagcaaagatggtaaaaagaagaaaaagaagtcaaagacaaagtgtataattatgtaaatacaatttgtacttttttcttaaggcatacttaagtaaaagtggtaatttttgtacattacactaaattattagcatttgttttagcattacctaattttctgctccatccaaactgttagcttttatcttgaatgcttattttaaatgacagtggaaactttttttcctctaagtgccagtattccctgagttttggtttttgaactagcaatgcctgtgaaaaagaaactgaatacctgagatttctgtcttggggtttttggtgcatgcagttgattacttcctatttttcttaccaattgtgaactttggtgtgaaacaaattaatgaaactttcgaatcatccctattctgtgtttcatgtagtcacatacatggattaattactaattataacttcagttgagatttcatgattcgttttactgaaacattgagggaacatgaatttatgggcttcttgtagattcatcttgtaggtattaatgtcctatagtttcagtcacccttaatgaatgtaaagttacactgttcataaaagtttctccatcttttcactgctgtttgtcatcgtcacgctcccccaaaatattatattttttctataaaaagggaaaaaaggaaaaaaatacaaggcaatggaaaatattaaaaggcatttactttctgtattagataaattcctataatactctgaatagcttttcctgttaaggcagacccagtatgtgatgaggattatagcaaccattttggggctatatttacatgctactaaatttttgtaataattgaaaaaattttaacatgtataaaa

SEQ ID NO: 56 - protein, 188 aa, Felis catus; identical to SEQ ID NO: 50

SEQ ID NO: 57 - DNA, 1512 bp, Felis catus
tgctgaaaatgactgaatataaacttgtggtagttggagctggtggcgtaggcaagagtgccttgacgatacagctaattcagaatcactttgtggatgaatatgatcctacaatagaggattcctacaggaaacaagtagtaattgatggagaaacctgtctcttggatattctcgacacagcaggtcaagaggagtacagtgcaatgagggaccagtacatgaggactggggagggctttctttgcgtatttgccataaataatactaaatcatttgaagatattcaccactatagagaacaaataaaaagagttaaagactctgaagatgtacctatggtcctagtaggaaataaatgtgatttgccttctagaacagtagatacaaaacaggctcaggacttagcaagaagttatggaattccttttattgaaacatcagcaaagacaagacagagagtggaggatgctttttatacattggtgagagagatccgacagtacagattgaaaaaaatcaacaaagaagaaaagactcctggctgtgtgaaaattaaaaaatgcattgtaatgggtgttgacgatgccttctatacattagttcgagaaattcgaaaacataaagaaaagatgagcaaagatggtaaaaagaagaaaaagaagtcaaagacaaagtgtataattatgtaaatacaatttgtacttttttcttaaggcatacttaagtaaaagtggtaatttttgtacattacactaaattattagcatttgttttagcattacctaattttctgctccatccaaactgttagcttttatcttgaatgcttattttaaatgacagtggaaactttttttcctctaagtgccagtattccctgagttttggtttttgaactagcaatgcctgtgaaaaagaaactgaatacctgagatttctgtcttggggtttttggtgcatgcagttgattacttcctatttttcttaccaattgtgaactttggtgtgaaacaaattaatgaaactttcgaatcatccctattctgtgtttcatgtagtcacatacatggattaattactaattataacttcagttgagatttcatgattcgttttactgaaacattgagggaacatgaatttatgggcttcttgtagattcatcttgtaggtattaatgtcctatagtttcagtcacccttaatgaatgtaaagttacactgttcataaaagtttctccatcttttcactgctgtttgtcatcgtcacgctcccccaaaatattatattttttctataaaaagggaaaaaaggaaaaaaatacaaggcaatggaaaatattaaaaggcatttactttctgtattagataaattcctataatactctgaatagcttttcctgttaaggcagacccagtatgtgatgaggattatagcaaccattttggggctatatttacatgctactaaatttttgtaataattgaaaaaattttaacatgtataaaa

SEQ ID NO: 58 - protein, 227 aa, Felis catus
MTEYKLVVVGAGGVGKSALTIQLIQNHFVDEYDPTIEDSYRKQVVIDGETCLLDILDTAGQEEYSAMRDQYMRTGEGFLCVFAINNTKSFEDIHHYREQIKRVKDSEDVPMVLVGNKCDLPSRTVDTKQAQDLARSYGIPFIETSAKTRQRVEDAFYTLVREIRQYRLKKINKEEKTPGCVKIKKCIVMGVDDAFYTLVREIRKHKEKMSKDGKKKKKKSKTKCIIM

SEQ ID NO: 59 - DNA, 2144 bp, Bos taurus
ggcggtggcggcggcggcggcggtggcggtggcggttcggccagtactcccggcccccgccatttctgactgggagcgagcgcggcgcaggcactgaaggcagcggcgggggccagaggctcggcggctcccaggtgagggagagaggcctgctgaaaatgactgaatataaacttgtggtagttggagctggtggcgtaggcaagagtgccttgacgatacagctaattcagaatcactttgtggatgaatatgatcctacgatagaggattcctacaggaaacaagtagtaattgatggagaaacctgtctcttggatattctcgacacagcaggtcaagaggagtacagtgcaatgagggaccagtacatgaggactggggagggctttctttgtgtatttgccataaataatactaaatcatttgaagatattcaccattatagagaacaaataaaaagagttaaagactctgaagatgtacctatggttctagtaggaaataaatgtgatttgccttctagaacagtagacacaaaacaggctcaggacttagcaagaagttatggaattccttttattgaaacatcagcaaagacaagacagggtgttgacgatgccttctatacattagttcgagaaattcgaaaacataaagaaaagatgagcaaagatggtaaaaagaagaaaaagaagtcaaagacaaagtgtataattatgtaaatacaatttgtacttttttcttaaggcatacttaagtaaaagtggtaatttttgtatattacactaaattattagcatttgttttagcattatctaattttctttctgctccatccatactgttagcttttatcttgaatgcttattttaaaatgacagtggaaacttttttcctctaagtgccagtattccctgcgttttggtttttgaactagcaatgcctgtgaaaaagaaactgaacacccaagatttttgtcttggggtttttggtgcatgcagttgattacttcctatttttcttatcaattgtgaactttagtgtgaaacaaattaatgaggctttcaaatcatccctattgtattgttttatctagtcacacacatggattaattactaattataacttcagttgagatttcatgattggttttactgaaacatcgagggaacatgaatttatgggcttcctatagtttcatcttgtaggtatcattgtcctatagtttcagttacccttaatgaatgtcaggttacactgttcacaaaggttttcttctttccactgctatttgtcaaatggtcacgttccctaaaatactatattttttctataaaaaaaagaaaaaaatggaaaaaaatacaaggcaatggaaaatattaaaaggccacttactttccacattaggtaaattcctataatgctctgaatagctttttatgttaaggcagacccagtaggtaatgaggattagaacaagcattttgggactatatttacatgctttaaatttttgtaataacaaaaaaattttaacatgtataaagaattctcataggaattaaatacagtctccctgtgtcagattgctctttcttagcataaatctttttcttgaacttcaatctttaaaagtagttttaattctactgatagtgatgtaaaagattatttgggccagttagcttggtaggtgttacagagaccagggtggcatagccgggccttgtgtgaacctttaagctacatggagagtttcacagtgtggactgcatccctgtggtcttccattgttgccatgccttggttggtcaaaaacaaggacttgcagagagattgaatagctcagcaaggtacattctcattatgtcgtagtcctactcaggaacatcacttttttaaaataaaaaaccccaaaaaacagaacttaaaaaaaaaaacaacattattttaaatgagattttcggtggggtggaaagattttaattttttttaaacgatgaaatgaaaaaatgtcaaaatcttgagtattggctagttctctttaacactggctaaagtaacatttttgtaaacacttcagtacagtctggtccattattaagaatatctaatgcttatacaataaagtaatgctaac

SEQ ID NO: 60 - protein, 188 aa, Bos taurus; identical to SEQ ID NO: 50

SEQ ID NO: 61 - DNA, 1010 bp, Bos taurus
ggcggtggcggcggcggcggcggtggcggtggcggttcggccagtactcccggcccccgccatttctgactgggagcgagcgcggcgcaggcactgaaggcagcggcgggggccagaggctcggcggctcccaggtgagggagagaggcctgctgaaaatgactgaatataaacttgtggtagttggagctggtggcgtaggcaagagtgccttgacgatacagctaattcagaatcactttgtggatgaatatgatcctacgatagaggattcctacaggaaacaagtagtaattgatggagaaacctgtctcttggatattctcgacacagcaggtcaagaggagtacagtgcaatgagggaccagtacatgaggactggggagggctttctttgtgtatttgccataaataatactaaatcatttgaagatattcaccattatagagaacaaataaaaagagttaaagactctgaagatgtacctatggttctagtaggaaataaatgtgatttgccttctagaacagtagacacaaaacaggctcaggacttagcaagaagttatggaattccttttattgaaacatcagcaaagacaagacagagagtggaggatgctttttatacattggtgagagagatccgacaatacagattgaaaaaaatcagcaaagaagaaaagactcctggctgtgtgaaaattaaaaaatgcattgtaatgggtgttgacgatgccttctatacattagttcgagaaattcgaaaacataaagaaaagatgagcaaagatggtaaaaagaagaaaaagaagtcaaagacaaagtgtataattatgtaaatacaatttgtacttttttcttaaggcatacttaagtaaaagtggtaatttttgtatattacactaaattattagcatttgttttagcattatctaattttctttctgctccatccatactgttagcttttatcttgaatgcttattttaaaatgacagtggaaactt

SEQ ID NO: 62 - protein, 227 aa, Bos taurus
MTEYKLVVVGAGGVGKSALTIQLIQNHFVDEYDPTIEDSYRKQVVIDGETCLLDILDTAGQEEYSAMRDQYMRTGEGFLCVFAINNTKSFEDIHHYREQIKRVKDSEDVPMVLVGNKCDLPSRTVDTKQAQDLARSYGIPFIETSAKTRQRVEDAFYTLVREIRQYRLKKISKEEKTPGCVKIKKCIVMGVDDAFYTLVREIRKHKEKMSKDGKKKKKKSKTKCIIM

SEQ ID NO: 63 - DNA, 797 bp, Bos taurus
gcggtggcggcggcggcggcggtggcggtggcggttcggccagtactcccggcccccgccatttctgactgggagcgagcgcggcgcaggcactgaaggcagcggcgggggccagaggctcggcggctcccaggtgagggagagaggcctgctgaaaatgactgaatataaacttgtggtagttggagctggtggcgtaggcaagagtgccttgacgatacagctaattcagaatcactttgtggatgaatatgatcctacgatagaggattcctacaggaaacaagtagtaattgatggagaaacctgtctcttggatattctcgacacagcaggtcaagaggagtacagtgcaatgagggaccagtacatgaggactggggagggctttctttgtgtatttgccataaataatactaaatcatttgaagatattcaccattatagagaacaaataaaaagagttaaagactctgaagatgtacctatggttctagtaggaaataaatgtgatttgccttctagaacagtagacacaaaacaggctcaggacttagcaagaagttatggaattccttttattgaaacatcagcaaagacaagacagagagtggaggatgctttttatacattggtgagagagatccgacaatacagattgaaaaaaatcagcaaagaagaaaagactcctggctgtgtgaaaattaaaaaatgcattgtaatgtaatctgggtgttgacgatgccttctatacattagttcgagaaattcgaaaacataaagaaaagatgagcaaa

SEQ ID NO: 64 - protein, 189 aa, Bos taurus
MTEYKLVVVGAGGVGKSALTIQLIQNHFVDEYDPTIEDSYRKQVVIDGETCLLDILDTAGQEEYSAMRDQYMRTGEGFLCVFAINNTKSFEDIHHYREQIKRVKDSEDVPMVLVGNKCDLPSRTVDTKQAQDLARSYGIPFIETSAKTRQRVEDAFYTLVREIRQYRLKKISKEEKTPGCVKIKKCIVM

SEQ ID NO: 65 - DNA, 1112 bp, Gallus gallus
caggtctgctaaaaaatgacagagtataagcttgttgtcgttggagctggtggtgtgggcaagagcgccttgacaatacagctcattcagaaccactttgtggatgagtatgaccctaccatagaggattcctacagaaagcaagtagtaattgatggggaaacctgtctcttggatattcttgatacagcaggtcaagaagaatatagtgcaatgagggaccaatatatgagaacaggagaaggctttctgtgtgtttttgctataaacaatacaaaatcttttgaagatattcaccattatagggaacaaataaagagagttaaagactctgaagatgtcccaatggtgctagtaggaaacaaatgtgatttgccttccagaacagtagatacaaaacaagctcaggatttagcaagaagttatggaattccttttattgaaacatcagcaaagacaagacagggtgttgatgatgccttctatacattagttcgagaaatcagaaaacacaaagagaagatgagcaaagatggtaaaaagaagaaaaagaagacaaagacaaagtgtataattatgtaaatacaatgtatccttattcttaagacgtactgaagtaatttttgtacattacactaaattattagcatttgtttttagcattactttactttctgcttcatgatcctgttagctttacctgaatgcttgttttaaatgacagtggaaacttcattcctcttaaagtgccagtattctttgagtgttggttcttgaactagcaatgcctgtgaagaaaaataaaaacaaatgaaaaaaaaaaaaacacacaaaaacctgagaactgtcttaggactctttggtgcatgcacagttgctaacttcctatttttcttactgattgtgaacttctgttccgtgcgtaaacaaaacaatgaaacgatctacacgttctaacatcccccttcatttgtactctcttattttttacatctggttgggaaaacggaccagttagtgacaaagactttattttcagacttccttctaatttcgactgactgcaatatagagagaccagaagcctttatagtcttcctgtagattttgct

SEQ ID NO: 66 - protein, 188 aa, Gallus gallus
MTEYKLVVVGAGGVGKSALTIQLIQNHFVDEYDPTIEDSYRKQVVIDGETCLLDILDTAGQEEYSAMRDQYMRTGEGFLCVFAINNTKSFEDIHHYREQIKRVKDSEDVPMVLVGNKCDLPSRTVDTKQAQDLARSYGIPFIETSAKTRQGVDDAFYTLVREIRKHKEKMSKDGKKKKKKTKTKCIIM

SEQ ID NO: 67 - DNA, 4454 bp, Homo sapiens
gaaacgtcccgtgtgggaggggcgggtctgggtgcggcctgccgcatgactcgtggttcggaggcccacgtggccggggcggggactcaggcgcctggggcgccgactgattacgtagcgggcggggccggaagtgccgctccttggtgggggctgttcatggcggttccggggtctccaacatttttcccggctgtggtcctaaatctgtccaaagcagaggcagtggagcttgaggttcttgctggtgtgaaatgactgagtacaaactggtggtggttggagcaggtggtgttgggaaaagcgcactgacaatccagctaatccagaaccactttgtagatgaatatgatcccaccatagaggattcttacagaaaacaagtggttatagatggtgaaacctgtttgttggacatactggatacagctggacaagaagagtacagtgccatgagagaccaatacatgaggacaggcgaaggcttcctctgtgtatttgccatcaataatagcaagtcatttgcggatattaacctctacagggagcagattaagcgagtaaaagactcggatgatgtacctatggtgctagtgggaaacaagtgtgatttgccaacaaggacagttgatacaaaacaagcccacgaactggccaagagttacgggattccattcattgaaacctcagccaagaccagacagggtgttgaagatgctttttacacactggtaagagaaatacgccagtaccgaatgaaaaaactcaacagcagtgatgatgggactcagggttgtatgggattgccatgtgtggtgatgtaacaagatacttttaaagttttgtcagaaaagagccactttcaagctgcactgacaccctggtcctgacttccctggaggagaagtattcctgttgctgtcttcagtctcacagagaagctcctgctacttccccagctctcagtagtttagtacaataatctctatttgagaagttctcagaataactacctcctcacttggctgtctgaccagagaatgcacctcttgttactccctgttatttttctgccctgggttcttccacagcacaaacacacctctgccaccccaggtttttcatctgaaaagcagttcatgtctgaaacagagaaccaaaccgcaaacgtgaaattctattgaaaacagtgtcttgagctctaaagtagcaactgctggtgattttttttttctttttactgttgaacttagaactatgctaatttttggagaaatgtcataaattactgttttgccaagaatatagttattattgctgtttggtttgtttataatgttatcggctctattctctaaactggcatctgctctagattcataaatacaaaaatgaatactgaattttgagtctatcctagtcttcacaactttgacgtaattaaatccaactttcacagtgaagtgcctttttcctagaagtggtttgtagacttcctttataatatttcagtggaatagatgtctcaaaaatccttatgcatgaaatgaatgtctgagatacgtctgtgacttatctaccattgaaggaaagctatatctatttgagagcagatgccattttgtacatgtatgaaattggttttccagaggcctgttttggggctttcccaggagaaagatgaaactgaaagcacatgaataatttcacttaataatttttacctaatctccacttttttcataggttactacctatacaatgtatgtaatttgtttcccctagcttactgataaacctaatattcaatgaacttccatttgtattcaaatttgtgtcataccagaaagctctacatttgcagatgttcaaatattgtaaaactttggtgcattgttatttaatagctgtgatcagtgattttcaaacctcaaatatagtatattaacaaattacattttcactgtatatcatggtatcttaatgatgtatataattgccttcaatccccttctcaccccaccctctacagcttcccccacagcaataggggcttgattatttcagttgagtaaagcatggtgctaatggaccagggtcacagtttcaaaacttgaacaatccagttagcatcacagagaaagaaattcttctgcatttgctcattgcaccagtaactccagctagtaattttgctaggtagctgcagttagccctgcaaggaaagaagaggtcagttagcacaaaccctttaccatgactggaaaactcagtatcacgtatttaaacatttttttttcttttagccatgtagaaactctaaattaagccaatattctcatttgagaatgaggatgtctcagctgagaaacgttttaaattctctttattcataatgttctttgaagggtttaaaacaagatgttgataaatctaagctgatgagtttgctcaaaacaggaagttgaaattgttgagacaggaatggaaaatataattaattgatacctatgaggatttggaggcttggcattttaatttgcagataataccctggtaattctcatgaaaaatagacttggataacttttgataaaagactaattccaaaatggccactttgttcctgtctttaatatctaaatacttactgaggtcctccatcttctatattatgaattttcatttattaagcaaatgtcatattaccttgaaattcagaagagaagaaacatatactgtgtccagagtataatgaacctgcagagttgtgcttcttactgctaattctgggagctttcacagtactgtcatcatttgtaaatggaaattctgcttttctgtttctgctccttctggagcagtgctactctgtaattttcctgaggcttatcacctcagtcatttcttttttaaatgtctgtgactggcagtgattctttttcttaaaaatctattaaatttgatgtcaaattagggagaaagatagttactcatcttgggctcttgtgccaatagcccttgtatgtatgtacttagagttttccaagtatgttctaagcacagaagtttctaaatggggccaaaattcagacttgagtatgttctttgaataccttaagaagttacaattagccgggcatggtggcccgtgcctgtagtcccagctacttgagaggctgaggcaggagaatcacttcaacccaggaggtggaggttacagtgagcagagatcgtgccactgcactccagcctgggtgacaagagagacttgtctccaaaaaaaaagttacacctaggtgtgaattttggcacaaaggagtgacaaacttatagttaaaagctgaataacttcagtgtggtataaaacgtggtttttaggctatgtttgtgattgctgaaaagaattctagtttacctcaaaatccttctctttccccaaattaagtgcctggccagctgtcataaattacatattccttttggtttttttaaaggttacatgttcaagagtgaaaataagatgttctgtctgaaggctaccatgccggatctgtaaatgaacctgttaaatgctgtatttgctccaacggcttactatagaatgttacttaatacaatatcatacttattacaatttttactataggagtgtaataggtaaaattaatctctattttagtgggcccatgtttagtctttcaccatcctttaaactgctgtgaatttttttgtcatgacttgaaagcaaggatagagaaacactttagagatatgtggggtttttttaccattccagagcttgtgagcataatcatatttgctttatatttatagtcatgaactcctaagttggcagctacaaccaagaaccaaaaaatggtgcgttctgcttcttgtaattcatctctgctaataaattataagaagcaaggaaaattagggaaaatattttatttggatggtttctataaacaagggactataattcttgtacattatttttcatctttgctgtttctttgagcagtctaatgtgccacacaattatctaaggtatttgttttctataagaattgttttaaaagtattcttgttaccagagtagttgtattatatttcaaaacgtaagatgatttttaaaagcctgagtactgacctaagatggaattgtatgaactctgctctggagggaggggaggatgtccgtggaagttgtaagacttttatttttttgtgccatcaaatataggtaaaaataattgtgcaattctgctgtttaaacaggaactattggcctccttggccctaaatggaagggccgatattttaagttgattattttattgtaaattaatccaacctagttctttttaatttggttgaatgttttttcttgttaaatgatgtttaaaaaataaaaactggaagttcttggcttagtcataattctt

SEQ ID NO: 68 - protein, 189 aa, Homo sapiens
MTEYKLVVVGAGGVGKSALTIQLIQNHFVDEYDPTIEDSYRKQVVIDGETCLLDILDTAGQEEYSAMRDQYMRTGEGFLCVFAINNSKSFADINLYREQIKRVKDSDDVPMVLVGNKCDLPTRTVDTKQAHELAKSYGIPFIETSAKTRQGVEDAFYTLVREIRQYRMKKLNSSDDGTQGCMGLPCVVM

SEQ ID NO: 69 - DNA, 1326 bp, Rattus norvegicus
gccgttcatggcggtttcggggtctccaacagcttctcaggttgaaatccaaaagcctcccgaggcggggtctgcggagtttgagatttttgcaggtgtgaaatgactgagtacaaactggtggtggttggagcaggtggcgttgggaaaagtgctttgacaatccagctaatccagaaccactttgtggatgaatatgatcccaccatagaggattcttaccgaaaacaagtggtgattgacggtgagacctgtctactggacatactggacacagctggacaagaggagtacagtgccatgagagaccaatacatgaggacaggcgaagggttcctctgtgtgtttgccatcaataatagcaaatcctttgcagatattaacctctacagggagcaaattaagcgcgtgaaagactctgatgatgtacccatggtgctggtagggaacaagtgtgacttgccaacaaggacagttgacacaaagcaagcccacgagctggccaagagttatggaattccattcattgaaacctcagccaagacccgacagggtgtggaggatgccttttacacgcttgtaagggagatacgccagtaccggatgaagaagctcaacagcagtgaggatggcactcaaggctgtatggggctgccctgtgtggtgatgtagtaagaccctttaaaagttctgtcatcagaaacgagccactttcaagcctcactgatgccctggttctgacatccctggaggagacgtgtttctgctgctctctgcatctcagagaagctcctgcttcctgcttccccaacttagttactgagcacagccatctaacctgagacctcttcagaataactacctcctcactcggctgtccgaccagagaaatgaacctgtttctccccagtagttctctgccctgggtttcccctagaaacaaacacacctgccagctggctttgtcctccgaaaagcagtttacattgatgcagagaaccaaactatagacaagcaattctgttgtcaacagtttcttaagctctaaggtaacaattgctggtgatttccccctttgcccccaactgttgaacttggccttgttagttttgggggaaatgtcaaaaattaatctcttcccgagaatagaattagtgttgctgattgcctgatttgcaatgtgatcagctatattctataagctggcgtctgctctgtattcataaatgcaaacatgagtactgacgtaagtgcatccctagtcttctcagctgcatgcaattaaatccaacgttcacaacaaaaaaaaaaaaaaaaaaaaaaaaa

SEQ ID NO: 70 - protein, 189 aa, Rattus norvegicus
MTEYKLVVVGAGGVGKSALTIQLIQNHFVDEYDPTIEDSYRKQVVIDGETCLLDILDTAGQEEYSAMRDQYMRTGEGFLCVFAINNSKSFADINLYREQIKRVKDSDDVPMVLVGNKCDLPTRTVDTKQAHELAKSYGIPFIETSAKTRQGVEDAFYTLVREIRQYRMKKLNSSEDGTQGCMGLPCVVM

SEQ ID NO: 71 - DNA, 4470 bp, Mus musculus
gggactggggcgccttgggcgcctagtgattacgtagcgggtggggccggaagtgccgctccctggcgggggctgttcatggcggtttcggggtctccaacagcttctcaggttgaagtccaaaagcctcccgaggcggggtctgcggagtttgaggtttttgctggtgtgaaatgactgagtacaaactggtggtggttggagcaggtggtgttgggaaaagcgccttgacgatccagctaatccagaaccactttgtggatgaatatgatcccaccatagaggattcttaccgaaagcaagtggtgattgatggtgagacctgcctgctggacatactggacacagctggacaagaggagtacagtgccatgagagaccagtacatgaggacaggcgaagggttcctctgtgtatttgccatcaataatagcaaatcatttgcagatattaacctctacagggagcaaattaagcgtgtgaaagattctgatgatgtccccatggtgctggtaggcaacaagtgtgacttgccaacaaggacagttgacacaaagcaagcccacgaactggccaagagttacggaattccattcattgagacctcagccaagacccgacagggtgtggaggatgccttttacacactggtaagggagatacgccagtaccgaatgaaaaagctcaacagcagtgacgatggcactcaaggttgtatggggctgccctgtgtgctgatgtagtaagacactttgaaagttctgtcatcagaaaagagccactttgaagctgcactgatgccctggttctgacatccctggaggagacctgttcctgctgctctctgcatctcagagaagctcctgcttcctgcttccccgactcagttactgagcacagccatctaacctgagacctcttcagaataactacctcctcactcggctgtctgaccagagaaatagacctgtctctcccggtcgttctctgccctgggttcccctagaaacagacacagcctccagctggctttgtcctctgaaaagcagtttacattgatgcagagaaccaaactagacatgccattctgttgacaacagtttcttatactctaaggtaacaactgctggtgattttcccctgcccccaactgttgaacttggccttgttggtttggggggaaaatgtcataaattactttcttcccaaaatataattagtgttgctgattgatttgtaatgtgatcagctatattccataaactggcatctgctctgtattcataaatgcaaacacgaatactctcaactgcatgcaattaaatccaacattcacaacaaagtgcctttttcctaaaagtgctctgtaggctccattacagtttgtaattggaatagatgtgtcaagaaccattgtataggaaagtgactctgagccatctacctttgagggaaaggtgtatgtacctgatggcagatgctttgtgtatgcacatgaagatagtttccctgtctgggattctcccaggagaaagatggaactgaaacaattacaagtaatttcatttaattctagctaatcttttttttttttttttttttttttggtagactatcacctataaatatttggaatatcttctagcttactgataatctaataattaatgagcttccattataatgaattggttcataccaggaagccctccatttatagtatagatactgtaaaaattggcatgttgttactttatagctgtgattaatgattcctcagaccttgctgagatatagttattagcagacaggttatatctttgctgcatagtttcttcatggaatatatatctatctgtatgtggagagaacgtggccctcagttcccttctcagcatccctcatctctcagcctagagaagttcgagcatcctagaggggcttgaacagttatctcggttaaaccatggtgctaatggaccgggtcatggtttcaaaacttgaacaagccagttagcatcacagagaaacagtccatccatatttgctccctgcctattattcctgcttacagacttttgcctgatgcctgctgttagtgctacaaggataaagcttgtgtggttctcaccaggactggaagtacctggtgagctctggggtaagcctagatatctttacattttcagacccttattcttagccacgtggaaactgaagccagagtccatacctccatctccttccccccccaaaaaaattagattaatgttctttatatagcttttttaaagtatttaaaacatgtctataagttaggctgccaactaacaaaagctgatgtgtttgttcaaataaagaggtatccttcgctactcgagagaagaatgtaaaatgccattgattgttgtcacttggaggcttgatgtttgccctgataattcattagtgggttttgtttgtcacatgatacctaagatgtaactcagctcagtaattctaatgaaaacataaattggataccttaattgaaaaaagcaaacctaattccaaaatggccattttctcttctgatcttgtaatacctaaaattctgaggtccttgggattcttttgtttataacaggatcttgctgtgtagtcctagctggcctcaaactcacaatactcttcctggatcaatctcccaagtgctgggattacaggcacattccaccacacacacctgactgagctcgttcctaatgagttttcattaagcaaattccccatcaccttgaaactaatcagaagggggaagaaacatttgctatgctcctgagtgctaacactgggatcattcacatggggtttgcattcctaggcaaactaaactgctgccttttacaacaaggctcagtcatcttcctgaagctgctgagaccagcacttggtcttgttttgttttaatatgtctatatgactggtggtggatccctaaatagtttattaattaaactccagttaaggagaaagttactcaccttgacccgtttgaccatatcccgtgtgtgtgtgtgtgtgtgtgtgtgtgtgtgtgtgtgtgtgtgtgtgcacgcgtatgtacgtacgtatgtatgtaggtatgtaggtggtttccagtataaacacagaaacaaatggagccaattcaggtttcagatgcccttactaacatatattcccacggggtgtgggttttggcacaacagtgacaaacttaaaagccaagtaagagccgggcgtggtggcgcacgcctttaatcccagcacttgggaggcagaggcaggcggatttctgagttctaggccatcctggtctacagtgagttccaggacagccagtgctacacagagaaaccctgtctcgaaaagccaaaaaaaaaaaaaaaaaaaaaaaaaaaaagccaagtaggtccagttggtatagtatcaaagtgtttttagagtaattagtgaaggtctgctttacctcaaagttgcagagcctctcttcctgagtttaagtgcctggccggcagtcacaaattaacatgttgctgtaaggcagttagttgaagctttgttcacacattggagagtatgaaaataaagtgttctaagagcgctgatactggatctgtgtaaacctggtaaatgccgtttgtccaggacttagcgtgtgtgagttggtagctcagtacgagtttactagttccgcagtgtgtacaatggaggcgggtttgttttagctggccacctgtagaatcagcctttaaactgctgtgaactttgtcatgacttgaatatgaagatagacaaaaactctgtaaagacaaatgtttgttttcccccttacagaacgtgtgagcttggttttatcttcctttgtatttagtcataacctctcaagctggcagctccgaccaaggatcagaagctgtgtgcgttccacctggtggaattagctcagctctatatgagaagtggagttaatggaaaacgtgttgactgggtggtttctatttaaaagagtgatgataattcttgaacagtagtttttattttgctatttctttaagctgactgatgtgccacaaaattattttaaggtatttgtgttttaagagtgttctcatgagattagttgtagatattttttaaaatacaactggtttttaaaatctgagtattgctctaagcaagtgtttagactcttacgggaaggtgggtggaagttgtttggcttccgtatttccatgcgtgccgtcagacataggtcagaacgccaactgtgcatcctgctgtttaaagacctcttggcctctgtgaccctcatgaaggggctgatattttaagttgactgtttgattgtaaattaatcctttctaatttttaaagacttgcttgactgttttccttgttaaataattttaaaaaaataaaaaactggaagttctttgcttaactgta

SEQ ID NO: 72 - protein, 189 aa, Mus musculus
MTEYKLVVVGAGGVGKSALTIQLIQNHFVDEYDPTIEDSYRKQVVIDGETCLLDILDTAGQEEYSAMRDQYMRTGEGFLCVFAINNSKSFADINLYREQIKRVKDSDDVPMVLVGNKCDLPTRTVDTKQAHELAKSYGIPFIETSAKTRQGVEDAFYTLVREIRQYRMKKLNSSDDGTQGCMGLPCVLM

SEQ ID NO: 73 - DNA, 570 bp, Cavia porcellus
atgactgagtataaactggtggtggttggagcaggtggtgtcgggaaaagtgcactgaccatccagctaattcagaaccactttgtcgatgaatatgatcccaccatagaggattcttaccgaaaacaggtggttatagatggtgaaacttgtctgttggatattctggatacagctggacaagaggagtacagtgccatgagagaccaatacatgaggacaggcgaaggcttcctctgtgtgtttgccatcaataatagcaaatcatttgcagatattaacctctacagggagcagattaaacgagtaaaagactcagatgatgtacctatggtgctggtagggaacaagtgtgatttgccaacaaggactgttgacacaaaacaagcccatgaactggccaagagttacgggattccattcattgaaacctcagccaagaccagacagggtgttgaagatgcattttacacactcgtaagagaaatacgccagtacagaatgaaaaaactcaacagcaatgatgatgggactcaaggttgtatggggttgccatgtgtggtgatgtaa

SEQ ID NO: 74 - protein, 189 aa, Cavia porcellus
MTEYKLVVVGAGGVGKSALTIQLIQNHFVDEYDPTIEDSYRKQVVIDGETCLLDILDTAGQEEYSAMRDQYMRTGEGFLCVFAINNSKSFADINLYREQIKRVKDSDDVPMVLVGNKCDLPTRTVDTKQAHELAKSYGIPFIETSAKTRQGVEDAFYTLVREIRQYRMKKLNSNDDGTQGCMGLPCVVM

SEQ ID NO: 75 - DNA, 1220 bp, Cavia porcellus
gttccggggtcctcaacgtttctcagggttgagattctatatccttttgaagctggggcggcagagcttgaggttcttgctggtgtgaaatgactgagtataaactggtggtggttggagcaggtggtgtcgggaaaagtgcactgaccatccagctaattcagaaccactttgtcgatgaatatgatcccaccatagaggattcttaccgaaaacaggtggttatagatggtgaaacttgtctgttggatattctggatacagctggacaagaggagtacagtgccatgagagaccaatacatgaggacaggcgaaggcttcctctgtgtgtttgccatcaataatagcaaatcatttgcagatattaacctctacagggagcagattaaacgagtaaaagactcagatgatgtacctatggtgctggtagggaacaagtgtgatttgccaacaaggactgttgacacaaaacaagcccatgaactggccaagagttacgggattccattcattgaaacctcagccaagaccagacagggtgttgaagatgcattttacacactcgtaagagaaatacgccagtacagaatgaaaaaactcaacagcaatgatgatgggactcaaggttgtatggggttgccatgtgtggtgatgtaacaagatatttaacaaagttctatcagaaaagagccactttcaagctgcactgataccctggtcctgacttccctggaggagaagtatccctgttgctctcttcatctcagagaagctcctgctgtttgtccacctctcagtgtatgagcacagtctctgcttgagaacttctcagaataactacctcctcacttggttgtctgaccagagaaatgcacctcttgttaattccccaataattttctgccctgggctctccccaacaaaaaacaaacacttctgccatccaaaaagcaacttggtctgaaacagaaccaaactgtagattgaaattctcttaaaaagtcttgagctctaaagttagcaaccgctggtgatttttattttcctttttatttttgaacttggaactgacctatgttagattttggagaaatgtcataaagtactgttgtgccaagaagataattatgttgctgaatggttgatttatagtgttatcagctatattttacaaactggcatctgctctgtattcataaatacaaaaatgaagccagg

SEQ ID NO: 76 - protein, 189 aa, Cavia porcellus; identical to SEQ ID NO: 74

SEQ ID NO: 77 - DNA, 1307 bp, Canis lupus
tgattacgtagcgggcggggccggaagtgccgctccctagtgggggctgttcatggcggttccggggtctccaacctttctcctagttgtggtcctaaatacgtcggaagcggaggcggcgaagcttgaggttcttgctggtgtgaaatgactgagtacaaactggtggtggttggagcaggtggtgttgggaaaagcgcactgacaatccagctaatccagaaccactttgtagatgaatatgatcccaccatagaggattcttaccgaaaacaggtggttatagacggtgaaacctgtctgttggatatactggatacagctggtcaagaagagtacagtgccatgagagaccaatacatgaggacaggcgaaggcttcctctgtgtatttgccatcaataatagcaaatcatttgcagacattaacctctacagggaacagattaagcgagtaaaagattcagatgatgtacctatggtgctagtaggaaacaagtgtgatttgccaacaaggacagttgacacaaaacaagcccatgaactggccaagagttatgggattccattcattgaaacctcagccaagaccagacagggtgtcgaggatgccttttacacactggtaagagaaatacgtcagtaccgaatgaagaaactcaacagcagtgatgatgggactcaaggttgtatggggttaccatgtgtggtgatgtaacaagacacttttaaagttctagcatcagaaaagagccactgtcaagctgcactgacaccctggtcctgacttccctggaggagaagtattcctgttgctatcttcagtctcacaaagaagctcctgctacttccccaactctcagtagatcagtacaatgttctctatttgagaagttctccgaacaactacctcctcacttggttgtctgaccagagaaatgaacctcttgttccttcccgctgtttttccaccctgaattctcccccaacacacataaacaaacctctgccatcccaggtttttcatctgaaaaataattcatgctctgaaacagagaacaaaactgtagacatgaaattctgtaggaaacaaggtcttgagctcaaaagtagcaactgctggtgacctttttttcccccctttttactgttgaacttggaactatgttggtttttggagaaatgtcataagttactgttttgctgagaatatagttaagttgacatttggtttgtttgtaatatcattagctattttctataaattggcatctgctctgcattcataaatacacgagtgaattctga

SEQ ID NO: 78 - protein, 189 aa, Canis lupus; identical to SEQ ID NO: 68

SEQ ID NO: 79 - DNA, 3104 bp, Felis catus
aaaaaataaataaatttaagaaaccattttaaaattatgcacagttgcagcctggaaaacttaaggtggcgccttatagtatcaatcttaggagctttatttggtgcatttaacgcaactggtaattgcaaaatccacttcgcctgtgtaagtgaaaaatatagactgttatcttgttggccctatgaaattctgcacttggtatttagcatatactctaccttcattactatctggcaagatgttctgccttagcactcagttgcattcttttccttttctttcctgttcattatgctttaattctgaggaccatatgagggtagaatatattaaaaattacaaaaattataaaaatttgtataggcaaaccatttccttaagttgatggccaaatgttaaaatgttatttttcatatcatttataatcttgtcacagtccacttaacgaagtttggttagatttcagtgaaaattatcttccagagtagtttttttttttttttcctgggattagggaggggggtaactttactgcaattagtatgtatggtgcagaatttcatgcaaatgaggtgtgccagcagtgtggtaatttaatcgtatttaaacaaaaacaaacaaaaaaaaaacgaatgcacaaacttgctgctgcttagatcactgcagcttctaggacccagtttcttttactgatttcaaaacaaaacaaaacaaaaaaataaaaaaagttgtgcctgaaatgaatcttgttttttttataagtagccgcctggttcctgtgtcctgtgaaatacaggcacttgacccttggtgtagcttctgttcgactttatatcacgggaatggattggtctgatttcttggccctcatcttgaattggccacatccagggtccctggccagtggactgaaggctttgtctaagaggacaagggcagctcaggggatgtgggggagggcgcttttatcttccccgttgtcgtttgaggttttgatcttctctgggtaaagaggccgtttatctttgtaaacacaaaacatttttgctttctccagttttctgttaatggcgaaagaatggaagcgaataaagttttactgatttttgagactctagcacctagcgctttcatttttgaaacgtcctgtgtgggaggggcgggtctgggtgcggcccgccgcgtgactcctgagtcgggggcccacgtggctggggcggggactcggacgccccgggcgccgactgattacgtagcgggcggggccggaagtgccgctccctagtgggggctgttcatggcggttccggggtctccatcctttttcccagttgttctaaatcagtcggaagcggaggcagcgaagtttgaggttctcgctggtgtgaaatgactgagtacaaactggtggtggttggagcaggtggtgttgggaaaagcgcactgacaatccagctaatccagaaccactttgtagatgaatatgatcccaccatagaggattcttaccgaaaacaggtggttatagacggtgaaacctgtctgttggacatactggatacagctggtcaagaagagtacagtgccatgagagaccaatacatgaggacaggcgaaggcttcctctgtgtatttgccatcaacaatagcaaatcatttgcagatattaacctttacagggaacagattaagcgagtaaaagactccgatgatgtacctatggtgctagtaggaaacaagtgtgatttgccaacaaggaccgtcgacacaaaacaagcccacgaactggccaagagttatgggattccattcattgaaacctcagccaagaccagacagggtgttgaagatgccttttacacactggtaagagaaatacgtcagtaccgaatgaagaaactcaacagcagtgatgacgggactcaaggttgtatggggttaccgtgtgtggtgatgtaacaagatacttttaaagttctagcatcagaaaagagccactgtcaagctgcactgacaccctggtcctgacttccctggaggagaagcgttcctgttgctattttcagtttcacaaagaagctcctgctatttccccaactctccgtagatcagtacattattctctgtttgagaagttctccgaataactacctcctcacttggttgtctgaccagagaaatgaacctcttgttactccccactgtttttccaccctggttctcccccagcacatataaacaaacctcccaggtttttcatctgaaaagtaattcatgctctgaaacagagaaccaaactgtagacatgaaattctgtaggaaacaatgtcttgagctctaaagtagcaactgctggtgactttttttttttttttttcctttttactgttgaacttggaactatgttggtttttggagaaatgtcgtaagttactgttttgctgagtatatagttaagtttaccattcggtttgtttgtaatgtcattggctatactctgtacctggcatctgctctgcattcataaatacaaaagtgaattctgacttttgagtctatcctagtgttctcaacttccacataattaaatctaacttttgcagcaaagtgcctttttcctagaagtggtttgtagatttgctttataatactttggtggaatagatgtctcaaaaaccattatacatgaaaatgaatgtctgagatacgtctatgatctgtctacctttgagggaaaaatataccgacataatagcagatgccatgtcttacgtgtatgaagttggatttccagagacctgatttgggtctcttccaagagaaagatgaaactggaaacaattatgaataacttcacttaatttttacctaatctctacttcggggtgggagggcagggagtaggttaccacttacaaaatatatgcaatttgtttcttctagcttactgataatgaacttccattcttatttaaatttaggtcatatcctaaagctttacatttgcaggtgttcgaaattgtaagtttaatgcagttttatttaatagctatgatcaatgattttcaagcctcagatgtattaacggacacattttcact

SEQ ID NO: 80 - protein, 189 aa, Felis catus; identical to SEQ ID NO: 68

SEQ ID NO: 81 - DNA, 4283 bp, Bos taurus
ggccgctccctagtgggggctgttcatggcggttccggggtctcccaacaattttcccggttgtggtcgtaatctatccgaagtggaggcagtggagctagaggttcttgctggtgtgaaatgactgagtacaaactggtggtggttggagcaggtggtgttgggaaaagtgcactgacaatccagctaatccagaaccactttgtagatgaatatgatcccaccatagaggattcctaccgaaaacaggtggttatagatggtgaaacctgtctgttggacatactggatacagctggacaagaggagtacagtgccatgagagaccaatacatgaggacaggcgaaggcttcctttgtgtgtttgccatcaataatagcaaatcatttgcagatattaacctctacagggaacagataaagcgtgtaaaggactcggatgatgtacctatggtgctagtaggaaacaagtgtgatttgccaacaaggacagttgacacaaaacaagcccatgaactggccaaaagttatgggattccattcattgaaacctcagccaagaccagacagggtgttgaagatgccttttacacactggtaagagaaatacgtcagtaccgaatgaaaaagctcaacagcagtgatgatggcactcaaggctgtatggggttgccgtgtgtggtgatgtaacaagatacttttaaagttctcacatcagaaaagagccactgtcaagctgcactgacaccctggtcctgacttccctggaggagaagtattcctgttgctatcttcagtttcaaaaagaagctcctgctatttccccaactctcagtagatcaatataatattctctatttgagaagttctcaagaataactacctcctcacttggttgtctgaccagagaattgaacctcttgttactcccagtatttttccaccctgggttctcccccagcacacacaaacgcacctctgccacccaggtttttcatctgaaaagcaattaatactctgaaacagagaaccaaactgtagaaacatgaaattctgtagaaaacaatgtcttgagctctaaagtagcaactgctggtgattttttttttttttttttcctttttattgttgaacttggaactatgttggtttgtggagaaatgtcataaattactgttttgctgagaatatagttaatgttgctctctggtttgtttgtaatgttatcagctatattctataaactggcatctactctgtatttagaaatacaaaaatgaatactgaccttttgagtctaccctcatcttctcgactttcttgtaattaaatgtaactttcacgatgaagtgccttttgcctgggagtgactcgtagacttcctttaaaatacttcagtggaatagatgtctcagaaactgttatacataagaataaatgtctgagatatgtctatgacccatctagctttgagggaaagatataccaatatgatagcagatgccatttcttacatctataacgttgattttctggagacctattttggggctctccgagagaaagatgagactataaatgattaggaataatttcacttaatttttacataacctccactttttgttttgtagtttactacctgcaaaacatataatttgattccttttagcttacagataatctaatgttaaatgaacttccattcatattttaatttggatcatatcaggaagtctacatttgcaggtgttcaaaaattgtaaaagtgtgatgcagttttatttaatagctgtgatcaatgattttcaagcctcaaatatgttaatagacacattttcactgtatatcatggtattaataattattgatgtatataattgtccttggtccccttctctgttcatcacctcatggcaatggcttgattaattatttcagctgagtaaagcatggtgctaatagaccagggtcacagtgtcaaaacttcagtgagccagtaagcatcacagagaaagaaattctttcacatttgctcaccattaactccagctaatagttttgccagatgtgtgtggttagtcctgcaaggaaaggagaagtcagttaatacaaattcttaaccaggactggaaaaacttgttttcctgagaagggtcagcttagaagtctttatctggactctatttttagccacatggaaatcaaattaagctgatcttttttctcaagtttttgagagtgaggatgcctcagatcaacatttttaaaatattctttattcttacgttcttttaagggtttaaaacaacgttgagtaattagtctgggcataccaggtaacaagctgataagtttgtgctgaacaagaagtagcctttggattgaaattgctgttttgagaagggatagaaaatataattaataattatgagacttgacttttctatttgcagataatatcctgataattctgatgaaaatagacttggataatttttgataaaagaatcgttccaaaatggccacttgctgttcttgtcttctaatgtgtaaatacttactgaggtcctcttctaatatgagttgtcatttattaagcaaattccacattgccttgaaatgaattcggaagagaagaaaaagtcatagtatacccagagaatgaaaaatccagagaattgtgctccttagtgttaattctgaagccttcgtagtccacacccatagacagaaactctctgccactttgcttctgctcctcttggagcattgcgctgtcatttccttgaggatagattgaggcttgtcaactcagttgtattgtcttcctcctcttcctcttgtctgtgtgactgacagtgtgactcttactaatgtcagatgcggggatgcggggaggtgggggggagtagctcattttaggctcttgcaccctttaccgttgtatgtgtgtgtcttttagttttctcaagaatgttctaagcacagaagtatctaaatggggccaaaattcagacttgaaaatgttcttttaatagcttcttaaaaagttacactttggtgtgaattttggcaggatagagtgacaaactcttaaacgctgaataacttcagttagtgtgttatagtttttagaatatgtttgtgattgctgaaaacaattatagtttacctcaaaatctgaaagtctctttccccaagttaagtgcctggccagctgtcaaagattacatattactttatgtttgtttgttttttaaaggttgcacattcaagattgtgaaaataaggtgttctgtctgaaagctaccatgcctgtctgtaaatgaatccactgagtgctgtacttgttccaacagcttactacagaatgctacttggtaatatcatactcgttacagttttcacttcaggagtgtactaggtagaatgatcctgtgtgtattgtagtgggctccatgtttagtcttttcagcatcctttaaactgctgtgaatttttgtcttgacttgaaagcaaggatagagaaacactttaaagagatactttgggtttttttccattccagaattggtgagcatagttagattttgctttacatttacagtcatgaactcttaagctggcagctacaaccaagaaccaaaagagggtgcattctgcttcttgtaattcatctttgctaataaattatgagaagcaaagataattaattagagaaactattttatttgggtggtttctataaacaagggactataattcttaaacattatttttcatttttgctgtttctttaagaaacctaatgtgccacaacattattttaaggtgtttcttaaaagaattgtttttaaaagtgttctcattttcagagtaattgtagatatatttcaaaatataactgataatttttaaaggcctgagtactgacctaagaagcagttgtatgaattctctggggggaagggaggagctcagtgaaagttgtatgacttttatatttctgtgccatcaaataaaggtaaaaatgtcttttgtgcagttttgctgttcaaacagaaactattggcctccttggccctaaatgaaagggctggtattttaagttgactattttattgtaaattaatccatcttaatttttttaaatttggttgaatgttctcttgttaaatgtttaaaaaataaaaactggaagttctttgcttagtcataaaaaaaaaaaaaaaaaaaaaaaaaaaaaaaaaaaaaaaaaaaaaaataaaaaaaaaaaaaaa

SEQ ID NO: 82 - protein, 189 aa, Bos taurus; identical to SEQ ID NO: 68

SEQ ID NO: 83 - DNA, 4825 bp, Gallus gallus
gcgccgggaccggaagccggaagctttgcagaagggtgttccgcgttcgcggtgcgggagcggtcagccggggtggcggggctggggccggccggggcaggcggctccgcgctccgcactgggccgctgggagggcgatgactgaatacaagctggtggtggtgggagctggcggcgtcgggaagagcgcgttgaccatccagctcatccagaaccacttcgtggacgagtacgaccccaccatcgaggattcgtacagaaagcaggttgtcatcgatggagagacgtgcttgttggacattctggacactgcaggacaggaagaatacagtgctatgcgtgatcagtacatgagaactggggaaggattcctttgtgtgtttgccattaacaacagtaaatcattcgctgatattaacctttacagagagcaaatcaagagagtgaaagattcagacgatgtgccaatggtgctggtggggaataagtgcgatttgccaacaaggacagtagacaccaaacaggctcaagagttagcaaaaagctacggcattcccttcatagagacatcagccaaaacgagacagggtgtggaagatgcgttttacacactggtgagggagattcggcagtaccggatgaaaaagctcaacagcaacgaagatgggaatcagggctgtatggggttgtcctgcattgtgatgtgataagatgccaggttcagatgtagctgctggacaagtctcgatgctactgtattgtgtctcatgctgatgccctgcagtattttggtgccagcgaccagactcttggtaccagttaattagctcaggatcctttcctgtgctccatctgaagaaaacatctctggtatctacctccttgctcagctcacagagcagtcatatctcttggtgtactgggattcttttctagctgtgttgtctgggtttgttcaagaagaaaaccagtcacaagaaaagtgaattacagagactaaatgctgtgaaaaagatcacactttacctccagagtaaaagctagaagtggcgtttgacccctttgcattggattcagatttgcggtgttgtcagaggagtggcagaagtaattttgccattacaaaggtttctgtcaccagtcggattggtatctgctgtctgtgcacccacacagtgtatctgcaacatctgcattgtgccagaagtatcacttaactgatgaactgatcctttatttttctgtaataaaaaggagatatctttgctaacttaagtgcctgtttgctcagaaggttggaggttgtatgctgttcccttgggctgaggagaaccccaaggatgaatttcttgggtgctcattgtcttgagcaggcaagttttgtgtgggtgatctcttttcatggcaggatattaaaatgggaatttgtagtctggaagatggagcagctgtttgtgagactcttgagttagggagagaaatgtataccacgtctgttctcgatccatcagaatggatccatccacctctttgtgtgtggaactgtgtatagtctgtattggttttctacagcacttggatctctttggaccaaattagcgagctgttcattttaacataactgccagtatttatagacaatttcttacggacagataatgaatttagaaactggaggttactttgggcagctgttcctcagctctgtctgtaacttgcaaattattctgagttattttctgcagaacctccttccttatcacgggaggagcctgggagttgaggttgactgtaattgggtcaatggttgtcacagacttaaggtgtccaggctgattggaggaggcactgagccctaacagagcactgagctgacttctaattgcagcatccttgcaaaatgaggaagggagttcagtgatgtctgcactgaagatgtatgatacactgatagcagttctgggtatgttgtaacagcttcaaagtagaaccgcagtactgcgtgagctgtgtgacttcttcctagaacacagcactgtcaccccatatggttgggacgtgcaggtgagaccaacacctaccaggttccctggcgtaccgtggccttctcagttcttgtgccagtgatactgggttctgttctgtggtgtcagacagcgtcctgtagcaaagctgaattcccacttagtctggtgagagaataaagagccatcagccaacagagggagcgttcattctgctggagcagtgcgagctgtaagcattacgagaggcgtagtttcagtttgttgcagtcaggttcctatattttcaaagctgaaatcagaaataagtaaatacggagaaaataagctgttgcttttaatgctctttcctccactaattgtactcttaattttcttcttgggaggccgaggatccatctgcataactttagctgtgatgctccagataagtgtttagaattcattttatctttgactgatgggactgataagaagttaacgcacaatatttttacatacaacatcgttttccagtgacctcctgagcggtgggaagcattatgggatagcaccggctgtgactcgagttcatttgaaggcgatctcttgcctgcaggttaaatgggacggagtcagaatcactgtgagccgtctgtaatcagcaaacagtctgtgggcttttcttactgtgttctctctgtttgccttagtttggtgcaggaagagttccttgtgacagcgtcctttgaggtgtgttgcaggagctgaccatttgctccttgagctgtgtgatgaactgttgtccacttaatggagttacagaagcagcttctgggagtcgcatctggtcgcatacattcagtgttttgggaagctgtcagtgtggtgtttgcactgtgtttgaatggtgttcatggtgggtctgttatgctcctggatgatttggggagatgtggggctgcttccgtggcagacaggatcagctcagggcgctgctgcctatggctgtgggaaacctcacagttggtgtttgaatagtggccaagtatgtcaattaaaaatacattttgaagggaggtttgtcatagctctgtactttggcatgctctgcttactgaaaacatactagctgtagctcaaaaaaagttgtgaatcctcagaataatacaggagctggcaattgtggctgctttctctttgtgttccttttctcttgggttggatgaagctttaaaaaggaaggagccctggtgagggttggtcagtgtgcatttcattcttggaaccagagaggaagttgcatcaactttcaggacgctgcagagctcacttgcacaggtggtgctccagtctatgtgatttttggggtcaaatcttgagatgatcttacaaaatcagattttgtacccatcatgagcatgaggtgagtggttgtgctcggtttctagctgcatgtatgtatacagacacgtgtatgcagacatgtctatgtgtgagtagttcgagtcagtcaaggttactggcagcacctaaagcgtatgcaccacataatgcatgcaggcaaaagtcctatcttaggagccatctcttcatgggtttgggtttatataggcagtatttttaaacagaatatccgaagcactttctggagttctgtggtaatgcagtgacacctatttggatgaaggaagatgtgtctgaggagcacgtaagcagatttgctgccctaacagagaggttttggtaaccgtggaaaaggttttctcctggatctgtgtgtgctcttggtgagctgcaatccatgacagggcacaaccagatgagaaggaaacccggccatcccatgcttgagcacagctctgactcagtagttccaccagatgtgccctttcagtcaaagtgttctgatctcttagagctttctgtagttcaagttaccactcactctccagcttgctcggttaatgtctgttggcggcgttgagttggacttgggaaaggtgtgtgtggtaggaacaagcagagtgtgatgtgcttctgttatcaggacttaagctagagtggttggcagataggaaatgcagctattccttgaaagcaagcagatcatggatggtcagccaaactgccctggctttggtgggagctgcactgcagaaggaccaaaccccaacaagatttggcacatttgtttagaagataagcacagatggttttgcacaaggcagctcctcataatggtggctttgtagatttagtccaaatgttcttatttagatctagcagcacatcactgtgtccgtgcccatctaacctcgctatcctaagtagagcagaccccaaacaaccttgttcaaaaactaccagtgcaaataactgaactaaatatttgttactgctgactgagaacagctgttcgagtgtagcattgtggcttgttaatgtgagtgccccaactctatggtcttattaaagaaacccaaacattgctcagattttgttcttattgtcatcataagacttgaatagtgatggtaatgcttacgtagacgtgtcttgtgagtgcacttcagtgatttagaaagaactggatttcaagcaactttggacctgtggggggagggagattaatgaaggtttgaatcacattctaattctatgtacagtccttcattactccacaagcctaaatcctatacagcctccaggatagctggaaactgttgagatctggactttttttttttaatccaagggctaacttgttgtaacttggtataattatctgctttcggaaatgcatctctgttggtttgaaa

SEQ ID NO: 84 - protein, 189 aa, Gallus gallus
MTEYKLVVVGAGGVGKSALTIQLIQNHFVDEYDPTIEDSYRKQVVIDGETCLLDILDTAGQEEYSAMRDQYMRTGEGFLCVFAINNSKSFADINLYREQIKRVKDSDDVPMVLVGNKCDLPTRTVDTKQAQELAKSYGIPFIETSAKTRQGVEDAFYTLVREIRQYRMKKLNSNEDGNQGCMGLSCIVM

SEQ ID NO: 85 - DNA, 2949 bp, Homo sapiens
cgcctcccttccccctccccgcccgacagcggccgctcgggccccggctctcggttataagatggcggcgctgagcggtggcggtggtggcggcgcggagccgggccaggctctgttcaacggggacatggagcccgaggccggcgccggcgccggcgccgcggcctcttcggctgcggaccctgccattccggaggaggtgtggaatatcaaacaaatgattaagttgacacaggaacatatagaggccctattggacaaatttggtggggagcataatccaccatcaatatatctggaggcctatgaagaatacaccagcaagctagatgcactccaacaaagagaacaacagttattggaatctctggggaacggaactgatttttctgtttctagctctgcatcaatggataccgttacatcttcttcctcttctagcctttcagtgctaccttcatctctttcagtttttcaaaatcccacagatgtggcacggagcaaccccaagtcaccacaaaaacctatcgttagagtcttcctgcccaacaaacagaggacagtggtacctgcaaggtgtggagttacagtccgagacagtctaaagaaagcactgatgatgagaggtctaatcccagagtgctgtgctgtttacagaattcaggatggagagaagaaaccaattggttgggacactgatatttcctggcttactggagaagaattgcatgtggaagtgttggagaatgttccacttacaacacacaactttgtacgaaaaacgtttttcaccttagcattttgtgacttttgtcgaaagctgcttttccagggtttccgctgtcaaacatgtggttataaatttcaccagcgttgtagtacagaagttccactgatgtgtgttaattatgaccaacttgatttgctgtttgtctccaagttctttgaacaccacccaataccacaggaagaggcgtccttagcagagactgccctaacatctggatcatccccttccgcacccgcctcggactctattgggccccaaattctcaccagtccgtctccttcaaaatccattccaattccacagcccttccgaccagcagatgaagatcatcgaaatcaatttgggcaacgagaccgatcctcatcagctcccaatgtgcatataaacacaatagaacctgtcaatattgatgacttgattagagaccaaggatttcgtggtgatggaggatcaaccacaggtttgtctgctaccccccctgcctcattacctggctcactaactaacgtgaaagccttacagaaatctccaggacctcagcgagaaaggaagtcatcttcatcctcagaagacaggaatcgaatgaaaacacttggtagacgggactcgagtgatgattgggagattcctgatgggcagattacagtgggacaaagaattggatctggatcatttggaacagtctacaagggaaagtggcatggtgatgtggcagtgaaaatgttgaatgtgacagcacctacacctcagcagttacaagccttcaaaaatgaagtaggagtactcaggaaaacacgacatgtgaatatcctactcttcatgggctattccacaaagccacaactggctattgttacccagtggtgtgagggctccagcttgtatcaccatctccatatcattgagaccaaatttgagatgatcaaacttatagatattgcacgacagactgcacagggcatggattacttacacgccaagtcaatcatccacagagacctcaagagtaataatatatttcttcatgaagacctcacagtaaaaataggtgattttggtctagctacagtgaaatctcgatggagtgggtcccatcagtttgaacagttgtctggatccattttgtggatggcaccagaagtcatcagaatgcaagataaaaatccatacagctttcagtcagatgtatatgcatttggaattgttctgtatgaattgatgactggacagttaccttattcaaacatcaacaacagggaccagataatttttatggtgggacgaggatacctgtctccagatctcagtaaggtacggagtaactgtccaaaagccatgaagagattaatggcagagtgcctcaaaaagaaaagagatgagagaccactctttccccaaattctcgcctctattgagctgctggcccgctcattgccaaaaattcaccgcagtgcatcagaaccctccttgaatcgggctggtttccaaacagaggattttagtctatatgcttgtgcttctccaaaaacacccatccaggcagggggatatggtgcgtttcctgtccactgaaacaaatgagtgagagagttcaggagagtagcaacaaaaggaaaataaatgaacatatgtttgcttatatgttaaattgaataaaatactctctttttttttaaggtgaaccaaagaacacttgtgtggttaaagactagatataatttttccccaaactaaaatttatacttaacattggatttttaacatccaagggttaaaatacatagacattgctaaaaattggcagagcctcttctagaggctttactttctgttccgggtttgtatcattcacttggttattttaagtagtaaacttcagtttctcatgcaacttttgttgccagctatcacatgtccactagggactccagaagaagaccctacctatgcctgtgtttgcaggtgagaagttggcagtcggttagcctgggttagataaggcaaactgaacagatctaatttaggaagtcagtagaatttaataattctattattattcttaataatttttctataactatttctttttataacaatttggaaaatgtggatgtcttttatttccttgaagcaataaactaagtttctttttataaaaa

SEQ ID NO: 86 - protein, 765 aa, Homo sapiens
AALSGGGGGGAEPGQALFNGDMEPEAGAGAGAAASSAADPAIPEEVWNIKQMIKLTQEHIEALLDKFGGEHNPPSIYLEAYEEYTSKLDALQQREQQLLESLGNGTDFSVSSSASMDTVTSSSSSSLSVLPSSLSVFQNPTDVARSNPKSPQKPIVRVFLPNKQRTVVPARCGVTVRDSLKKALMMRGLIPECCAVYRIQDGEKKPIGWDTDISWLTGEELHVEVLENVPLTTHNFVRKTFFTLAFCDFCRKLLFQGFRCQTCGYKFHQRCSTEVPLMCVNYDQLDLLFVSKFFEHHPIPQEEASLAETALTSGSSPSAPASDSIGPQILTSPSPSKSIPIPQPFRPADEDHRNQFGQRDRSSSAPNVHINTIEPVNIDDLIRDQGFRGDGGSTTGLSATPPASLPGSLTNVKALQKSPGPQRERKSSSSSEDRNRMKTLGRRDSSDDWEIPDGQITVGQRIGSGSFGTVYKGKWHGDVAVKMLNVTAPTPQQLQAFKNEVGVLRKTRHVNILLFMGYSTKPQLAIVTQWCEGSSLYHHLHIIETKFEMIKLIDIARQTAQGMDYLHAKSIIHRDLKSNNIFLHEDLTVKIGDFGLATVKSRWSGSHQFEQLSGSILWMAPEVIRMQDKNPYSFQSDVYAFGIVLYELMTGQLPYSNINNRDQIIFMVGRGYLSPDLSKVRSNCPKAMKRLMAECLKKKRDERPLFPQILASIELLARSLPKIHRSASEPSLNRAGFQTEDFSLYACASPKTPIQAGGYGAFPVH

SEQ ID NO: 87 - DNA, 3906 bp, Rattus norvegicus
atggcggcgctgagtggcggcggtggcagcagcagcggtggcggtggcggcggcggcggcggcggtggtggcggcggcggcggcggcgccgaacagggacaggctctgttcaatggcgacatggagccggaggccggcgctggcgccgcggcctcttcggccgcggacccggccattcctgaagaggtgtggaatatcaagcaaatgattaagttgacacaggaacatatagaggccctattggacaagtttggtggggagcataacccaccgtcaatatacctggaggcctatgaagagtacaccagcaagctagatgcccttcagcagagagagcagcagctgttggaatccctggtttttcaaactcccacagatgtatcacggaacaaccccaagtcaccacagaaacctatcgttcgtgtcttcctgcccaacaaacagaggacagtggtgcccgcaagatgtggtgtaacggtccgagacagtctaaagaaagcactaatgatgaggggtctcatcccagagtgctgtgctgtttacagaattcaggacggagagaagaaaccaattggctgggacactgacatttcctggcttactggagaggagctacatgttgaagtactagagaatgttcctctgacaacccacaacttcgtacggaaaacttttttcaccttagcattttgtgacttttgccgaaagctgcttttccagggtttccgctgtcaaacatgtggttataagtttcaccagcgttgtagtacagaggttccactgatgtgtgttaattatgaccaacttgatttgctgtttgtctccaagttctttgagcatcacccagtaccacaggaggaggccttctcagcagagactacccttccatctggatgctcttccgcacccccctcagactctattgggccccaaatcctcaccagtccatctccttcaaaatccattccaattccacagcccttccggccagcagatgaagatcatcgcaatcagtttgggcaacgagaccgctcctcctccgctcccaatgttcatataaacacaatcgaacctgtcaatattgatgaaaaattcccagaagtggaattacaggatcaaagggatttgattagagaccaggggtttcgtggggatggagcccctttgaaccagctgatgcgctgtcttcggaaataccaatcccggactcccagccccctcctccattctgtccccagtgaaatagtgtttgattttgagcctggcccagtgttcagagggtcaaccacaggcttgtcggccaccccacctgcctcattacctggctcactcactaacgtgaaagccttacagaaatctccaggacctcagcgggaaaggaagtcctcctcctcctcctcctccacggaagacagaagtcggatgaaaacacttggtagaagagattcaagtgatgattgggagattcctgatggacagattacagtgggacagagaattggatctgggtcctttggaactgtctacaagggaaagtggcatggcgacgtggcagtgaaaatgctgaatgtgacagcacccacacctcagcagttacaggccttcaaaaacgaagtcggagtactcaggaaaactcgacatgtgaacatcctccttttcatgggctattctacaaagccacagctggctattgttacacagtggtgtgaaggctccagcttatatcaccatctccacatcattgagaccaaatttgagatgatcaaacttatagatattgcacggcagactgcacagggcatggattacttacacgccaagtcaatcatccacagagacctcaagagtaataatatatttcttcatgaagacctcacggtaaaaataggtgactttggtttagccacagtgaagtcccgatggagtgggtcccatcagtttgaacagttgtctggatctattttgtggatggcacccgaagtaatcagaatgcaagataaaaacccatatagctttcagtcagacgtgtatgcatttgggattgttctgtatgaactgatgactggtcagctaccttattcaaacatcaacaacagggatcagataatttttatggtgggacgaggatacctatctccagatctcagtaaggtacggagtaactgtccaaaagccatgaagagattaatggcagagtgcctcaaaaagaaaagagacgagagaccactctttccccaaattctcgcctctattgagctgctggcccgctcattgccaaaaattcaccgcagtgcatcagaaccctccttgaatcgggctggtttccaaacagaagattttagtctgtatgcttgtgcttctccaaaaacacccatccaagcagggggatatggagaatttgcagccttcaagtagccactccatcatggcagcatctactctttatttcttaagtcttgtgttcatacaatttgttaacatcaaaacacagttctgttcctcaaattttttttaaagatacaaaattttcaatgcataagctcgtgtggaacagaatggaatttcctattcaacaaaagagggaagaatgttttaggaaccagaattctctgctgcccgtgtttcttcttcaacacaaatatcatgtgcatacaactctgcccattcccaagaagaaagaggagagaccccgaattctgcccttttggtggtcaggcatgatggaaagaatttgctgctgcagcttgggaaaaattgctatggaaagtctgccagtcaactttgcccttctaaccaccagatccatttgtggctggtcatctgatggggcgatttcaatcaccaagcatcgttcttgcctgttgtgggattatgtcgtggagcactttccctatccaccaccgttaatttccgagggatggagtaaatgcagcataccctttgtgtagcacctgtccagtcctcaaccaatgctatcacagtgaagctctttaaatttaagtggtgggtgagtgttgaggagagactgccttgggggcagagaaaaggggatgctgcatcttcttcctcacctccagctctctcacctcgggttgccttgcacactgggctccgcctaaccactcgggctgggcagtgctggcacacattgccgccttttctcattgggtccagcaattgagcagagggttgggggattgtttcctccacaatgtagcaaattctcaggaaaatacagtccatatcttcctctcagctcttccagtcaccaaatacttacgtggctcctttgtccaggacataaaacaccgtggacaacacctaattaaaagcctacaaaactgcttactgacagttttgaatgtgagacatttgtgtaatttaaatgtaaggtacaggtcttaatttcttctattaagtttcttctatttttatttaaacgaagaaaataattttcaggtttaattggaataaacgaatacttcccaaaagactatataccctgaaaattatatttttgttaattgtaaacaacttttaaaaaatggttattatccttttctctacctaaaattatgggaaatcttagcataatgacaattatttatactttttaaataaatggtacttgctggatccacactaacatctttgctaacattcccattgtttcttccaacttcactcctacactacatcctccatcctctttctagtcttttatctataatatgcaacctaaaataaaagtggtggtgtctccattcattcttcttcttccttttttccccaagcctggtcttcaaaaggttgggtaatttagtagctgagttccctaggtagaaatagaactattagggacattggggttgtaggaaagcgtgaggcctgtcaccagttgttctt

SEQ ID NO: 88 - protein, 804 aa, Rattus norvegicus
MAALSGGGGSSSGGGGGGGGGGGGGGGGGAEQGQALFNGDMEPEAGAGAAASSAADPAIPEEVWNIKQMIKLTQEHIEALLDKFGGEHNPPSIYLEAYEEYTSKLDALQQREQQLLESLVFQTPTDVSRNNPKSPQKPIVRVFLPNKQRTVVPARCGVTVRDSLKKALMMRGLIPECCAVYRIQDGEKKPIGWDTDISWLTGEELHVEVLENVPLTTHNFVRKTFFTLAFCDFCRKLLFQGFRCQTCGYKFHQRCSTEVPLMCVNYDQLDLLFVSKFFEHHPVPQEEAFSAETTLPSGCSSAPPSDSIGPQILTSPSPSKSIPIPQPFRPADEDHRNQFGQRDRSSSAPNVHINTIEPVNIDEKFPEVELQDQRDLIRDQGFRGDGAPLNQLMRCLRKYQSRTPSPLLHSVPSEIVFDFEPGPVFRGSTTGLSATPPASLPGSLTNVKALQKSPGPQRERKSSSSSSSTEDRSRMKTLGRRDSSDDWEIPDGQITVGQRIGSGSFGTVYKGKWHGDVAVKMLNVTAPTPQQLQAFKNEVGVLRKTRHVNILLFMGYSTKPQLAIVTQWCEGSSLYHHLHIIETKFEMIKLIDIARQTAQGMDYLHAKSIIHRDLKSNNIFLHEDLTVKIGDFGLATVKSRWSGSHQFEQLSGSILWMAPEVIRMQDKNPYSFQSDVYAFGIVLYELMTGQLPYSNINNRDQIIFMVGRGYLSPDLSKVRSNCPKAMKRLMAECLKKKRDERPLFPQILASIELLARSLPKIHRSASEPSLNRAGFQTEDFSLYACASPKTPIQAGGYGEFAAFK

SEQ ID NO: 89 - DNA, 9728 bp, Mus musculus
ccctcaggctcggctgcgccggggccgccggcgggttccagaggtggcctccgccccggccgctccgcccacgccccccgcgcctccgcgcccgcctccgcccgccctgcgcctcccttccccctccccgccccgcggcggccgctcggcccggctcgcgcttcgaagatggcggcgctgagtggcggcggtggcagcagcagcggtggcggcggcggcggtggcggcggcggtggcggtggcgacggcggcggcggcgccgagcagggccaggctctgttcaatggcgacatggagccggaggccggcgctggcgccgcggcctcttcggctgcggacccggccattcctgaagaggtatggaatatcaagcaaatgattaagttgacacaggaacatatagaggccctattggacaaatttggtggagagcataacccaccatcaatatacctggaggcctatgaagagtacaccagcaagctagatgcccttcagcaaagagaacagcagcttttggaatccctggtttttcaaactcccacagatgcatcacggaacaaccccaagtcaccacagaaacctatcgttagagtcttcctgcccaacaaacagaggacagtggtacccgcaagatgtggtgttacagttcgagacagtctaaagaaagcactgatgatgagaggtctcatcccagaatgctgtgctgtttacagaattcaggatggagagaagaaaccaattggctgggacacggacatttcctggcttactggagaggagttacatgttgaagtactggagaatgtcccacttacaacacacaactttgtacggaaaacttttttcaccttagcattttgtgacttttgccgaaagctgcttttccagggtttccgttgtcaaacatgtggttataaatttcaccagcgttgtagtacagaggttccactgatgtgtgtaaattatgaccaacttgatttgctgtttgtctccaagttctttgagcatcacccagtaccacaggaggaggcctccttcccagagactgcccttccatctggatcctcttccgcacccccctcagactctactgggccccaaatcctcaccagtccatctccttcaaaatccattccaattccacagcccttccgaccagcagatgaagatcatcgcaatcagtttgggcaacgagaccggtcctcctcagctcccaatgttcatataaacacaattgagcctgtgaatatcgatgaaaaattcccagaagtggaattacaggatcaaagggatttgattagagaccaggggtttcgtggtgatggagcccccttgaaccaactgatgcgctgtcttcggaaataccaatcccggactcccagccccctcctccattctgtccccagtgaaatagtgtttgattttgagcctggcccagtgttcagagggtcaaccacaggcttgtccgccaccccgcctgcctcattacctggctcactcactaacgtgaaagccttacagaaatctccaggtcctcagcgggaaaggaagtcatcttcttcctcatcctcggaggacagaagtcggatgaaaacacttggtagaagagattcaagtgatgactgggagattcctgatggacagattacagtgggacagagaattggatctgggtcatttggaactgtctacaagggaaagtggcatggtgatgtggcagtgaaaatgttgaatgtgacagcacccacacctcaacagctacaggccttcaaaaatgaagtaggagtgctcaggaaaactcgacatgtgaatatcctccttttcatgggctattctacaaagccacaactggcaattgttacacagtggtgtgagggctccagcttatatcaccatctccacatcattgagaccaaatttgagatgatcaaacttatagatattgctcggcagactgcacagggcatggattacttacacgccaagtcaatcatccacagagacctcaagagtaataatatatttcttcatgaagacctcacggtaaaaataggtgactttggtctagccacagtgaaatctcggtggagtgggtcccatcagtttgaacagttgtctggatctattttgtggatggcaccagaagtaatcagaatgcaagataaaaacccgtatagctttcagtcagacgtgtatgcgtttgggattgttctgtacgaactgatgaccggccagctaccttattcaaacatcaacaacagggatcagataatttttatggtgggacgaggatacctatctccagatctcagtaaggtacggagtaactgtccaaaagccatgaagagattaatggcagagtgcctcaaaaagaaaagagacgagagaccactctttccccaaattctcgcctccattgagctgctggcccgctcattgccaaaaattcaccgcagtgcatcagaaccttccttgaatcgggctggtttccaaacagaagattttagtctgtatgcttgtgcttctccgaaaacacccatccaagcagggggatatggagaatttgcagccttcaagtagccagtccatcatggcagcatctactctttatttcttaagtcttgtgttcatacagtttgttaacatcaaaacacagttctgttcctcaaaaaattttttaaagatacaaaattttcaatgcataagttcatgtggaacagaatggaatttcctattcaacaaaagagggaagaatgttttaggaaccagaattctctgctgcccgtgtttcttcttcaacataactatcacgtgcatacaagtctgcccattcccaagaagaaagaggagagaccctgaattctgcccttttggtggtcaggcatgatggaaagaatttgctgctgcagcttgggaaaattgctatggaaagtctgccagtcgactttgcccttctaaccaccagatcagcctgtggctggtcatctgatggggcgatttccatcaccaagcatcgttcttgcctattctgggattatgttgtggagcactttccctgtccagcaccgttcatttctgagggatggagtaaatgcagcattcccttgtgtagcgcctgttcagtcctcagcagctgctgtcacagcgaagctttttacagttaagtggtgggggagagttgaggagagcctgcctcggggcagagaaaagggggtgctgcatcttcttcctcacctccagctctctcacctcgggttgccttgctcactgggctccgcctaaccactcaggctgctcagtgctggcacacattgccttcttttctcattgggtccagcaattgaggagagggttgggggattgtttcctcctcaatgtagcaaattctcaggaaaatacagtccatatcttcctctcagctcttccagtcaccaaatacttacgtggctcctttgtccaggacataaaacaccgtggacaacacctaattaaaagcctacaaaactgcttactgacagttttgaatgtgagacacttgtgtaatttaaatgtaaggtacaggttttaatttctgagtttcttctatttttatttaaaagaagaaaataattttcagttttaattggaataaatgagtacttcccacaagactatataccctgaaaattatatttttgttaattgtaaacaacttttaaagaataattattatccttttctctacctaaaaattatggggaatcttagcataatgacaattatttatactttttaaataaatggtacttgctggatccacactaacatctttgctaacaatcccattgtttcttccaacttaactcctacactacatcctacatcctctttctagtcttttatctataatatgcaacctaaaataaacgtggtggcgtctccattcattctccctcttcctgttttccccaagcctggtcttcaaaaggttgggtaatcggtccctgagctccctagctggcaatgcaactattagggacattggagttgcaggagagcaggaagcctgtccccagctgttcttctagaaccctaaatcttatctttgcacagatcaaaagtatcacctcgtcacagttctccttagcctttacttacaggtaatataaataaaaatcaccatagtagtaaagaaaacaactggatggattgatgaccagtacctctcagagccaggaatcttgaatctccaggatttatacgtgcaaatttaaggagatgtacttagcaacttcaagccaagaacttccaaaatactagcgaatctaaaataaaatggaattttgagttatttttaaagttcaaattataattgataccactatgtatttaagcctactcacagcaagttagatggattttgctaaactcattgccagactgtggtggtggtggtggtagtgtgcacctttaatccaagcaactcagcaatcagaatgaggtaaatctctgtgaatacaaggcctgcctagtctgcagcgctagttccaggatagccagggctacacacacaaaaaccctctctcaaaaaaaacaaaattaattagttgataataaaaaataactaaagtatcatcaaaggaaggcctactggaagttttatatattcccagtaaattgaaaaatattctgaagttattaaccagttagcaacaatgtgtttttaagtcttacataaacagagcaaagtcttcaaatgtttcagagctgagaagataattgtgcttgatatgaaaaatagcctctccatatgatgtgccacattgaaaggcgtcattacccttttaaatacttcttaatgtggctttgttccctttacccaggattagctagaaagagctaggtaggcttcggccacagttgcacatttcgggcctgctgaagaatgggagctttgaaggctggccttggtggaggagcccctcagtgctggagggtggggcgtgtacgcagcatggaagtggtctagacagagtgcaaagggacagacttctttctcattttagtatagggtgatgtctcacttgaaatgagaaagtagagttgatattaaacgaagctgtgcccagaaaccaggctcagggtattgtgagattttctttttaaatagagaatataaaagatagaaataaatatttaaaccttccttcttattttctatcaaatagattttttttatcatttgcaaacaacataaaaaaaggtttcttttgtggggttttctttccttcttttttttttttttttttttttaagactgcagataatcttgttgagctcctcggaaaatacaaggaagtccgtgtttgtgcagagcgctttatgagtaactgtatagacagtgtggctgcttcactcatcccagagggctgcagctgtcggcccatgaagtggctgcagtgcctcgtgagatctgctttgttttgtttggagtgaagtctttgaaaggtttgagtgcaactatataggactgtttttaaataagtagtattcctcatgaactttctcattgttaagctacaggacccaaactctaccactaagatattattaacctcaaaatgtagtttatagaaggaatttgcaaatagaatatccagttcgtacttatatgcatcttcaacaaagattctctgtgacttgttggatttggttcctgaacagcccatttctgtatttgaggttaggagggcataatgaggcatcctaaaagacaatctgatataaactgtatgctagatgtatgctggtaggggagaaagcattctgtaaagacatgatttaagacttcagctctgtcaaccagaaaccttgtaaatacttcctgtcttggtgcagccccgcccctttgatcacacgatgttgtcttgtgcttgtcagacactgtcagagctgctgttcgtccctctgcagatctcacctgtccccactgcacacccacctcctgcctcttgcagacctcagcatctagctttagttggaaacagttcagggttcaggtgacttcttaaaaaaaaaaaaaaaccctacctcctcagaatgaggtaatgaatagttatttatttaaagtatgaagagtcaggagcgctcgaacatgaaggtgatttaagatggttcctttcgtgtgtattgtagctgagcacttgtttttgtcctaaagggcattatacatttaagcagtgattctgtttaaagatgtttttctttaaaggtgtagctcagagtatctgttgttggaattggtgccagagtctgcttaatagatttcagaatcctaagcttaagtcagtcgcatgaagttaagtagttatggtaacactttgctagccatgatataattctactttttaggagtaggtttggcaaaactgtatgccttcaaagtgagttggccacagctttgtcacatgcacagatactcatctgaagagactgcccagctaagagggcggaaggatacccttttttcctacgattcgcttctttgtccacgttggcattgttagtactagtttatcagcaccttgaccagcagatgtcaaccaataagctatttttaaaaccatagccagagatggagaggtcactgtgagtagaaacagcaggacgcttacaggagtgaaatggtgtagggaggctctagaaaaatatcttgacaatttgccaaatgatcttactgtgccttcatgatgcaataaaaaagctaacattttagcagaaatcagtgatttacgaagagagtggccagtctggtttaactcagctgggataatatttttagagtgcaatttagactgcgaagataaatgcactaaagagtttatagccaattcacatttgaaaaataagaaaatggtaaattttcagtgaaatatttttttaaagcacataatccctagtgtagccagaaatatttaccacatagagcagctaggctgagatacagtccagtgacatttctagagaaaccttttctactcccacgggctcctcaaagcatggaaattttatacaaaatgtttgacattttaagatactgctgtagtttagttttgaaatagtatgtgctgagcagcaatcatgtactaactcagagagagaaaacaacaacaaattgtgcatctgatttgttttcagagaaatgctgccaacttagatactgagttctcagagcttcaagtgtaaacttgcctcccaagtcctgtttgcaaatgaagttggctagtgctactgactgctccagcacatgatggaaggcagggggctgtctctgaagtgtcttctataaagggacaatagaatagtgagagacctggtcagtgtgtgtcagctggacactccatgctatgggacttgcatcttctgtcctcaccatccccaagacattgtgctttcctcagttgtcctctagctgtttcactcagacaccaagatgaattactgatgccagaaggggccaaaatggccagtgtgttttgggggttgtatcagttgactggacaataactttaatagtttcagatcatttatttttacttccattttgacagacatttaaatggaaatttagtcctaacttttgtcatttgaaaggaaaaattaacagttcctataagatacttttgaggtggaatctgacatcctaattttttttcttttcagtgggtttgcagcgagggtcttgtatgcactaggcaagggttctaccactaagccacatttcccaggaaataaaatgttaacagttaaaacatacacacaaatacacaaacaccttattaccactttagtaaagtgagagatgtgcgtcctttgtctcagtctccacgatttcagctgccccttgtatgaataactcagtctcgctaaactgtttacttttatttacctggtttgactagttgcagctatataaccagttgtgcatgaggacaacagccagtgtgtttgttttgtttttggttttttgtggtacattttttgtaaagaattctgtagattgaagtgctctttgaaaacagaactgagatatatttattcttgttagcatcaaaaaacattttgtgcaaatgatttgcttttcctggcaggctgagtaccatatccagcgcccacaattgcgggttcccatctaccatgtccacaggggagacagacgggaagcacatgaggggtgtgtttacagagttgtaggagttatgtagttctcttgttgccttggaaatcactgttgttttaagactgttgaacccgtgtgtttggctgggctgtgagttacatgaagaaactgcaaactagcatatgcagacaaagctcacagactaggcgtaaatggaggaaaatggaccaaaataaggcagggtgacacataaaccttgggcttcggagaaaactaagggtggagatgaactataatcacctgaatacaatgtaagagtgcaataagtgtgcttattctaagctgtgaacttcttttaaatcattcctttctaatacatttatgtatgttccattgctgactaaaaccagctatgagaacatatgcctttttattcatgttaactaccagtttaagtggctaaccttaatgtcttatttatcttcattttgtattagtttacataccaggtatgtgtgtgtgctgtactcttcttccctttatttgaaaacacttttcactgggtcatctccttggccattccacaacacaactttggtttggctttcaatgtcaccttatttgatggcctgtgtcccagtagcagaatttatggtattcccattgctggctgctcttccgaccctttgcttctacagcacttgtctctcctaagatagtcagaaactaactgatcaggggatggacttcaccattcatcgtgtctcttcaattctattaaatagaccactcttgggctttagaccaggaaaaaggagacagctctagccatctaccaagcctcaccctaaaaggtcacccgtacttcttggtctgaggacaagtctccactccagtaagggagaggggaggaaatgcttcctgtttgaaatgcagtgaattcctatggctcctgtttcaccacccgcacctatggcaacccatatacattcctcttgtctgtaactgccaaaggttgggtttatgtcacttcagttccactcaagcattgaaaaggttctcatggagtctggggtgtgcccagtgaaaagatggggactttttcattatccacagacctctctatacctgctttgcaaaaattataatggagtaactatttttaaagcttatttttcaattcataagaaaaagacatttattttcaatcaaatggatgatgtctcttatcccttatccctcaatgtttgcttgaattttgtttgttccctatacctactccctaattctttagttccttcctgctcaggtcccttcatttgtactttggagtttttctcatgtaaatttgtataatggaaaatattgttcagtttggatagaaagcatggagaaataaataaaaaaagatagctgaaaatcaaattgaagaaatttatttctgtgtaaagttatttaaaaactctgtattatatttaaagaaaaaagcccaaccccccaaaaagtgctatgtaattgatgtgaatatgcgaatactgctataataaagattgactgcatggagaaa

SEQ ID NO: 90 - protein, 804 aa, Mus musculus
MAALSGGGGSSSGGGGGGGGGGGGGDGGGGAEQGQALFNGDMEPEAGAGAAASSAADPAIPEEVWNIKQMIKLTQEHIEALLDKFGGEHNPPSIYLEAYEEYTSKLDALQQREQQLLESLVFQTPTDASRNNPKSPQKPIVRVFLPNKQRTVVPARCGVTVRDSLKKALMMRGLIPECCAVYRIQDGEKKPIGWDTDISWLTGEELHVEVLENVPLTTHNFVRKTFFTLAFCDFCRKLLFQGFRCQTCGYKFHQRCSTEVPLMCVNYDQLDLLFVSKFFEHHPVPQEEASFPETALPSGSSSAPPSDSTGPQILTSPSPSKSIPIPQPFRPADEDHRNQFGQRDRSSSAPNVHINTIEPVNIDEKFPEVELQDQRDLIRDQGFRGDGAPLNQLMRCLRKYQSRTPSPLLHSVPSEIVFDFEPGPVFRGSTTGLSATPPASLPGSLTNVKALQKSPGPQRERKSSSSSSSEDRSRMKTLGRRDSSDDWEIPDGQITVGQRIGSGSFGTVYKGKWHGDVAVKMLNVTAPTPQQLQAFKNEVGVLRKTRHVNILLFMGYSTKPQLAIVTQWCEGSSLYHHLHIIETKFEMIKLIDIARQTAQGMDYLHAKSIIHRDLKSNNIFLHEDLTVKIGDFGLATVKSRWSGSHQFEQLSGSILWMAPEVIRMQDKNPYSFQSDVYAFGIVLYELMTGQLPYSNINNRDQIIFMVGRGYLSPDLSKVRSNCPKAMKRLMAECLKKKRDERPLFPQILASIELLARSLPKIHRSASEPSLNRAGFQTEDFSLYACASPKTPIQAGGYGEFAAFK

SEQ ID NO: 91 - DNA, 2232 bp, Oryctolagus cuniculus
atggggaatgtgtggaatatcaaacaaatgattaagttgacacaggagcatatagaggccctattggacaaatttggtggggagcataatccaccatcaatatatctggaggcctacgaagaatacaccagcaagctagatgccctccaacaaagagaacagcagttattggaatccctagtttttcaaaatcccacagatgtgtcacggagcaaccccaagtcaccacaaaaacctattgttagagtcttcctgcccaacaaacagaggacagtggtacctgcaagatgtggagttacggttcgagacagtctaaagaaagcgctgatgatgagaggtctgatcccagaatgctgtgctgtttacagaattcaggatggagagaagaagccaattggctgggacactgatatttcctggctcactggagaagagctgcatgtggaagtgttagagaatgtcccactcaccacacataactttgtacggaaaacttttttcaccttagcattttgtgacttctgtagaaagctgcttttccagggtttccgctgtcaaacatgtggctacaaatttcaccagcgttgtagtacggaagttccactgatgtgtgttaattatgaccaacttgatttgctgtttgtctccaagttctttgaacaccacccagtaccacaggaggaggcctccttagcagagactgccctcacatctgggtcatcgccttccgcacctccctcagactctattgggcaccaaattctcaccagtccgtccccttcaaaatccattccgattccacagtccttccgaccagcagatgaagatcatcgaaatcagtttgggcaacgagaccggtcttcatcagcgcctaatgttcacattaacacaatagaacctgtcaatattgatgaaaaattcccagaagtggaattacaggatcaaagggacttgattagagaccaagggtttcgtggtgatggagcccctttgaaccagctgatgcgctgtcttcggaaataccaatcccggactcccagtcccctcctaccttctgtccccagtgacatagtgtttgattttgagcctggcccagtgttcagaggatcgaccacgggtttgtctgccactccccctgcctcattacctggctcactcactagtgtgaaagctgtacagagatccccaggacctcagcgagagaggaagtcgtcttcctcctcagaagacaggaatcgaatgaaaactcttggtagacgggattcaagtgatgattgggagattcctgatgggcagatcaccgtgggacagagaattggatctggatcatttggaaccgtctacaagggaaaatggcacggtgatgtggcagtaaaaatgttgaatgtgacagcacctacacctcagcagttacaggccttcaaaaatgaagtaggagtactcaggaaaacacgacatgtgaatatcctacttttcatgggctattccacaaagccacagctggctattgttacccagtggtgtgagggctccagtttatatcaccatctccacatcattgagaccaaattcgagatgatcaaacttatagatattgcacggcagactgcacagggcatggattacttacacgccaagtcaatcatccacagagacctcaagagtaataatatatttcttcatgaagacctcacagtaaaaataggtgattttggtctagccacagtgaaatctcgatggagtgggtcccatcagtttgaacaattgtctggatccattttgtggatggcaccagaagtaatcagaatgcaagacaaaaacccatatagctttcagtcagatgtatatgcatttgggattgttctgtatgaattgatgactgggcagttaccttactcaaacatcaacaacagggaccagatcatttttatggtgggacgtggctacctgtctccagacctcagtaaggtacggagtaactgtccgaaagccatgaagagattaatggcagagtgcctcaaaaagaaaagagatgagagaccactctttccccaaattctcgcctccattgagctgctggcccgctcattgccaaaaatccaccgcagtgcatcagaaccctccttgaatcgggctggtttccagacagaggattttagtctatatgcttgtgcttctccaaaaacacccatccaggcagggggatatggagaatttgcagccttcaagtag

SEQ ID NO: 92 - protein, 743 aa, Oryctolagus cuniculus
MGNVWNIKQMIKLTQEHIEALLDKFGGEHNPPSIYLEAYEEYTSKLDALQQREQQLLESLVFQNPTDVSRSNPKSPQKPIVRVFLPNKQRTVVPARCGVTVRDSLKKALMMRGLIPECCAVYRIQDGEKKPIGWDTDISWLTGEELHVEVLENVPLTTHNFVRKTFFTLAFCDFCRKLLFQGFRCQTCGYKFHQRCSTEVPLMCVNYDQLDLLFVSKFFEHHPVPQEEASLAETALTSGSSPSAPPSDSIGHQILTSPSPSKSIPIPQSFRPADEDHRNQFGQRDRSSSAPNVHINTIEPVNIDEKFPEVELQDQRDLIRDQGFRGDGAPLNQLMRCLRKYQSRTPSPLLPSVPSDIVFDFEPGPVFRGSTTGLSATPPASLPGSLTSVKAVQRSPGPQRERKSSSSSEDRNRMKTLGRRDSSDDWEIPDGQITVGQRIGSGSFGTVYKGKWHGDVAVKMLNVTAPTPQQLQAFKNEVGVLRKTRHVNILLFMGYSTKPQLAIVTQWCEGSSLYHHLHIIETKFEMIKLIDIARQTAQGMDYLHAKSIIHRDLKSNNIFLHEDLTVKIGDFGLATVKSRWSGSHQFEQLSGSILWMAPEVIRMQDKNPYSFQSDVYAFGIVLYELMTGQLPYSNINNRDQIIFMVGRGYLSPDLSKVRSNCPKAMKRLMAECLKKKRDERPLFPQILASIELLARSLPKIHRSASEPSLNRAGFQTEDFSLYACASPKTPIQAGGYGEFAAFK

SEQ ID NO: 93 - DNA, 2186 bp, Cavia porcellus
atggcggcgctcagcggcggcggtggcgcggagcagggccaggctctgttcaacggggacatggagctcgaggccggcgccggcgccgcagcctcttcggctgcagaccctgccattcccgaggaggtatggaatatcaaacaaatgattaagttgacgcaggaacacatagaggccctattggacaaatttggtggagagcataatccaccatcaatatacctggaggcctatgaagaatacaccagcaaactagatgccctccaacaaagagaacagcagttactggaatccctcgggaatggaactgatttttctgtttctagctctgcatcactggacaccgttacatcttcttcttcttctagcctttcagtactaccttcatctctttcagtttttcaaaatcctacagatgtgtcacggagcaaccccaaatcaccacaaaaacctattgttagagtcttcctgcccaacaaacagaggacagtggtacctgcaaggtgtggagttacagtccgagacagtctgaagaaagcactcatgatgagaggtcttatcccagagtgctgtgctgtgtacagaattcaggatggagaaaagaaaccaattggctgggacactgacatttcctggcttactggggaagaattacatgtagaagtattggagaatgttccacttacaacacacaattttgtatgtatctttatattttttttgctgtttgtctccaagttctttgaacaccacccaataccacaggaggaggcttccttagcagagaccacccttacatctggatcatccccttctgcacccccctcagagtccattgggcccccaattctcaccagcccatctccttcaaaatccattccaattccacagcctttccggccaggagaggaagatcatcgaaatcaatttgggcagcgagaccggtcctcatctgctcccaatgtgcatataaacacaatagaacctgtcaatattgatgatttgattagagaccaagggtttcgtagtgatggaggatcaactacaggtttgtctgccaccccacctgcctcattacctggctcactcactaatgtgaaagccttacagaaatctccaggacctcagcgagaaaggaagtcatcttcatcctcagaagacagaaatcgaatgaaaacgcttggtagacgggactcaagtgatgattgggagattcctgatgggcagattacagtgggacaaagaattggatctgggtcatttggaacagtctacaaggggaagtggcatggtgacgtggcagtgaaaatgttgaatgtgacagcacccacacctcaacagttacaggccttcaaaaatgaagtaggagtactcaggaaaacacgacatgtgaatatcctactcttcatgggctattccacaaagccacagctagctattgttacccagtggtgtgagggctccagcttataccaccatctccacatcatcgagaccaaatttgagatgatcaaacttatagatattgcacgacagactgcccagggcatggattacttacacgccaagtcaatcatccacagagacctcaagagtaataatatatttcttcacgaagacctcacggttaaaataggtgattttggtctagccacagtgaaatctcgatggagtgggtcccatcagtttgaacagttgtctggatccattttgtggatggcaccagaagtaatcagaatgcgagataaaaacccatacagttttcagtccgatgtatatgcatttgggattgttctatatgaattgatgactgggcagttaccctattcaaatatcaacaacagggaccagataatttttatggtgggacgaggatatctatctccagatctcagcaaggtacggagtaactgtccaaaagccatgaagaggttaatggcggagtgcctcaaaaagaaaagagatgagagaccactctttccccaaattctcgcctctattgagctgctggcccgctcattgccaaaaattcaccgcagtgcatcagaaccctccttgaatcgggctggtttccaaacagaggattttagtctctatgcttgtgcttctccaaaaacacccatccaggcagggggatatggtgcgtttcctgtccactgatgcaaattaaatgagtgagaaataaa

SEQ ID NO: 94 - protein, 719 aa, Cavia porcellus
MAALSGGGGAEQGQALFNGDMELEAGAGAAASSAADPAIPEEVWNIKQMIKLTQEHIEALLDKFGGEHNPPSIYLEAYEEYTSKLDALQQREQQLLESLGNGTDFSVSSSASLDTVTSSSSSSLSVLPSSLSVFQNPTDVSRSNPKSPQKPIVRVFLPNKQRTVVPARCGVTVRDSLKKALMMRGLIPECCAVYRIQDGEKKPIGWDTDISWLTGEELHVEVLENVPLTTHNFVCIFIFFLLFVSKFFEHHPIPQEEASLAETTLTSGSSPSAPPSESIGPPILTSPSPSKSIPIPQPFRPGEEDHRNQFGQRDRSSSAPNVHINTIEPVNIDDLIRDQGFRSDGGSTTGLSATPPASLPGSLTNVKALQKSPGPQRERKSSSSSEDRNRMKTLGRRDSSDDWEIPDGQITVGQRIGSGSFGTVYKGKWHGDVAVKMLNVTAPTPQQLQAFKNEVGVLRKTRHVNILLFMGYSTKPQLAIVTQWCEGSSLYHHLHIIETKFEMIKLIDIARQTAQGMDYLHAKSIIHRDLKSNNIFLHEDLTVKIGDFGLATVKSRWSGSHQFEQLSGSILWMAPEVIRMRDKNPYSFQSDVYAFGIVLYELMTGQLPYSNINNRDQIIFMVGRGYLSPDLSKVRSNCPKAMKRLMAECLKKKRDERPLFPQILASIELLARSLPKIHRSASEPSLNRAGFQTEDFSLYACASPKTPIQAGGYGAFPVH

SEQ ID NO: 95 - DNA, 3229 bp, Canis lupus
gtaatgctggattttcatggaataagtttgacctgtgctgcagtggcctccagcaaggtacccgcaagatgtggagttacagtccgggacagtctaaagaaagctctgatgatgagaggtctaatcccagagtgctgtgctgtttacagaattcaggatggagagaagaaaccgattggctgggacactgatatttcctggctcactggagaggaattgcatgtagaagtgttggaaaatgttccgcttaccacacacaactttgtacggaaaacttttttcaccttagcattttgtgacttttgtcgaaagctgcttttccagggttttcgctgtcaaacatgtggttataaatttcaccagcgttgtagtacagaggttccactgatgtgtgttaattatgaccaacttgatttgctgtttgtctccaagttctttgaacaccacccaataccacaggaggaggcctccatagcagagactgcccttacgtctggatcatccccttctgctcccccctccgattctcctgggcccccaattctgaccagtccgtctccttcaaaatccattccaattccacagcctttccgaccagcagatgaagatcatcgaaatcagtttggacaacgagaccggtcctcatcagctccaaatgtgcatataaacacaatagaacccgtcaacattgatgacttgattagagaccaagggtttcgtagtgatggaggatcaaccacaggtttgtctgccaccccccctgcctcattgcctggctcactcactaatgtaaaagcattacagaaatctccaggacctcagcgggaaagaaaatcatcttcatcctcagaagataggaatcgaatgaaaacacttggtagacgggattcaagtgatgattgggagatacctgatgggcagatcacagtgggacagagaattggatccgggtcatttgggacagtctacaagggaaagtggcatggtgacgtggcagtgaaaatgttgaatgtgacagcacccacacctcagcagttacaggccttcaaaaatgaagtaggagtactcaggaaaactcgacatgtgaatatcctactctttatgggctattcaacaaagccccaactggctattgttacccagtggtgtgagggctccagcttatatcaccatctccacatcattgagaccaaatttgagatgataaagcttatagatattgcacggcagactgcacagggcatggattacttacacgccaagtcaatcatccacagagacctcaagagtaataatatttttcttcatgaagacctcacagtaaaaataggtgattttggtctagccacagtgaaatctcgatggagtgggtcccatcagtttgaacagttgtctggatccattttgtggatggcaccagaagtgatccgaatgcaagacaaaaacccatatagcttccagtcagatgtatacgcatttgggattgttctatatgaattgatgacagggcagttaccttattcaaacatcaacaacagggaccagataatttttatggtgggacgaggatatctttctccagatctcagtaaggtacggagtaactgtccaaaagccatgaagagattgatggcagagtgcctaaaaaagaaaagagatgagaggccactctttccccaaattctcgcctctattgagctgctggcccgctcattgccaaaaattcaccgcagtgcatcagaaccctccttgaatcgggctggcttccaaacagaggattttagtctctatgcttgcgcttctccaaaaacacccatccaggcagggggatacggagaatttgcagccttcaagtagccacaccatcatggcaacaactactcttatttcttaagtcttgtgttcgtacaatttgttaacatcaaaacacagttctgttcctcaaatctttttttaaagatacagaattttcaatgcataagctggtgtggaacagaatggaatttcccatccaacaaaagagggaagaatgttttaggaaccagaattctctgctgccagtgtttcttcttcaacacaaataccacgtgcatacaagtctgcccactcccaggaaggaagaggagagcctgagttctgaccttttgatggtcaggcatgatggaaagaaactgctgctacagcttgggagattggctgtggagagcctgcccgtcagctctgcccttctaaccgccagatgagtgtgtggctggtcacctgacagggcagctgcaatcgccaagcatcgttctctttcctgtcctgggattttgtcgtggagctctttccccctagtcaccaccggttcatttctgagggatggaacaaaaatgcagcatggcctttctgtgtggtgcatgtccggtctttgacaaatttttatcaagtgaagctcttgtatttaaatggagaatgagaggcgagggggggggatcacgttttggtgtaggggcaaagggaatgctgcatctttttcctgacccactgggtttctggcctttgtttccttgctcactgagggtgtctgcctataaccacgcaggctggaaagtgctggcacacattgccttctcttctcactgggtccagcaatgaagacaagtgttggggatttttttttttgccctccacaatgtagcaagttctcaggaaaatacagttaatatcttcctcctaagctcttccagtcatcaagtacttatgtggctactttgtccagggcacaaaatgccatggcggtatccaattaaaagcctacaaaactgcttgataacagttttgaatgtgtgagacatttatgtaatttaaatgtaaggtacaagttttaatttctgagtttctctattatatttttattaaaaagaaaataattttcagatttaattgaattggaataaaataatacttcccaccagaattatatatcctggaaaattgtatttttgttatataaacaacttttaaagaaagatcattatccttttctctacctaaatatggggagtcttagcataatgacagatatttataatttttaaattaatggtacttgctggatccacactaacatctttgctaatatctcatgttttcctccaacttactcctacactacatcctccatcctctttccagtcttttatctagaatatgcaacctaaaataaaaatggtggtgtctccattca

SEQ ID NO: 96 - protein, 617 aa, Canis lupus
MLDFHGISLTCAAVASSKVPARCGVTVRDSLKKALMMRGLIPECCAVYRIQDGEKKPIGWDTDISWLTGEELHVEVLENVPLTTHNFVRKTFFTLAFCDFCRKLLFQGFRCQTCGYKFHQRCSTEVPLMCVNYDQLDLLFVSKFFEHHPIPQEEASIAETALTSGSSPSAPPSDSPGPPILTSPSPSKSIPIPQPFRPADEDHRNQFGQRDRSSSAPNVHINTIEPVNIDDLIRDQGFRSDGGSTTGLSATPPASLPGSLTNVKALQKSPGPQRERKSSSSSEDRNRMKTLGRRDSSDDWEIPDGQITVGQRIGSGSFGTVYKGKWHGDVAVKMLNVTAPTPQQLQAFKNEVGVLRKTRHVNILLFMGYSTKPQLAIVTQWCEGSSLYHHLHIIETKFEMIKLIDIARQTAQGMDYLHAKSIIHRDLKSNNIFLHEDLTVKIGDFGLATVKSRWSGSHQFEQLSGSILWMAPEVIRMQDKNPYSFQSDVYAFGIVLYELMTGQLPYSNINNRDQIIFMVGRGYLSPDLSKVRSNCPKAMKRLMAECLKKKRDERPLFPQILASIELLARSLPKIHRSASEPSLNRAGFQTEDFSLYACASPKTPIQAGGYGEFAAFK

SEQ ID NO: 97 - DNA, 1889 bp, Canis lupus
ggaatatcaaacaaatgattaagttgacacaggaacatatagaagccctattggacaagtttggtggggagcataatccaccatcaatatatctggaggcctatgaagaatacaccagcaaactagatgccctccaacagcgagaacaacagttattggaatccctggggaatggaactgatttttctgtttctagctctgcatcaacggacaccgttacatcttcttcctcttctagcctttcagtgctaccttcatctctttcagtttttcaaaatcccacagatatatcacggagcaatcccaagtcaccacaaaaacctatcgttagagtcttcctgcccaataaacagaggacggtggtacccgcaagatgtggagttacagtccgggacagtctaaagaaagctctgatgatgagaggtctaatcccagagtgctgtgctgtttacagaattcaggatggagagaagaaaccgattggctgggacactgatatttcctggctcactggagaggaattgcatgtagaagtgttggaaaatgttccgcttaccacacacaactttgtacggaaaacttttttcaccttagcattttgtgacttttgtcgaaagctgcttttccagggttttcgctgtcaaacatgtggttataaatttcaccagcgttgtagtacagaggttccactgatgtgtgttaattatgaccaacttgatttgctgtttgtctccaagttctttgaacaccacccaataccacaggaggaggcctccatagcagagactgcccttacgtctggatcatccccttctgctcccccctccgattctcctgggcccccaattctgaccagtccgtctccttcaaaatccattccaattccacagcctttccgaccagcagatgaagatcatcgaaatcagtttggacaacgagaccggtcctcatcagctccaaatgtgcatataaacacaatagaacccgtcaacattgatgacttgattagagaccaagggtttcgtagtgatggaggatcaaccacaggtttgtctgccaccccccctgcctcattgcctggctcactcactaatgtaaaagcattacagaaatctccaggacctcagcgggaaagaaaatcatcttcatcctcagaagataggaatcgaatgaaaacacttggtagacgggattcaagtgatgattgggagatacctgatgggcagatcacagtgggacagagaattggatccgggtcatttgggacagtctacaagggaaagtggcatggtgacgtggcagtgaaaatgttgaatgtgacagcacccacacctcagcagttacaggccttcaaaaatgaagtaggagtactcaggaaaactcgacatgtgaatatcctactctttatgggctattcaacaaagccccaactggctattgttacccagtggtgtgagggctccagcttatatcaccatctccacatcattgagaccaaatttgagatgataaagcttatagatattgcacggcagactgcacagggcatggattacttacacgccaagtcaatcatccacagagacctcaagagtaataatatttttcttcatgaagacctcacagtaaaaataggtgattttggtctagccacagtgaaatctcgatggagtgggtcccatcagtttgaacagttgtctggatccattttgtggatggcaccagaagtgatccgaatgcaagacaaaaacccatatagcttccagtcagatgtatacgcatttgggattgttctatatgaattgatgacagggcagttaccttattcaaacatcaacaacagggaccagctcagatcatgatcacggtgtcatgagatcaagccccac

SEQ ID NO: 98 - protein, 615 aa, Canis lupus
MIKLTQEHIEALLDKFGGEHNPPSIYLEAYEEYTSKLDALQQREQQLLESLGNGTDFSVSSSASTDTVTSSSSSSLSVLPSSLSVFQNPTDISRSNPKSPQKPIVRVFLPNKQRTVVPARCGVTVRDSLKKALMMRGLIPECCAVYRIQDGEKKPIGWDTDISWLTGEELHVEVLENVPLTTHNFVRKTFFTLAFCDFCRKLLFQGFRCQTCGYKFHQRCSTEVPLMCVNYDQLDLLFVSKFFEHHPIPQEEASIAETALTSGSSPSAPPSDSPGPPILTSPSPSKSIPIPQPFRPADEDHRNQFGQRDRSSSAPNVHINTIEPVNIDDLIRDQGFRSDGGSTTGLSATPPASLPGSLTNVKALQKSPGPQRERKSSSSSEDRNRMKTLGRRDSSDDWEIPDGQITVGQRIGSGSFGTVYKGKWHGDVAVKMLNVTAPTPQQLQAFKNEVGVLRKTRHVNILLFMGYSTKPQLAIVTQWCEGSSLYHHLHIIETKFEMIKLIDIARQTAQGMDYLHAKSIIHRDLKSNNIFLHEDLTVKIGDFGLATVKSRWSGSHQFEQLSGSILWMAPEVIRMQDKNPYSFQSDVYAFGIVLYELMTGQLPYSNINNRDQLRS

SEQ ID NO: 99 - DNA, 3521 bp, Felis catus
  misc_feature (630)..(649): n is a, c, g, or t
atgcctaacctcagtctctgccaccacggccaatttgctcatgtgcccactgtgtcggcactgggatattttgtgatttgccttggccattgtccactgtccttgacattgcctgaaggagaaccactgatgctaatgttgaaggtgacctttgcaggctctccactactcataccaaagatgcggccccctgataatcccagagccactgtctgcacatgggcaaaacaggctacattctgtgcagactggggagaaaggttccaagaacacagtgccatagttttgggcagagagtttcaacacagcatagtgtctatggcagtatctggatttggccgggggaagtgcccaagaggagacagtcaggctgtgtcctacggccaaggacctgcacttatttttgcatgcagtggtttagcacagggaagagaacgaagtaggaaatcggagccatggaaacggcagagcggaggaaacgtgcacgcgcgagggtgggcacgaaaggaaagaaccctccccagaagactgcgcgagggcgctcctaggattacgtcacgcaccccgcgaaaactgaaatgtactgtgtgtggtcttttaattgaactatcttccttatgtgcacttaannnnnnnnnnnnnnnnnnnngcggcggcggcggtggcgcggagcagggccaggctctgttcaacggggacatggagcccgaagccggcgccgcggcctcttcggctgcggaccctgccattcccgaggaggtgtggaatatcaaacaaatgattaagttgacacaggaacatatagaggccctattggacaaatttggtggggagcataatccaccatcaatatatctagaggcctatgaagaatacaccagcaagctagatgccctccaacagagagaacaacagttattggaatccctggggaatggaactgatttttctgtttctagctctgcatcaacagacaccgttacatcttcctcctcttctagcctttcagtgctaccttcatctctttcagtttttcaaaaccccacagatgtgtcacggagcaatcccaagtcaccacagaaacctatcgttagagtcttcctgcctaataaacagaggacagtggtacctgcaagatgtggagttacagtccgggacagtctaaagaaagctctgatgatgagaggtctaatccctgagtgctgtgctgtttacagaattcaggatggagagaagaaaccaattggctgggacactgatatctcctggctcaccggagaggaattgcatgtagaagtgttggaaaatgttccacttacaactcacaactttgtatgtacggaaaacgttttcaccttagcattttgtgacttttgtcgaaagctgcttttccaaggttttcgctgtcaaacgtgtggttataaatttcaccagcgttgtagtacagaggttccactgatgtgtgttaattatgaccaacttgatttgctgtttgtctccaagttctttgaacaccacccaataccacaggaggaggcctccatagcagagactgccctaacgtctggatcgtccccttctgcccccccctccgattctactgggccccaaattctcaccagtccgtctccttcaaaatccattccaattccacagcctttccgaccagcagatgaagatcatcgaaatcaatttggacagcgagaccggtcctcatcagctccaaatgtgcatataaatacaatagaacctgtcaatattgatgacttgattagagaccaggggtttcgtagtgatggaggatcaaccacaggcttgtctgccaccccccctgcctcattgccgggctctctcactaatgtaaaagcattacagaaatctccagggcctcagcgggaaaggaaatcttcttcatcctcagaagataggaatcgaatgaaaacacttggtagaagggattcaagtgatgattgggagattcctgatgggcagatcacagtgggacagagaattggatccgggtcatttgggacagtctacaagggaaagtggcatggtgatgtggcagtgaaaatgttgaatgtgacagcacccacacctcagcagttacaggccttcaaaaatgaagtaggagtactcaggaaaactcggcatgtgaacatcctgctcttcatgggctattcaacaaagccccagctggctattgtcacccagtggtgtgagggctccagcttataccaccatctccacatcatcgagaccaaattcgagatgatcaagctgatagatattgctcggcagactgcgcagggcatggattacttacacgccaagtcaatcatccacagagacctcaagagtaataatatttttcttcacgaagacctcacagtaaaaataggtgattttggtctagccacagtgaaatctcgatggagtgggtcccatcagtttgaacagttgtctggatccattttgtggatggcaccagaagtaattcgaatgcaagataaaaacccatatagctttcagtcagatgtatatgcatttgggattgttctatatgaattgatgactggacagttaccttattcaaacatcaacaacagggaccagataatttttatggtgggacgaggatatctttctccagatctcagtaaggtacgaagtaactgtccaaaagccatgaagagattgatggcagagtgcctaaaaaagaaaagagatgagaggccactgtttccccaaattcttgcctctattgagctgctggcccgctcattgccaaaaattcaccgcagtgcatcagaaccctccttgaatcgggctggcttccagacagaggattttagtctctatgcttgtgcttctccaaaaacacccatccaggcagggggatatggtgcgtttcccgtccactgagataagttagatgagtgcgcgagtgcagggggccggggccaaggaggtggaaatgtgcgtgcttctgtactaagttggatagcatcttcttttttaaaaaaagatgaaccaaagaatgtgtatgtttttaaagactagatataattatttcctgatctaaaatgtatacttagctttggattttcaatatccaagggttttcaaaatgcacagacattgctgaacatttgcagtacctcttctggaggctttacttcctgttacaaattggttttgtttactggcttatcctaattattaaacttcaattaaacttttctcctgcaccttttgttatgagctatcacatgtcccttagggactcgcaagagcagtactgcccccgtgtacgggcttgcaggtagaaaggggatgacgggttttaacacctgtgtgaggcaaggcagtccgaacagatctcatttaggaagccacgagagttgaataagttatttttattcttagtattttttctgtaactactttttattataacttggaaaatatggatgtcctttatacaccttagcaatagactgaatttctttttataaatt

SEQ ID NO: 100 - protein, 974 aa, Felis catus
  misc_feature (210)..(217): Xaa can be any naturally occurring amino acid
MPNLSLCHHGQFAHVPTVSALGYFVICLGHCPLSLTLPEGEPLMLMLKVTFAGSPLLIPKMRPPDNPRATVCTWAKQATFCADWGERFQEHSAIVLGREFQHSIVSMAVSGFGRGKCPRGDSQAVSYGQGPALIFACSGLAQGRERSRKSEPWKRQSGGNVHARGWARKERTLPRRLREGAPRITSRTPRKLKCTVCGLLIELSSLCALXXXXXXXXGGGGGAEQGQALFNGDMEPEAGAAASSAADPAIPEEVWNIKQMIKLTQEHIEALLDKFGGEHNPPSIYLEAYEEYTSKLDALQQREQQLLESLGNGTDFSVSSSASTDTVTSSSSSSLSVLPSSLSVFQNPTDVSRSNPKSPQKPIVRVFLPNKQRTVVPARCGVTVRDSLKKALMMRGLIPECCAVYRIQDGEKKPIGWDTDISWLTGEELHVEVLENVPLTTHNFVCTENVFTLAFCDFCRKLLFQGFRCQTCGYKFHQRCSTEVPLMCVNYDQLDLLFVSKFFEHHPIPQEEASIAETALTSGSSPSAPPSDSTGPQILTSPSPSKSIPIPQPFRPADEDHRNQFGQRDRSSSAPNVHINTIEPVNIDDLIRDQGFRSDGGSTTGLSATPPASLPGSLTNVKALQKSPGPQRERKSSSSSEDRNRMKTLGRRDSSDDWEIPDGQITVGQRIGSGSFGTVYKGKWHGDVAVKMLNVTAPTPQQLQAFKNEVGVLRKTRHVNILLFMGYSTKPQLAIVTQWCEGSSLYHHLHIIETKFEMIKLIDIARQTAQGMDYLHAKSIIHRDLKSNNIFLHEDLTVKIGDFGLATVKSRWSGSHQFEQLSGSILWMAPEVIRMQDKNPYSFQSDVYAFGIVLYELMTGQLPYSNINNRDQIIFMVGRGYLSPDLSKVRSNCPKAMKRLMAECLKKKRDERPLFPQILASIELLARSLPKIHRSASEPSLNRAGFQTEDFSLYACASPKTPIQAGGYGAFPVH

SEQ ID NO: 101 - DNA, 3853 bp, Bos taurus
ctcagctgcgccgggtctcacaagacggttcccgaggtggcccaggcgccgtcccaccgccgacgccgcccgggccgcccgggccgtccctccccgctgccccccgtcctccgcctccgcctccccccgccctcagcctcccttccccctccccgcccagcagcggtcgctcgggcccggctctcggttataagatggcggcgctgagtggcggcggcggcggcggcggcggtggcgcggagcagggccaggctctgttcaacggggacatggagcccgaggccggcgccgcggcctcttcggctgcggaccccgccattcccgaggaggtgtggaatatcaaacaaatgattaagttgacacaggagcatatagaggccctattggacaaatttggtggggagcataatccaccatcaatatatctggaggcctatgaagaatacaccagcaagctagatgccctccaacaaagagaacaacagttattggaatccctggggaatggaactgatttttctgtttctagctctgcatcaacggacaccgttacatcttcttcctcttctagcctttcagtgctgccttcatctctttcagtttttcaaaatcccacagatgtgtcacggagcaaccccaagtcaccacaaaaacctatcgttagagtcttcctgcccaataaacagaggacagtggtacctgcacggtgtggagtcacagtccgggacagcctgaagaaggcactgatgatgagaggtctaatcccagagtgctgtgctgtttacagaattcaggatggggagaagaaaccaattggctgggacactgatatttcctggcttactggagaggagttgcatgtagaagtgttggagaatgttccacttacaacacacaactttgtacggaaaacttttttcaccttagcattttgtgacttctgtagaaagctgcttttccagggattccgctgtcaaacatgtggttataaatttcaccagcgttgtagtacagaggttccactgatgtgtgttaattatgaccaactagatttgctgtttgtctccaagttctttgaacaccacccaataccacaggaggaggcctccttagcagagactacccttccatgtggctcatccccttctgcacccccctccgattctattgggcccccaattctcaccagtccatctccttcaaaatccattccaattccacagcctttccgaccagcagatgaagatcatcgaaatcagtttggacaacgagaccggtcctcatcagctccaaatgtgcatataaacacaatagaacccgtcaatattgatgacttgattagagaccaagggtttcgtagtgatggaggatcaaccacaggtttatccgccacaccccctgcctcattacctggctcactctctaatgtgaaagcattgcagaaatctccaggacctcagcgagaaagaaagtcctcttcatcctcagaagacaggaatcgaatgaaaacgcttggtagacgggattcaagtgacgattgggagattcctgatggacagatcacagtgggacaaagaattggatcagggtcatttgggacagtctacaagggaaagtggcatggtgatgtggcagtgaaaatgttgaatgtgacagcacccacacctcagcagttacaggccttcaaaaatgaagtaggagtactcaggaaaacgcgacatgtgaatatcctcctcttcatgggttattcaacaaagccacaactggctattgttacccagtggtgtgagggctccagtttatatcatcatctccacatcattgagaccaaattcgagatgatcaaacttatagatattgcacggcagactgcacagggcatggattacttacacgccaagtcaatcatccacagagacctcaagagtaataatatttttcttcatgaagacctcacagtaaaaataggtgattttggtctagccacagtgaaatctcgatggagtgggtcccatcagtttgaacagttgtctggatccattttgtggatggcaccagaagtaatcagaatgcaagataaaaacccatatagctttcagtcagatgtatatgcatttgggattgttctgtatgaattgatgaccggacagttaccttattcaaatatcaacaacagggaccagataatttttatggtgggacgaggatatctgtctccagatctcagtaaggtacggagtaactgtccaaaagccatgaagagattaatggcagagtgcctaaaaaagaaaagagatgaaagaccactctttccccaaattctcgcctctattgagctgctggcccgctcattgccaaaaattcaccgcagtgcatcagaaccctccttgaatcgggctggcttccaaacagaggattttagtctatatgcttgtgcttctccaaaaacacccattcaggcagggggatatggtacgtttcctgttcactgaaacaaaccgagtgagtgacagcatgtaggagggtagggacaaaagaaagtgaacaaatgtttgcttatatatttgttaaattgaataggattttctttttctttaaaggtgaacaagagaacatgtgtgtttttaaagtttggatatagttttcttcccagtctaaaacccatagttagcattacattttcaacatcgaatttttttttaattcatagacattgctgaaaatttataataccttttccagaggctttacttcccattccaagtttgttttgtttacttggttagtctaatcattaaactttaaactttccccacctaccttttgctgttagctatcccgcatccattaggggctccaagaacagcactgtctgcgtgtgtgtgttggcaggtgggaagctgatggtaagttaggctgtgttagtgaaggtaaactgaccaggtctaattaggagtcactagaattgaataagcttatttttattaatattttttcttataactatttctttttgtaataatttagaaaatataattgttctttattcccttacagcagtataaattattggtgcaggtaaccaaagatattactgaggagtggcatgtttgacatgagtgacatggtttaactttggatttttagttaatatttctttatatattaaggatgtcttacacattatagaagtcaaatttactgacaaaggtattgcctcctcttcctccccaaaaacacagcaaaattctctgggaactcgtagcattgttggttttcttttggatgactatggttgccaaacaaccaagtaattgattttttttaaattattattgctttagattatactcacctctcatgatgcctgttagcaatcacctttatccatgtgtcttgtaaaatatctttcctccttatattctttgcccaacaagagtctacttgttatgaatgagtactattttctttttttgattccccagtataattagtatgtttagtgctttctaggacttccactttcttatgttaaaaaaaaaaacaaactaatgtggcagtcagtatattcttactgtgaatcagagtctttactgggaatcaaagtgaaagaagcagctgttctgacttcagagtcagcctagggaccaaaaccagcctcttaaatacaccttcatttattcagtttggatttgtgatgattttcattatagctgacagttcaaggttattcagtggcacacagatagcatctgcataaatgcctttcttcttgaaaataaaggagaaaattgggaagactttacaccaatagtttagtctttaagtaccacagataacacacaccataaat

SEQ ID NO: 102 - protein, 764 aa, Bos taurus
AALSGGGGGGGGGAEQGQALFNGDMEPEAGAAASSAADPAIPEEVWNIKQMIKLTQEHIEALLDKFGGEHNPPSIYLEAYEEYTSKLDALQQREQQLLESLGNGTDFSVSSSASTDTVTSSSSSSLSVLPSSLSVFQNPTDVSRSNPKSPQKPIVRVFLPNKQRTVVPARCGVTVRDSLKKALMMRGLIPECCAVYRIQDGEKKPIGWDTDISWLTGEELHVEVLENVPLTTHNFVRKTFFTLAFCDFCRKLLFQGFRCQTCGYKFHQRCSTEVPLMCVNYDQLDLLFVSKFFEHHPIPQEEASLAETTLPCGSSPSAPPSDSIGPPILTSPSPSKSIPIPQPFRPADEDHRNQFGQRDRSSSAPNVHINTIEPVNIDDLIRDQGFRSDGGSTTGLSATPPASLPGSLSNVKALQKSPGPQRERKSSSSSEDRNRMKTLGRRDSSDDWEIPDGQITVGQRIGSGSFGTVYKGKWHGDVAVKMLNVTAPTPQQLQAFKNEVGVLRKTRHVNILLFMGYSTKPQLAIVTQWCEGSSLYHHLHIIETKFEMIKLIDIARQTAQGMDYLHAKSIIHRDLKSNNIFLHEDLTVKIGDFGLATVKSRWSGSHQFEQLSGSILWMAPEVIRMQDKNPYSFQSDVYAFGIVLYELMTGQLPYSNINNRDQIIFMVGRGYLSPDLSKVRSNCPKAMKRLMAECLKKKRDERPLFPQILASIELLARSLPKIHRSASEPSLNRAGFQTEDFSLYACASPKTPIQAGGYGTFPVH

SEQ ID NO: 103 - DNA, 4936 bp, Bos taurus
ctcagctgcgccgggtctcacaagacggttcccgaggtggcccaggcgccgtcccaccgccgacgccgcccgggccgcccgggccgtccctccccgctgccccccgtcctccgcctccgcctccccccgccctcagcctcccttccccctccccgcccagcagcggtcgctcgggcccggctctcggttataagatggcggcgctgagtggcggcggcggcggcggcggcggtggcgcggagcagggccaggctctgttcaacggggacatggagcccgaggccggcgccgcggcctcttcggctgcggaccccgccattcccgaggaggtgtggaatatcaaacaaatgattaagttgacacaggagcatatagaggccctattggacaaatttggtggggagcataatccaccatcaatatatctggaggcctatgaagaatacaccagcaagctagatgccctccaacaaagagaacaacagttattggaatccctggggaatggaactgatttttctgtttctagctctgcatcaacggacaccgttacatcttcttcctcttctagcctttcagtgctgccttcatctctttcagtttttcaaaatcccacagatgtgtcacggagcaaccccaagtcaccacaaaaacctatcgttagagtcttcctgcccaataaacagaggacagtggtacctgcacggtgtggagtcacagtccgggacagcctgaagaaggcactgatgatgagaggtctaatcccagagtgctgtgctgtttacagaattcaggatggggagaagaaaccaattggctgggacactgatatttcctggcttactggagaggagttgcatgtagaagtgttggagaatgttccacttacaacacacaactttgtacggaaaacttttttcaccttagcattttgtgacttctgtagaaagctgcttttccagggattccgctgtcaaacatgtggttataaatttcaccagcgttgtagtacagaggttccactgatgtgtgttaattatgaccaactagatttgctgtttgtctccaagttctttgaacaccacccaataccacaggaggaggcctccttagcagagactacccttccatgtggctcatccccttctgcacccccctccgattctattgggcccccaattctcaccagtccatctccttcaaaatccattccaattccacagcctttccgaccagcagatgaagatcatcgaaatcagtttggacaacgagaccggtcctcatcagctccaaatgtgcatataaacacaatagaacccgtcaatattgatgacttgattagagaccaagggtttcgtagtgatggaggatcaaccacaggtttatccgccacaccccctgcctcattacctggctcactctctaatgtgaaagcattgcagaaatctccaggacctcagcgagaaagaaagtcctcttcatcctcagaagacaggaatcgaatgaaaacgcttggtagacgggattcaagtgacgattgggagattcctgatggacagatcacagtgggacaaagaattggatcagggtcatttgggacagtctacaagggaaagtggcatggtgatgtggcagtgaaaatgttgaatgtgacagcacccacacctcagcagttacaggccttcaaaaatgaagtaggagtactcaggaaaacgcgacatgtgaatatcctcctcttcatgggttattcaacaaagccacaactggctattgttacccagtggtgtgagggctccagtttatatcatcatctccacatcattgagaccaaattcgagatgatcaaacttatagatattgcacggcagactgcacagggcatggattacttacacgccaagtcaatcatccacagagacctcaagagtaataatatttttcttcatgaagacctcacagtaaaaataggtgattttggtctagccacagtgaaatctcgatggagtgggtcccatcagtttgaacagttgtctggatccattttgtggatggcaccagaagtaatcagaatgcaagataaaaacccatatagctttcagtcagatgtatatgcatttgggattgttctgtatgaattgatgaccggacagttaccttattcaaatatcaacaacagggaccagataatttttatggtgggacgaggatatctgtctccagatctcagtaaggtacggagtaactgtccaaaagccatgaagagattaatggcagagtgcctaaaaaagaaaagagatgaaagaccactctttccccaagtaggaaagactctcctaagcaagagacaaaattcagaagttatcagggaaaaagataagcagattctcgcctctattgagctgctggcccgctcattgccaaaaattcaccgcagtgcatcagaaccctccttgaatcgggctggcttccaaacagaggattttagtctatatgcttgtgcttctccaaaaacacccattcaggcagggggatatgaagcagatttggctcttacatcaaataaaaatagagtagaagttgggatttagagatttcctgacatgcaagaaggaataagcaagaaaaaaaggtttgttttccccaaatcatatctattgtcttttacttctattttttcttaaattttttgtgatttcagagacatgtagagttttattgatacctaaactatgagttcttttttttttttttttttcattattttgatttttttggccaagaggcatatgggatcttagcttgagaaagcaacaattttcttgatgtcattttgggtgagggcacatattgctgtgaacagtgtggtgatagccaccagggaccaaactcacacccgctgcattgaaaggtgaagtcttaaacactggaccagcagagaaattcctactctatgagttctttttgtcatcccctccccgcaccctccacccccaacctaaagtctgatgatgaaatcaacaactattccattagaagcagtagattctggtagcatgatctttagtttgttagtaagattttgtgctttgtggggttgtgtcgttttaaggctaatatttaagtttgtcaaatagaatgctgttcagattgtaaaaatgagtaataaacatctgaagttttttttaagttatttttaacatggtatatacagttgagcttagagtttatcattttctgatattctcttacttagtagatgaattctagccattttttataaagatttctgttaagcaaatcctgttttcacatgggcttcctttaagggattttagattctgctggatatggtgactgctcataagactgttgaaaattacttttaagatgtattagaatacttctgaaaaaaaatagcaaccttaaaaccataagcaaaagtagtaagggtgtttatacatttctagagtccctgtttaggtaatagcctcctatgattgtactttaaatgttttgctctccaaggttttagtaacttggctttttttctaatcagtgccaaactcccccagtttttttaactttaaatatgaggtaataaatcttttacccttccttgatcttttgacttataataccttggtcagttgtttcttaaaaggaatccttaaatggaaagagacaatatcactgtctgcagttctgattagtagttttattcagaatggaaaaacagattattcatttttgaaaattgttcaggggtatgttcattgttaggaccttggactttggagtcagtgcctagctatgcattccaggtctgccattttctggctgtgaaattttggacaagttacttaaccactttaaaccccagctttaagaagtaaattaaccccagtaaattaagaagtaatagcagccacttcgtagagttgttatgaggctcagatgcagtgcaaatgtgtataaagtattcagggagtcacctggtatactataatagacactagaatagttgccaatattatcagcatacaatctgaggattctgtcagccaatcattagcaatctgttgtttgttgggacatgccagtgttctccagttgaaatcagtagcaatctaaaaatggatagattattcctcatttaaatagtgtgttcatataagtgattgcttggatccttatcagaagttgctgttactgaaaaatgataaggctgactaaattgtgatagttgtcagttactaaccaactcccagaaatgaataagaggaacctatctctagttcctagtagaaggtatggacaaaatagtaggtgaaaaataatgtcttgaacccccaaattaagtaagctttaaagagtacaatacctcaaagggtctttgcggtttaaaatttgtatgctgagaatgatgttcattgacatgtgcctatatgtaattttttgatagtttaaaaggtgaaatgaactacagatgggagaggtctgaattttcttgccttcagtcaaatgtgtaatgtggacatattatttgacctgtgaattttatcttttaaaaaagattaattcctgcttcttccttcctaatagttgcattataataatgaaaatgagttgataatttggggggaaagtattctacaaatcaaccttattattttaccattggtttctgagaaattttgttcatttgaaccgtttatagcttgattagaatcatagcatgtaaaacccaactgagggattatctgcagacttaatgtagtattatgtaagttgtcttctttcatttcgaccttttttgcttttgttgttgctagatctgtagtatgtagctagtcacctttcagcgaggtttcagcgaggcttttctgtgtctctaggttatttgagataacttttttaaaattagctcttgtcctcc

SEQ ID NO: 104 - protein, 797 aa, Bos taurus
MAALSGGGGGGGGGAEQGQALFNGDMEPEAGAAASSAADPAIPEEVWNIKQMIKLTQEHIEALLDKFGGEHNPPSIYLEAYEEYTSKLDALQQREQQLLESLGNGTDFSVSSSASTDTVTSSSSSSLSVLPSSLSVFQNPTDVSRSNPKSPQKPIVRVFLPNKQRTVVPARCGVTVRDSLKKALMMRGLIPECCAVYRIQDGEKKPIGWDTDISWLTGEELHVEVLENVPLTTHNFVRKTFFTLAFCDFCRKLLFQGFRCQTCGYKFHQRCSTEVPLMCVNYDQLDLLFVSKFFEHHPIPQEEASLAETTLPCGSSPSAPPSDSIGPPILTSPSPSKSIPIPQPFRPADEDHRNQFGQRDRSSSAPNVHINTIEPVNIDDLIRDQGFRSDGGSTTGLSATPPASLPGSLSNVKALQKSPGPQRERKSSSSSEDRNRMKTLGRRDSSDDWEIPDGQITVGQRIGSGSFGTVYKGKWHGDVAVKMLNVTAPTPQQLQAFKNEVGVLRKTRHVNILLFMGYSTKPQLAIVTQWCEGSSLYHHLHIIETKFEMIKLIDIARQTAQGMDYLHAKSIIHRDLKSNNIFLHEDLTVKIGDFGLATVKSRWSGSHQFEQLSGSILWMAPEVIRMQDKNPYSFQSDVYAFGIVLYELMTGQLPYSNINNRDQIIFMVGRGYLSPDLSKVRSNCPKAMKRLMAECLKKKRDERPLFPQVGKTLLSKRQNSEVIREKDKQILASIELLARSLPKIHRSASEPSLNRAGFQTEDFSLYACASPKTPIQAGGYEADLALTSNKNRVEVGI

SEQ ID NO: 105 - DNA, 4154 bp, Bos taurus
ctcagctgcgccgggtctcacaagacggttcccgaggtggcccaggcgccgtcccaccgccgacgccgcccgggccgcccgggccgtccctccccgctgccccccgtcctccgcctccgcctccccccgccctcagcctcccttccccctccccgcccagcagcggtcgctcgggcccggctctcggttataagatggcggcgctgagtggcggcggcggcggcggcggcggtggcgcggagcagggccaggctctgttcaacggggacatggagcccgaggccggcgccgcggcctcttcggctgcggaccccgccattcccgaggaggtgtggaatatcaaacaaatgattaagttgacacaggagcatatagaggccctattggacaaatttggtggggagcataatccaccatcaatatatctggaggcctatgaagaatacaccagcaagctagatgccctccaacaaagagaacaacagttattggaatccctggggaatggaactgatttttctgtttctagctctgcatcaacggacaccgttacatcttcttcctcttctagcctttcagtgctgccttcatctctttcagtttttcaaaatcccacagatgtgtcacggagcaaccccaagtcaccacaaaaacctatcgttagagtcttcctgcccaataaacagaggacagtggtacctgcacggtgtggagtcacagtccgggacagcctgaagaaggcactgatgatgagaggtctaatcccagagtgctgtgctgtttacagaattcaggatggggagaagaaaccaattggctgggacactgatatttcctggcttactggagaggagttgcatgtagaagtgttggagaatgttccacttacaacacacaactttgtacggaaaacttttttcaccttagcattttgtgacttctgtagaaagctgcttttccagggattccgctgtcaaacatgtggttataaatttcaccagcgttgtagtacagaggttccactgatgtgtgttaattatgaccaactagatttgctgtttgtctccaagttctttgaacaccacccaataccacaggaggaggcctccttagcagagactacccttccatgtggctcatccccttctgcacccccctccgattctattgggcccccaattctcaccagtccatctccttcaaaatccattccaattccacagcctttccgaccagcagatgaagatcatcgaaatcagtttggacaacgagaccggtcctcatcagctccaaatgtgcatataaacacaatagaacccgtcaatattgatgacttgattagagaccaagggtttcgtagtgatggaggatcaaccacaggtttatccgccacaccccctgcctcattacctggctcactctctaatgtgaaagcattgcagaaatctccaggacctcagcgagaaagaaagtcctcttcatcctcagaagacaggaatcgaatgaaaacgcttggtagacgggattcaagtgacgattgggagattcctgatggacagatcacagtgggacaaagaattggatcagggtcatttgggacagtctacaagggaaagtggcatggtgatgtggcagtgaaaatgttgaatgtgacagcacccacacctcagcagttacaggccttcaaaaatgaagtaggagtactcaggaaaacgcgacatgtgaatatcctcctcttcatgggttattcaacaaagccacaactggctattgttacccagtggtgtgagggctccagtttatatcatcatctccacatcattgagaccaaattcgagatgatcaaacttatagatattgcacggcagactgcacagggcatggattacttacacgccaagtcaatcatccacagagacctcaagagtaataatatttttcttcatgaagacctcacagtaaaaataggtgattttggtctagccacagtgaaatctcgatggagtgggtcccatcagtttgaacagttgtctggatccattttgtggatggcaccagaagtaatcagaatgcaagataaaaacccatatagctttcagtcagatgtatatgcatttgggattgttctgtatgaattgatgaccggacagttaccttattcaaatatcaacaacagggaccagataatttttatggtgggacgaggatatctgtctccagatctcagtaaggtacggagtaactgtccaaaagccatgaagagattaatggcagagtgcctaaaaaagaaaagagatgaaagaccactctttccccaagtaggaaagactctcctaagcaagagacaaaattcagaagttatcagggaaaaagataagcagattctcgcctctattgagctgctggcccgctcattgccaaaaattcaccgcagtgcatcagaaccctccttgaatcgggctggcttccaaacagaggattttagtctatatgcttgtgcttctccaaaaacacccattcaggcagggggatatggctgagcacattgtccatcacccacaagtggctggttctcatcgcagaatctacgtagggaatcgggcgtgaaattcacttaagagatagagcagaggaagtgttctgtttacaggaatggagatgagagttatgagtaagttgcttagtcagttggctttgttttgaaaattattgtgttatatttgtgttaacctacttgtgttttgacagtatatgtcacataggaagaaacctcagactagcataataacaaagctcagactaggcacagatgtacacagaatggaccaaaatgggatgggggaaggtatgggaataagtctaggggtagggaaaaattgatgtgagggtgggaaataaactgtaattacctgaaataaaatgtaagagtgcaataagtgtgctttttattctaagctgtgaatgggttttttaaaaaaagcattccttcccaatgcatttgcctatgttccatagctgattaaaaccagctatataaacatatgcctttttattcatgttaattaccaatataaatggctaacctttacgtcttatttatcttcatgttatgttagtttacatacagggatgtgtgtgtgtgtgtatgctataaattttccctccttcgtttaaaaacgcgtttgttggatcctctctgtttccttaggccatgccacagctcatagtctcagcttggccttcctgtcacctgatctgaaggactatcacagtgacgtagctcgttcattggttgtacacactctaacccttttccttgctcagcaattactgtgtcttctaaaacaggagtgtacaaccatgagattgcaattaattgtttgacatatgtccctttgaattctatttattagttatgattgattgctctttggtttggaccaagaaaaacgaaatcccacctccccaccttttcacttatttcttactttgaggacaattctgtaagagagaggaaagggaactccttcatgttttaactgcagcaagttaatggccctggtttacaccaaacattatggtgattcacattcacattcctctcctctcttgctgccagaggtttgggttttgttcagttctgctcaagcactgaaaaagttttcatggagtctggagagtgcccagtgaaaagatggtttttaattgtccacagacctttctgttcctgctttgcaaaaattacaaaggagtaactatttttaaagcttatttttcaattcataaaaaagacatttattttcagtcagatgatgtctccttgtcccttaatcctcaatgtttgcttgaatcttttttttttttctgattttctcccatccccacttcttgatacttcttgagttctctttcctgctcaggtcctttcatttgtactttggagttttttctcatgtaaatttgtacaatggaaaatattgttcagtttggatagaacgcatggagaattaaataaaaaagatagctgaaattcagattgaaatttatttgtgtaaagttatttaaaaactctgtactatataaaaggcaaaaaaagttctatgtacttgatgtgaatatgcgaatactgctataataaagattgactgcatgga

SEQ ID NO: 106 - protein, 781 aa, Bos taurus
MAALSGGGGGGGGGAEQGQALFNGDMEPEAGAAASSAADPAIPEEVWNIKQMIKLTQEHIEALLDKFGGEHNPPSIYLEAYEEYTSKLDALQQREQQLLESLGNGTDFSVSSSASTDTVTSSSSSSLSVLPSSLSVFQNPTDVSRSNPKSPQKPIVRVFLPNKQRTVVPARCGVTVRDSLKKALMMRGLIPECCAVYRIQDGEKKPIGWDTDISWLTGEELHVEVLENVPLTTHNFVRKTFFTLAFCDFCRKLLFQGFRCQTCGYKFHQRCSTEVPLMCVNYDQLDLLFVSKFFEHHPIPQEEASLAETTLPCGSSPSAPPSDSIGPPILTSPSPSKSIPIPQPFRPADEDHRNQFGQRDRSSSAPNVHINTIEPVNIDDLIRDQGFRSDGGSTTGLSATPPASLPGSLSNVKALQKSPGPQRERKSSSSSEDRNRMKTLGRRDSSDDWEIPDGQITVGQRIGSGSFGTVYKGKWHGDVAVKMLNVTAPTPQQLQAFKNEVGVLRKTRHVNILLFMGYSTKPQLAIVTQWCEGSSLYHHLHIIETKFEMIKLIDIARQTAQGMDYLHAKSIIHRDLKSNNIFLHEDLTVKIGDFGLATVKSRWSGSHQFEQLSGSILWMAPEVIRMQDKNPYSFQSDVYAFGIVLYELMTGQLPYSNINNRDQIIFMVGRGYLSPDLSKVRSNCPKAMKRLMAECLKKKRDERPLFPQVGKTLLSKRQNSEVIREKDKQILASIELLARSLPKIHRSASEPSLNRAGFQTEDFSLYACASPKTPIQAGGYG

SEQ ID NO: 107 - DNA, 7914 bp, Bos taurus
ctcagctgcgccgggtctcacaagacggttcccgaggtggcccaggcgccgtcccaccgccgacgccgcccgggccgcccgggccgtccctccccgctgccccccgtcctccgcctccgcctccccccgccctcagcctcccttccccctccccgcccagcagcggtcgctcgggcccggctctcggttataagatggcggcgctgagtggcggcggcggcggcggcggcggtggcgcggagcagggccaggctctgttcaacggggacatggagcccgaggccggcgccgcggcctcttcggctgcggaccccgccattcccgaggaggtgtggaatatcaaacaaatgattaagttgacacaggagcatatagaggccctattggacaaatttggtggggagcataatccaccatcaatatatctggaggcctatgaagaatacaccagcaagctagatgccctccaacaaagagaacaacagttattggaatccctggggaatggaactgatttttctgtttctagctctgcatcaacggacaccgttacatcttcttcctcttctagcctttcagtgctgccttcatctctttcagtttttcaaaatcccacagatgtgtcacggagcaaccccaagtcaccacaaaaacctatcgttagagtcttcctgcccaataaacagaggacagtggtacctgcacggtgtggagtcacagtccgggacagcctgaagaaggcactgatgatgagaggtctaatcccagagtgctgtgctgtttacagaattcaggatggggagaagaaaccaattggctgggacactgatatttcctggcttactggagaggagttgcatgtagaagtgttggagaatgttccacttacaacacacaactttgtacggaaaacttttttcaccttagcattttgtgacttctgtagaaagctgcttttccagggattccgctgtcaaacatgtggttataaatttcaccagcgttgtagtacagaggttccactgatgtgtgttaattatgaccaactagatttgctgtttgtctccaagttctttgaacaccacccaataccacaggaggaggcctccttagcagagactacccttccatgtggctcatccccttctgcacccccctccgattctattgggcccccaattctcaccagtccatctccttcaaaatccattccaattccacagcctttccgaccagcagatgaagatcatcgaaatcagtttggacaacgagaccggtcctcatcagctccaaatgtgcatataaacacaatagaacccgtcaatattgatgacttgattagagaccaagggtttcgtagtgatggaggatcaaccacaggtttatccgccacaccccctgcctcattacctggctcactctctaatgtgaaagcattgcagaaatctccaggacctcagcgagaaagaaagtcctcttcatcctcagaagacaggaatcgaatgaaaacgcttggtagacgggattcaagtgacgattgggagattcctgatggacagatcacagtgggacaaagaattggatcagggtcatttgggacagtctacaagggaaagtggcatggtgatgtggcagtgaaaatgttgaatgtgacagcacccacacctcagcagttacaggccttcaaaaatgaagtaggagtactcaggaaaacgcgacatgtgaatatcctcctcttcatgggttattcaacaaagccacaactggctattgttacccagtggtgtgagggctccagtttatatcatcatctccacatcattgagaccaaattcgagatgatcaaacttatagatattgcacggcagactgcacagggcatggattacttacacgccaagtcaatcatccacagagacctcaagagtaataatatttttcttcatgaagacctcacagtaaaaataggtgattttggtctagccacagtgaaatctcgatggagtgggtcccatcagtttgaacagttgtctggatccattttgtggatggcaccagaagtaatcagaatgcaagataaaaacccatatagctttcagtcagatgtatatgcatttgggattgttctgtatgaattgatgaccggacagttaccttattcaaatatcaacaacagggaccagataatttttatggtgggacgaggatatctgtctccagatctcagtaaggtacggagtaactgtccaaaagccatgaagagattaatggcagagtgcctaaaaaagaaaagagatgaaagaccactctttccccaaattctcgcctctattgagctgctggcccgctcattgccaaaaattcaccgcagtgcatcagaaccctccttgaatcgggctggcttccaaacagaggattttagtctatatgcttgtgcttctccaaaaacacccattcaggcagggggatatggagaatttgcagccttcaagtagccacaccatcatgacagcatctactcttatttcttaagtcttgtgttcgtacaatttgttaacatcaaaacacagttctgttcctcaactctttttaaagttaaaatttttcagtgcataagctggtgtggaacagaaggaaatttcccatccaacaaaagagggaagaatgttttaggaaccagaattctctgctgccagtgtttcttcttcaacacaaatatcacaagtctgcccactcccaggaagaaagaggagagaccctgagttctgaccttttgatggtcaggcatgatggaaagaaactgctgctacagcttgggagatttgctctgggaagtctgccagtcaactttgcccttctaaccaccagatcaatatgtggctgatcatctgatggggcagttgcaatcaccaagccttgttctctttcctgttctgggattgtgttgtggaacccttttccctagccaccaccagttcatttctgagggatggaacaaaaatgcagcatgcccttcctgtgtggtgcatgttcagtccttgacaaatttttaccaaaatgaagctactttatttaaaaggagggtgagaggtgaggaggtcactttgggtgtggcggaaagggaatgctgcatctttttcctgggctgctggggctctggccttggcttgccagccggaagcgctggcacgcatcgccttcttttcccattgggtccagcaatgaagacgagtgtttggggttttttttttctccaccatgtagcaagttctcaggaaaatacaattgatatcttcctcctaagctcttccaatcagtcaccaagtacttatgtggttactttgtccagggcacaaaatgcctgtatctaattaaaagcctacaaaactgcttgataacagttttgaatgtgagacatttatgtaatttaaatgtaaggtacaagttttaatttctgagtttcttctattatatttttattaaaaaaagaaaataattttcagattgaattggagtaaaataatattacttcccactagaattatatatcctggaaaattgtatttttgttacataagcagcttttaaagaaagatcattacccttttctctacataaatatatggggagtcttagcctaatgacaaatatttataatttttaaattaatggtacttgctggatccatactaacatctttactaatacctcattgtttcttccaacttactcctacactacatcctacatcttcttcctagtcttttatctagaatatgcaacctcaaataaaaatggtggtgtcctcattcattctcctccttccttttttcccaagcctgatcttcaaaaggttggttaatttggcagctgagttcctccccaggcagagaatagaccaattttaggtgtattgggactgagggaggatgtgtaaagattaacatcagtaaagaaccgctgtggagtaattaagaactttgttctttataactggagaatataacctaaccctaacatccctcagcctttactaaagtgtggcgtaaatcacagtagtagcaaagaaagtgactctggatgtgttcctggccagtacctcccttatcatgaatgtagactctctcatcaagatttaggaatataaatcaaatcaaatgtgcccagccaagctatgtagtaagggacttgaacaatattaggcagaacctataaaataaatcagggaattagaaattatttaaagttttcaaattgtaaattgccccggtgtctttcagcctactgccattatttttgctacaatacctacatttcagaggagggcctactgaaaattccatgcaagtggaaaataatcctcaagttattaatgagtttgaaaagcaatgagttcttaagtctttgtgagtagagcaagatcctacaaaattcagaaatagtaaaaatggattcatgctgatttgaagagcatctgtgtgcataatataatgctgcatctcttttaaaagcagtctatttttctttttaaatttgtccccatagatgcttttgaacatgaacatgcttatgttaccttttccgaggttgggaagagccaggagctctcaggcagggccccctccctcagctgggcaggagctgctcaggaggagctagttatagaggaagcttagcgttggcattttcaaaattcaaggtgataacgctttcttcttcctttctgttttagaatagattgctgtctgatttgaaaaagggaaatagatttgatctcaaatgaatctgtgcccagaagccaggctcagggtattcagagatttgtatagtgccctcaaaaaataacaaaattttagctttccttttttcttcttttctccatcaaattcttttttctctagtttacaaatgacatggaaaaggaatttcccctgagttttgtatgcctttttttttttggcttagactatagataggcgtgttgagctcctaagaaaatacaaggaggaactctttgttgtgcagagcactttatgagtagtttgtgtggataatatgtgactgcttccctgacgagcttgtgaggctgtacttatgtctttcctgtaaggcagcttcagtgccttctgtagtgtatataaggaaagattacgccttctgaaaaatctcagagcaaccataagattattttaaaatatgtagtatgactgatggactttttcatcattaaattagtctagcatctaaacttttaccactgaaataatattgaccaaaaagcaatttataaaaggtatttgtgaatagaaaatacaatgtgatcatttgtacttatgtgcaccttaaaagaggaattctgtctagctgtcaaattctggttccttaacatccagtccttgattgtgattgagatctggtaggacgtgctggggcacgctagcagataaaatcccgtatactttaggatagatgttacatttatgtcagtgttggcaaagagcattgtgtagtaataaagaattcaagacttcagcaatgtcaacctgaaactttgtaaatatttcctagattgttatttgatgcagtcacagctctttatcacacaatgttgtctttccctcatcaggcaattttagaactgctgcacacccctcctcagatctcacctgcccctcctgtacattcacctctccagccttgtgcacacctcatttagctttagtttgaaacacattgcagggttcaggtgacctcttcaaaaactacctcctcagaatgaggtaatgaatagttatttattttaaaatatgaaaagtcaggagctctagaatatgaagatgatctaagattttaacttttatgtatacttgttgagcactctccttttgtcctaaagggcattatacatttaagcagtaatactgaaaaatgtagctcagagtaactgaatgttgttgaaagtggtgccagaatctgttttaggggtacgtatcagaatcttaatcttaaatcggttacatgaaattaaatagttaatggtaacacttgactaacagatataattttaattttcggtaggcttttagcaagacagtaagtacatcttcataatgagttagccacagcttcatcacatgcacagattttcctgttgagagactgcccagttaagagggtagaatgatgaaccatttttcaggattctcttctttgtccaaactggcattgtgagtgctagaatatcagcactttcaaactagtgattccaactattaggctattaaaaagcaaaacaaaccaaacaaaccatagccagacatgggaagtttactatgagtataaacagcaaatagcttacaggtcatacattgaaatggtgtaggtaaggcgttagaaaaataccttgacaatttgccaaatgatcttactgtgccttcatgatgcaataaaaaaaaaaaaaatttagcataaatcagtgatttgtgaagagagcagccaccctggtctaactcagctgtgttaatattttttagcgtgcaatttagactgcaaagataaatgcactaaagagtttatagccaaaatcacatttaaaaaatgagagaaaacacaggtaaattttcagtgaacaaaattatttttttaaagtacataatccctagtatagtcagatatatttatcacatagagcaaataggttgaaatcacaattcagtgacatttctagagaaactttttctactcccataggttcttcaaagcatggaacttttatataacagaaatgtgtgacggtcattttaaattgctgtagtttggggctgaagtactgtgtgctgggcagcaatcacatgtattaactagtgagaaaggagaaattaagatataggacagaatttgattttcttgttcccagattactgctgccaacctagacactgagtttccagaggctgaaacgtaaacttgcagctcagcaactgttttgcaaagttagtgggactgtcctgcttatgctgttcaaaaatgctctgagggccaggtggggcctccaggggctcctctctgaggggacatcagactagctaacgacctggcgggcggatgtgaaccggacacactccatggtgtgcttcttgtatcggtccctcgccaccctcaagaaaggcttcagcgggttctctagacgtctccactaaggtgtgttactaacagccatgggttgttgagcacccgaggagtgcaatagcatctctgcatgattgtatattggcccgaagagaatgaagtggccagtgtactcatgttccatgttgctagctctggtaaactgaaaatactggtaagatttttgttttatcagtacactagagagtaagctttgttttgttgtttttagataatgttttcacttccatttggaaagacatttaaattgagtttcagtcctaaattttgccagtcatggtaattagcagtttctatcaggtatttttaaggtagaagaggatagaaacataagttctaaaagcttaaggtaaccgtggtttattttaaaatgtttaggggtggttagtctctacctcaaaaaaagtgagtgaatcttttatttcagcattcacaagttcggctgttgtttttgtaatacattttttttttaaccttttgacccccctttacctaagtgtcaatgtagttttattaattactaagtcagtttcattaaaatgtttatttagcagttttgactaattgcaatgattaatatagccagttgtgcatgaggacacagccagtgagtatatctgggttttttttgtgatgctttttttcttaagacttctgtagatttatgaagtactcattgaaaacaactaaaatacgtttattcgtgttaatatggaaaaaaaaaaa

SEQ ID NO: 108 - protein, 766 aa, Bos taurus
MAALSGGGGGGGGGAEQGQALFNGDMEPEAGAAASSAADPAIPEEVWNIKQMIKLTQEHIEALLDKFGGEHNPPSIYLEAYEEYTSKLDALQQREQQLLESLGNGTDFSVSSSASTDTVTSSSSSSLSVLPSSLSVFQNPTDVSRSNPKSPQKPIVRVFLPNKQRTVVPARCGVTVRDSLKKALMMRGLIPECCAVYRIQDGEKKPIGWDTDISWLTGEELHVEVLENVPLTTHNFVRKTFFTLAFCDFCRKLLFQGFRCQTCGYKFHQRCSTEVPLMCVNYDQLDLLFVSKFFEHHPIPQEEASLAETTLPCGSSPSAPPSDSIGPPILTSPSPSKSIPIPQPFRPADEDHRNQFGQRDRSSSAPNVHINTIEPVNIDDLIRDQGFRSDGGSTTGLSATPPASLPGSLSNVKALQKSPGPQRERKSSSSSEDRNRMKTLGRRDSSDDWEIPDGQITVGQRIGSGSFGTVYKGKWHGDVAVKMLNVTAPTPQQLQAFKNEVGVLRKTRHVNILLFMGYSTKPQLAIVTQWCEGSSLYHHLHIIETKFEMIKLIDIARQTAQGMDYLHAKSIIHRDLKSNNIFLHEDLTVKIGDFGLATVKSRWSGSHQFEQLSGSILWMAPEVIRMQDKNPYSFQSDVYAFGIVLYELMTGQLPYSNINNRDQIIFMVGRGYLSPDLSKVRSNCPKAMKRLMAECLKKKRDERPLFPQILASIELLARSLPKIHRSASEPSLNRAGFQTEDFSLYACASPKTPIQAGGYGEFAAFK

SEQ ID NO: 109 - DNA, 4670 bp, Bos taurus
ggtgtgtcatagtgcagcagattgaatgcagaagatatgaaaattcagatgtcttctgttaaggtgtggaatatcaaacaaatgattaagttgacacaggagcatatagaggccctattggacaaatttggtggggagcataatccaccatcaatatatctggaggcctatgaagaatacaccagcaagctagatgccctccaacaaagagaacaacagttattggaatccctggggaatggaactgatttttctgtttctagctctgcatcaacggacaccgttacatcttcttcctcttctagcctttcagtgctgccttcatctctttcagtttttcaaaatcccacagatgtgtcacggagcaaccccaagtcaccacaaaaacctatcgttagagtcttcctgcccaataaacagaggacagtggtacctgcacggtgtggagtcacagtccgggacagcctgaagaaggcactgatgatgagaggtctaatcccagagtgctgtgctgtttacagaattcaggatggggagaagaaaccaattggctgggacactgatatttcctggcttactggagaggagttgcatgtagaagtgttggagaatgttccacttacaacacacaactttgtacggaaaacttttttcaccttagcattttgtgacttctgtagaaagctgcttttccagggattccgctgtcaaacatgtggttataaatttcaccagcgttgtagtacagaggttccactgatgtgtgttaattatgaccaactagatttgctgtttgtctccaagttctttgaacaccacccaataccacaggaggaggcctccttagcagagactacccttccatgtggctcatccccttctgcacccccctccgattctattgggcccccaattctcaccagtccatctccttcaaaatccattccaattccacagcctttccgaccagcagatgaagatcatcgaaatcagtttggacaacgagaccggtcctcatcagctccaaatgtgcatataaacacaatagaacccgtcaatattgatgacttgattagagaccaagggtttcgtagtgatggaggatcaaccacaggtttatccgccacaccccctgcctcattacctggctcactctctaatgtgaaagcattgcagaaatctccaggacctcagcgagaaagaaagtcctcttcatcctcagaagacaggaatcgaatgaaaacgcttggtagacgggattcaagtgacgattgggagattcctgatggacagatcacagtgggacaaagaattggatcagggtcatttgggacagtctacaagggaaagtggcatggtgatgtggcagtgaaaatgttgaatgtgacagcacccacacctcagcagttacaggccttcaaaaatgaagtaggagtactcaggaaaacgcgacatgtgaatatcctcctcttcatgggttattcaacaaagccacaactggctattgttacccagtggtgtgagggctccagtttatatcatcatctccacatcattgagaccaaattcgagatgatcaaacttatagatattgcacggcagactgcacagggcatggattacttacacgccaagtcaatcatccacagagacctcaagagtaataatatttttcttcatgaagacctcacagtaaaaataggtgattttggtctagccacagtgaaatctcgatggagtgggtcccatcagtttgaacagttgtctggatccattttgtggatggcaccagaagtaatcagaatgcaagataaaaacccatatagctttcagtcagatgtatatgcatttgggattgttctgtatgaattgatgaccggacagttaccttattcaaatatcaacaacagggaccagataatttttatggtgggacgaggatatctgtctccagatctcagtaaggtacggagtaactgtccaaaagccatgaagagattaatggcagagtgcctaaaaaagaaaagagatgaaagaccactctttccccaagtaggaaagactctcctaagcaagagacaaaattcagaagttatcagggaaaaagataagcagattctcgcctctattgagctgctggcccgctcattgccaaaaattcaccgcagtgcatcagaaccctccttgaatcgggctggcttccaaacagaggattttagtctatatgcttgtgcttctccaaaaacacccattcaggcagggggatatgaagcagatttggctcttacatcaaataaaaatagagtagaagttgggatttagagatttcctgacatgcaagaaggaataagcaagaaaaaaaggtttgttttccccaaatcatatctattgtcttttacttctattttttcttaaattttttgtgatttcagagacatgtagagttttattgatacctaaactatgagttcttttttttttttttttttcattattttgatttttttggccaagaggcatatgggatcttagcttgagaaagcaacaattttcttgatgtcattttgggtgagggcacatattgctgtgaacagtgtggtgatagccaccagggaccaaactcacacccgctgcattgaaaggtgaagtcttaaacactggaccagcagagaaattcctactctatgagttctttttgtcatcccctccccgcaccctccacccccaacctaaagtctgatgatgaaatcaacaactattccattagaagcagtagattctggtagcatgatctttagtttgttagtaagattttgtgctttgtggggttgtgtcgttttaaggctaatatttaagtttgtcaaatagaatgctgttcagattgtaaaaatgagtaataaacatctgaagttttttttaagttatttttaacatggtatatacagttgagcttagagtttatcattttctgatattctcttacttagtagatgaattctagccattttttataaagatttctgttaagcaaatcctgttttcacatgggcttcctttaagggattttagattctgctggatatggtgactgctcataagactgttgaaaattacttttaagatgtattagaatacttctgaaaaaaaatagcaaccttaaaaccataagcaaaagtagtaagggtgtttatacatttctagagtccctgtttaggtaatagcctcctatgattgtactttaaatgttttgctctccaaggttttagtaacttggctttttttctaatcagtgccaaactcccccagtttttttaactttaaatatgaggtaataaatcttttacccttccttgatcttttgacttataataccttggtcagttgtttcttaaaaggaatccttaaatggaaagagacaatatcactgtctgcagttctgattagtagttttattcagaatggaaaaacagattattcatttttgaaaattgttcaggggtatgttcattgttaggaccttggactttggagtcagtgcctagctatgcattccaggtctgccattttctggctgtgaaattttggacaagttacttaaccactttaaaccccagctttaagaagtaaattaaccccagtaaattaagaagtaatagcagccacttcgtagagttgttatgaggctcagatgcagtgcaaatgtgtataaagtattcagggagtcacctggtatactataatagacactagaatagttgccaatattatcagcatacaatctgaggattctgtcagccaatcattagcaatctgttgtttgttgggacatgccagtgttctccagttgaaatcagtagcaatctaaaaatggatagattattcctcatttaaatagtgtgttcatataagtgattgcttggatccttatcagaagttgctgttactgaaaaatgataaggctgactaaattgtgatagttgtcagttactaaccaactcccagaaatgaataagaggaacctatctctagttcctagtagaaggtatggacaaaatagtaggtgaaaaataatgtcttgaacccccaaattaagtaagctttaaagagtacaatacctcaaagggtctttgcggtttaaaatttgtatgctgagaatgatgttcattgacatgtgcctatatgtaattttttgatagtttaaaaggtgaaatgaactacagatgggagaggtctgaattttcttgccttcagtcaaatgtgtaatgtggacatattatttgacctgtgaattttatcttttaaaaaagattaattcctgcttcttccttcctaatagttgcattataataatgaaaatgagttgataatttggggggaaagtattctacaaatcaaccttattattttaccattggtttctgagaaattttgttcatttgaaccgtttatagcttgattagaatcatagcatgtaaaacccaactgagggattatctgcagacttaatgtagtattatgtaagttgtcttctttcatttcgaccttttttgcttttgttgttgctagatctgtagtatgtagctagtcacctttcagcgaggtttcagcgaggcttttctgtgtctctaggttatttgagataacttttttaaaattagctcttgtcctcc

SEQ ID NO: 110 - protein, 761 aa, Bos taurus
MKIQMSSVKVWNIKQMIKLTQEHIEALLDKFGGEHNPPSIYLEAYEEYTSKLDALQQREQQLLESLGNGTDFSVSSSASTDTVTSSSSSSLSVLPSSLSVFQNPTDVSRSNPKSPQKPIVRVFLPNKQRTVVPARCGVTVRDSLKKALMMRGLIPECCAVYRIQDGEKKPIGWDTDISWLTGEELHVEVLENVPLTTHNFVRKTFFTLAFCDFCRKLLFQGFRCQTCGYKFHQRCSTEVPLMCVNYDQLDLLFVSKFFEHHPIPQEEASLAETTLPCGSSPSAPPSDSIGPPILTSPSPSKSIPIPQPFRPADEDHRNQFGQRDRSSSAPNVHINTIEPVNIDDLIRDQGFRSDGGSTTGLSATPPASLPGSLSNVKALQKSPGPQRERKSSSSSEDRNRMKTLGRRDSSDDWEIPDGQITVGQRIGSGSFGTVYKGKWHGDVAVKMLNVTAPTPQQLQAFKNEVGVLRKTRHVNILLFMGYSTKPQLAIVTQWCEGSSLYHHLHIIETKFEMIKLIDIARQTAQGMDYLHAKSIIHRDLKSNNIFLHEDLTVKIGDFGLATVKSRWSGSHQFEQLSGSILWMAPEVIRMQDKNPYSFQSDVYAFGIVLYELMTGQLPYSNINNRDQIIFMVGRGYLSPDLSKVRSNCPKAMKRLMAECLKKKRDERPLFPQVGKTLLSKRQNSEVIREKDKQILASIELLARSLPKIHRSASEPSLNRAGFQTEDFSLYACASPKTPIQAGGYEADLALTSNKNRVEVGI

SEQ ID NO: 111 - DNA, 4816 bp, Bos taurus
ctcagctgcgccgggtctcacaagacggttcccgaggtggcccaggcgccgtcccaccgccgacgccgcccgggccgcccgggccgtccctccccgctgccccccgtcctccgcctccgcctccccccgccctcagcctcccttccccctccccgcccagcagcggtcgctcgggcccggctctcggttataagatggcggcgctgagtggcggcggcggcggcggcggcggtggcgcggagcagggccaggctctgttcaacggggacatggagcccgaggccggcgccgcggcctcttcggctgcggaccccgccattcccgaggaggtgtggaatatcaaacaaatgattaagttgacacaggagcatatagaggccctattggacaaatttggtggggagcataatccaccatcaatatatctggaggcctatgaagaatacaccagcaagctagatgccctccaacaaagagaacaacagttattggaatccctggggaatggaactgatttttctgtttctagctctgcatcaacggacaccgttacatcttcttcctcttctagcctttcagtgctgccttcatctctttcagtttttcaaaatcccacagatgtgtcacggagcaaccccaagtcaccacaaaaacctatcgttagagtcttcctgcccaataaacagaggacagtggtacctgcacggtgtggagtcacagtccgggacagcctgaagaaggcactgatgatgagaggtctaatcccagagtgctgtgctgtttacagaattcaggatggggagaagaaaccaattggctgggacactgatatttcctggcttactggagaggagttgcatgtagaagtgttggagaatgttccacttacaacacacaactttgtacggaaaacttttttcaccttagcattttgtgacttctgtagaaagctgcttttccagggattccgctgtcaaacatgtggttataaatttcaccagcgttgtagtacagaggttccactgatgtgtgttaattatgaccaactagagcccccaattctcaccagtccatctccttcaaaatccattccaattccacagcctttccgaccagcagatgaagatcatcgaaatcagtttggacaacgagaccggtcctcatcagctccaaatgtgcatataaacacaatagaacccgtcaatattgatgacttgattagagaccaagggtttcgtagtgatggaggatcaaccacaggtttatccgccacaccccctgcctcattacctggctcactctctaatgtgaaagcattgcagaaatctccaggacctcagcgagaaagaaagtcctcttcatcctcagaagacaggaatcgaatgaaaacgcttggtagacgggattcaagtgacgattgggagattcctgatggacagatcacagtgggacaaagaattggatcagggtcatttgggacagtctacaagggaaagtggcatggtgatgtggcagtgaaaatgttgaatgtgacagcacccacacctcagcagttacaggccttcaaaaatgaagtaggagtactcaggaaaacgcgacatgtgaatatcctcctcttcatgggttattcaacaaagccacaactggctattgttacccagtggtgtgagggctccagtttatatcatcatctccacatcattgagaccaaattcgagatgatcaaacttatagatattgcacggcagactgcacagggcatggattacttacacgccaagtcaatcatccacagagacctcaagagtaataatatttttcttcatgaagacctcacagtaaaaataggtgattttggtctagccacagtgaaatctcgatggagtgggtcccatcagtttgaacagttgtctggatccattttgtggatggcaccagaagtaatcagaatgcaagataaaaacccatatagctttcagtcagatgtatatgcatttgggattgttctgtatgaattgatgaccggacagttaccttattcaaatatcaacaacagggaccagataatttttatggtgggacgaggatatctgtctccagatctcagtaaggtacggagtaactgtccaaaagccatgaagagattaatggcagagtgcctaaaaaagaaaagagatgaaagaccactctttccccaagtaggaaagactctcctaagcaagagacaaaattcagaagttatcagggaaaaagataagcagattctcgcctctattgagctgctggcccgctcattgccaaaaattcaccgcagtgcatcagaaccctccttgaatcgggctggcttccaaacagaggattttagtctatatgcttgtgcttctccaaaaacacccattcaggcagggggatatgaagcagatttggctcttacatcaaataaaaatagagtagaagttgggatttagagatttcctgacatgcaagaaggaataagcaagaaaaaaaggtttgttttccccaaatcatatctattgtcttttacttctattttttcttaaattttttgtgatttcagagacatgtagagttttattgatacctaaactatgagttcttttttttttttttttttcattattttgatttttttggccaagaggcatatgggatcttagcttgagaaagcaacaattttcttgatgtcattttgggtgagggcacatattgctgtgaacagtgtggtgatagccaccagggaccaaactcacacccgctgcattgaaaggtgaagtcttaaacactggaccagcagagaaattcctactctatgagttctttttgtcatcccctccccgcaccctccacccccaacctaaagtctgatgatgaaatcaacaactattccattagaagcagtagattctggtagcatgatctttagtttgttagtaagattttgtgctttgtggggttgtgtcgttttaaggctaatatttaagtttgtcaaatagaatgctgttcagattgtaaaaatgagtaataaacatctgaagttttttttaagttatttttaacatggtatatacagttgagcttagagtttatcattttctgatattctcttacttagtagatgaattctagccattttttataaagatttctgttaagcaaatcctgttttcacatgggcttcctttaagggattttagattctgctggatatggtgactgctcataagactgttgaaaattacttttaagatgtattagaatacttctgaaaaaaaatagcaaccttaaaaccataagcaaaagtagtaagggtgtttatacatttctagagtccctgtttaggtaatagcctcctatgattgtactttaaatgttttgctctccaaggttttagtaacttggctttttttctaatcagtgccaaactcccccagtttttttaactttaaatatgaggtaataaatcttttacccttccttgatcttttgacttataataccttggtcagttgtttcttaaaaggaatccttaaatggaaagagacaatatcactgtctgcagttctgattagtagttttattcagaatggaaaaacagattattcatttttgaaaattgttcaggggtatgttcattgttaggaccttggactttggagtcagtgcctagctatgcattccaggtctgccattttctggctgtgaaattttggacaagttacttaaccactttaaaccccagctttaagaagtaaattaaccccagtaaattaagaagtaatagcagccacttcgtagagttgttatgaggctcagatgcagtgcaaatgtgtataaagtattcagggagtcacctggtatactataatagacactagaatagttgccaatattatcagcatacaatctgaggattctgtcagccaatcattagcaatctgttgtttgttgggacatgccagtgttctccagttgaaatcagtagcaatctaaaaatggatagattattcctcatttaaatagtgtgttcatataagtgattgcttggatccttatcagaagttgctgttactgaaaaatgataaggctgactaaattgtgatagttgtcagttactaaccaactcccagaaatgaataagaggaacctatctctagttcctagtagaaggtatggacaaaatagtaggtgaaaaataatgtcttgaacccccaaattaagtaagctttaaagagtacaatacctcaaagggtctttgcggtttaaaatttgtatgctgagaatgatgttcattgacatgtgcctatatgtaattttttgatagtttaaaaggtgaaatgaactacagatgggagaggtctgaattttcttgccttcagtcaaatgtgtaatgtggacatattatttgacctgtgaattttatcttttaaaaaagattaattcctgcttcttccttcctaatagttgcattataataatgaaaatgagttgataatttggggggaaagtattctacaaatcaaccttattattttaccattggtttctgagaaattttgttcatttgaaccgtttatagcttgattagaatcatagcatgtaaaacccaactgagggattatctgcagacttaatgtagtattatgtaagttgtcttctttcatttcgaccttttttgcttttgttgttgctagatctgtagtatgtagctagtcacctttcagcgaggtttcagcgaggcttttctgtgtctctaggttatttgagataacttttttaaaattagctcttgtcctcc

SEQ ID NO: 112 - protein, 757 aa, Bos taurus
MAALSGGGGGGGGGAEQGQALFNGDMEPEAGAAASSAADPAIPEEVWNIKQMIKLTQEHIEALLDKFGGEHNPPSIYLEAYEEYTSKLDALQQREQQLLESLGNGTDFSVSSSASTDTVTSSSSSSLSVLPSSLSVFQNPTDVSRSNPKSPQKPIVRVFLPNKQRTVVPARCGVTVRDSLKKALMMRGLIPECCAVYRIQDGEKKPIGWDTDISWLTGEELHVEVLENVPLTTHNFVRKTFFTLAFCDFCRKLLFQGFRCQTCGYKFHQRCSTEVPLMCVNYDQLEPPILTSPSPSKSIPIPQPFRPADEDHRNQFGQRDRSSSAPNVHINTIEPVNIDDLIRDQGFRSDGGSTTGLSATPPASLPGSLSNVKALQKSPGPQRERKSSSSSEDRNRMKTLGRRDSSDDWEIPDGQITVGQRIGSGSFGTVYKGKWHGDVAVKMLNVTAPTPQQLQAFKNEVGVLRKTRHVNILLFMGYSTKPQLAIVTQWCEGSSLYHHLHIIETKFEMIKLIDIARQTAQGMDYLHAKSIIHRDLKSNNIFLHEDLTVKIGDFGLATVKSRWSGSHQFEQLSGSILWMAPEVIRMQDKNPYSFQSDVYAFGIVLYELMTGQLPYSNINNRDQIIFMVGRGYLSPDLSKVRSNCPKAMKRLMAECLKKKRDERPLFPQVGKTLLSKRQNSEVIREKDKQILASIELLARSLPKIHRSASEPSLNRAGFQTEDFSLYACASPKTPIQAGGYEADLALTSNKNRVEVGI

SEQ ID NO: 113 - DNA, 2499 bp, Bos taurus
ctcagctgcgccgggtctcacaagacggttcccgaggtggcccaggcgccgtcccaccgccgacgccgcccgggccgcccgggccgtccctccccgctgccccccgtcctccgcctccgcctccccccgccctcagcctcccttccccctccccgcccagcagcggtcgctcgggcccggctctcggttataagatggcggcgctgagtggcggcggcggcggcggcggcggtggcgcggagcagggccaggctctgttcaacggggacatggagcccgaggccggcgccgcggcctcttcggctgcggaccccgccattcccgaggaggtgtggaatatcaaacaaatgattaagttgacacaggagcatatagaggccctattggacaaatttggtggggagcataatccaccatcaatatatctggaggcctatgaagaatacaccagcaagctagatgccctccaacaaagagaacaacagttattggaatccctggggaatggaactgatttttctgtttctagctctgcatcaacggacaccgttacatcttcttcctcttctagcctttcagtgctgccttcatctctttcagtttttcaaaatcccacagatgtgtcacggagcaaccccaagtcaccacaaaaacctatcgttagagtcttcctgcccaataaacagaggacagtggtacctgcacggtgtggagtcacagtccgggacagcctgaagaaggcactgatgatgagaggtctaatcccagagtgctgtgctgtttacagaattcaggatggggagaagaaaccaattggctgggacactgatatttcctggcttactggagaggagttgcatgtagaagtgttggagaatgttccacttacaacacacaactttgtacggaaaacttttttcaccttagcattttgtgacttctgtagaaagctgcttttccagggattccgctgtcaaacatgtggttataaatttcaccagcgttgtagtacagaggttccactgatgtgtgttaattatgaccaactagatttgctgtttgtctccaagttctttgaacaccacccaataccacaggaggaggcctccttagcagagactacccttccatgtggctcatccccttctgcacccccctccgattctattgggcccccaattctcaccagtccatctccttcaaaatccattccaattccacagcctttccgaccagcagatgaagatcatcgaaatcagtttggacaacgagaccggtcctcatcagctccaaatgtgcatataaacacaatagaacccgtcaatattgatgacttgattagagaccaagggtttcgtagtgatggaggatcaaccacaggtttatccgccacaccccctgcctcattacctggctcactctctaatgtgaaagcattgcagaaatctccaggacctcagcgagaaagaaagtcctcttcatcctcagaagacaggaatcgaatgaaaacgcttggtagacgggattcaagtgacgattgggagattcctgatggacagatcacagtgggacaaagaattggatcagggtcatttgggacagtctacaagggaaagtggcatggtgatgtggcagtgaaaatgttgaatgtgacagcacccacacctcagcagttacaggccttcaaaaatgaagtaggagtactcaggaaaacgcgacatgtgaatatcctcctcttcatgggttattcaacaaagccacaactggctattgttacccagtggtgtgagggctccagtttatatcatcatctccacatcattgagaccaaattcgagatgatcaaacttatagatattgcacggcagactgcacagggcatggattacttacacgccaagtcaatcatccacagagacctcaagagtaataatatttttcttcatgaagacctcacagtaaaaataggtgattttggtctagccacagtgaaatctcgatggagtgggtcccatcagtttgaacagttgtctggatccattttgtggatggcaccagaagtaatcagaatgcaagataaaaacccatatagctttcagtcagatgtatatgcatttgggattgttctgtatgaattgatgaccggacagttaccttattcaaatatcaacaacagggaccagataatttttatggtgggacgaggatatctgtctccagatctcagtaaggtacggagtaactgtccaaaagccatgaagagattaatggcagagtgcctaaaaaagaaaagagatgaaagaccactctttccccaagtaggaaagactctcctaagcaagagacaaaattcagaagttatcagggaaaaagataagcaggaaaagtatgtttctttagtacattccaggcatttgggattacagtaaaaacaatattctcgcctctattgagctgctggcccgctcattgccaaaaattcaccgcagtgcatcagaa

SEQ ID NO: 114 - protein, 744 aa, Bos taurus
MAALSGGGGGGGGGAEQGQALFNGDMEPEAGAAASSAADPAIPEEVWNIKQMIKLTQEHIEALLDKFGGEHNPPSIYLEAYEEYTSKLDALQQREQQLLESLGNGTDFSVSSSASTDTVTSSSSSSLSVLPSSLSVFQNPTDVSRSNPKSPQKPIVRVFLPNKQRTVVPARCGVTVRDSLKKALMMRGLIPECCAVYRIQDGEKKPIGWDTDISWLTGEELHVEVLENVPLTTHNFVRKTFFTLAFCDFCRKLLFQGFRCQTCGYKFHQRCSTEVPLMCVNYDQLDLLFVSKFFEHHPIPQEEASLAETTLPCGSSPSAPPSDSIGPPILTSPSPSKSIPIPQPFRPADEDHRNQFGQRDRSSSAPNVHINTIEPVNIDDLIRDQGFRSDGGSTTGLSATPPASLPGSLSNVKALQKSPGPQRERKSSSSSEDRNRMKTLGRRDSSDDWEIPDGQITVGQRIGSGSFGTVYKGKWHGDVAVKMLNVTAPTPQQLQAFKNEVGVLRKTRHVNILLFMGYSTKPQLAIVTQWCEGSSLYHHLHIIETKFEMIKLIDIARQTAQGMDYLHAKSIIHRDLKSNNIFLHEDLTVKIGDFGLATVKSRWSGSHQFEQLSGSILWMAPEVIRMQDKNPYSFQSDVYAFGIVLYELMTGQLPYSNINNRDQIIFMVGRGYLSPDLSKVRSNCPKAMKRLMAECLKKKRDERPLFPQVGKTLLSKRQNSEVIREKDKQEKYVSLVHSRHLGLQ

SEQ ID NO: 115 - DNA, 2404 bp, Bos taurus
ctcagctgcgccgggtctcacaagacggttcccgaggtggcccaggcgccgtcccaccgccgacgccgcccgggccgcccgggccgtccctccccgctgccccccgtcctccgcctccgcctccccccgccctcagcctcccttccccctccccgcccagcagcggtcgctcgggcccggctctcggttataagatggcggcgctgagtggcggcggcggcggcggcggcggtggcgcggagcagggccaggctctgttcaacggggacatggagcccgaggccggcgccgcggcctcttcggctgcggaccccgccattcccgaggaggtgtggaatatcaaacaaatgattaagttgacacaggagcatatagaggccctattggacaaatttggtggggagcataatccaccatcaatatatctggaggcctatgaagaatacaccagcaagctagatgccctccaacaaagagaacaacagttattggaatccctggggaatggaactgatttttctgtttctagctctgcatcaacggacaccgttacatcttcttcctcttctagcctttcagtgctgccttcatctctttcagtttttcaaaatcccacagatgtgtcacggagcaaccccaagtcaccacaaaaacctatcgttagagtcttcctgcccaataaacagaggacagtggtacctgcacggtgtggagtcacagtccgggacagcctgaagaaggcactgatgatgagaggtctaatcccagagtgctgtgctgtttacagaattcaggatggggagaagaaaccaattggctgggacactgatatttcctggcttactggagaggagttgcatgtagaagtgttggagaatgttccacttacaacacacaactttgtacggaaaacttttttcaccttagcattttgtgacttctgtagaaagctgcttttccagggattccgctgtcaaacatgtggttataaatttcaccagcgttgtagtacagaggttccactgatgtgtgttaattatgaccaactagatttgctgtttgtctccaagttctttgaacaccacccaataccacaggaggaggcctccttagcagagactacccttccatgtggctcatccccttctgcacccccctccgattctattgggcccccaattctcaccagtccatctccttcaaaatccattccaattccacagcctttccgaccagcagatgaagatcatcgaaatcagtttggacaacgagaccggtcctcatcagctccaaatgtgcatataaacacaatagaacccgtcaatattgatgacttgattagagaccaagggtttcgtagtgatggaggatcaaccacaggtttatccgccacaccccctgcctcattacctggctcactctctaatgtgaaagcattgcagaaatctccaggacctcagcgagaaagaaagtcctcttcatcctcagaagacaggaatcgaatgaaaacgcttggtagacgggattcaagtgacgattgggagattcctgatggacagatcacagtgggacaaagaattggatcagggtcatttgggacagtctacaagggaaagtggcatggtgatgtggcagtgaaaatgttgaatgtgacagcacccacacctcagcagttacaggccttcaaaaatgaagtaggagtactcaggaaaacgcgacatgtgaatatcctcctcttcatgggttattcaacaaagccacaactggctattgttacccagtggtgtgagggctccagtttatatcatcatctccacatcattgagaccaaattcgagatgatcaaacttatagatattgcacggcagactgcacagggcatggattacttacacgccaagtcaatcatccacagagacctcaagagtaataatatttttcttcatgaagacctcacagtaaaaataggtgattttggtctagccacagtgaaatctcgatggagtgggtcccatcagtttgaacagttgtctggatccattttgtggatggcaccagaagtaatcagaatgcaagataaaaacccatatagctttcagtcagatgtatatgcatttgggattgttctgtatgaattgatgaccggacagttaccttattcaaatatcaacaacagggaccagataatttttatggtgggacgaggatatctgtctccagatctcagtaaggtacggagtaactgtccaaaagccatgaagagattaatggcagagtgcctaaaaaagaaaagagatgaaagaccactctttccccaagatctctcttcccaccatagacacaaaaatttcagatggctacaggtttacatgtaaaaaacagaattataacaaatgatttttat

SEQ ID NO: 116 - protein, 726 aa, Bos taurus
MAALSGGGGGGGGGAEQGQALFNGDMEPEAGAAASSAADPAIPEEVWNIKQMIKLTQEHIEALLDKFGGEHNPPSIYLEAYEEYTSKLDALQQREQQLLESLGNGTDFSVSSSASTDTVTSSSSSSLSVLPSSLSVFQNPTDVSRSNPKSPQKPIVRVFLPNKQRTVVPARCGVTVRDSLKKALMMRGLIPECCAVYRIQDGEKKPIGWDTDISWLTGEELHVEVLENVPLTTHNFVRKTFFTLAFCDFCRKLLFQGFRCQTCGYKFHQRCSTEVPLMCVNYDQLDLLFVSKFFEHHPIPQEEASLAETTLPCGSSPSAPPSDSIGPPILTSPSPSKSIPIPQPFRPADEDHRNQFGQRDRSSSAPNVHINTIEPVNIDDLIRDQGFRSDGGSTTGLSATPPASLPGSLSNVKALQKSPGPQRERKSSSSSEDRNRMKTLGRRDSSDDWEIPDGQITVGQRIGSGSFGTVYKGKWHGDVAVKMLNVTAPTPQQLQAFKNEVGVLRKTRHVNILLFMGYSTKPQLAIVTQWCEGSSLYHHLHIIETKFEMIKLIDIARQTAQGMDYLHAKSIIHRDLKSNNIFLHEDLTVKIGDFGLATVKSRWSGSHQFEQLSGSILWMAPEVIRMQDKNPYSFQSDVYAFGIVLYELMTGQLPYSNINNRDQIIFMVGRGYLSPDLSKVRSNCPKAMKRLMAECLKKKRDERPLFPQDLSSHHRHKNFRWLQVYM

SEQ ID NO: 117 - DNA, 2331 bp, Bos taurus
ctcagctgcgccgggtctcacaagacggttcccgaggtggcccaggcgccgtcccaccgccgacgccgcccgggccgcccgggccgtccctccccgctgccccccgtcctccgcctccgcctccccccgccctcagcctcccttccccctccccgcccagcagcggtcgctcgggcccggctctcggttataagatggcggcgctgagtggcggcggcggcggcggcggcggtggcgcggagcagggccaggctctgttcaacggggacatggagcccgaggccggcgccgcggcctcttcggctgcggaccccgccattcccgaggaggtgtggaatatcaaacaaatgattaagttgacacaggagcatatagaggccctattggacaaatttggtggggagcataatccaccatcaatatatctggaggcctatgaagaatacaccagcaagctagatgccctccaacaaagagaacaacagttattggaatccctggggaatggaactgatttttctgtttctagctctgcatcaacggacaccgttacatcttcttcctcttctagcctttcagtgctgccttcatctctttcagtttttcaaaatcccacagatgtgtcacggagcaaccccaagtcaccacaaaaacctatcgttagagtcttcctgcccaataaacagaggacagtggtacctgcacggtgtggagtcacagtccgggacagcctgaagaaggcactgatgatgagaggtctaatcccagagtgctgtgctgtttacagaattcaggatggggagaagaaaccaattggctgggacactgatatttcctggcttactggagaggagttgcatgtagaagtgttggagaatgttccacttacaacacacaactttgtacggaaaacttttttcaccttagcattttgtgacttctgtagaaagctgcttttccagggattccgctgtcaaacatgtggttataaatttcaccagcgttgtagtacagaggttccactgatgtgtgttaattatgaccaactagatttgctgtttgtctccaagttctttgaacaccacccaataccacaggaggaggcctccttagcagagactacccttccatgtggctcatccccttctgcacccccctccgattctattgggcccccaattctcaccagtccatctccttcaaaatccattccaattccacagcctttccgaccagcagatgaagatcatcgaaatcagtttggacaacgagaccggtcctcatcagctccaaatgtgcatataaacacaatagaacccgtcaatattgatgacttgattagagaccaagggtttcgtagtgatggaggatcaaccacaggtttatccgccacaccccctgcctcattacctggctcactctctaatgtgaaagcattgcagaaatctccaggacctcagcgagaaagaaagtcctcttcatcctcagaagacaggaatcgaatgaaaacgcttggtagacgggattcaagtgacgattgggagattcctgatggacagatcacagtgggacaaagaattggatcagggtcatttgggacagtctacaagggaaagtggcatggtgatgtggcagtgaaaatgttgaatgtgacagcacccacacctcagcagttacaggccttcaaaaatgaagtaggagtactcaggaaaacgcgacatgtgaatatcctcctcttcatgggttattcaacaaagccacaactggctattgttacccagtggtgtgagggctccagtttatatcatcatctccacatcattgagaccaaattcgagatgatcaaacttatagatattgcacggcagactgcacagggcatggattacttacacgccaagtcaatcatccacagagacctcaagagtaataatatttttcttcatgaagacctcacagtaaaaataggtgattttggtctagccacagtgaaatctcgatggagtgggtcccatcagtttgaacagttgtctggatccattttgtggatggcaccagaagtaatcagaatgcaagataaaaacccatatagctttcagtcagatgtatatgcatttgggattgttctgtatgaattgatgaccggacagttaccttattcaaatatcaacaacagggaccaggtgctttgtcctccatgggagtgtaataaatgctgtgcaagggcttacttcccatgagagaagtgagtgaccaacagaaggataatttttatggtgggacgaggatatctgtctccagatctcagtaaggtacggagtaactgtccaa

SEQ ID NO: 118 - protein, 681 aa, Bos taurus
MAALSGGGGGGGGGAEQGQALFNGDMEPEAGAAASSAADPAIPEEVWNIKQMIKLTQEHIEALLDKFGGEHNPPSIYLEAYEEYTSKLDALQQREQQLLESLGNGTDFSVSSSASTDTVTSSSSSSLSVLPSSLSVFQNPTDVSRSNPKSPQKPIVRVFLPNKQRTVVPARCGVTVRDSLKKALMMRGLIPECCAVYRIQDGEKKPIGWDTDISWLTGEELHVEVLENVPLTTHNFVRKTFFTLAFCDFCRKLLFQGFRCQTCGYKFHQRCSTEVPLMCVNYDQLDLLFVSKFFEHHPIPQEEASLAETTLPCGSSPSAPPSDSIGPPILTSPSPSKSIPIPQPFRPADEDHRNQFGQRDRSSSAPNVHINTIEPVNIDDLIRDQGFRSDGGSTTGLSATPPASLPGSLSNVKALQKSPGPQRERKSSSSSEDRNRMKTLGRRDSSDDWEIPDGQITVGQRIGSGSFGTVYKGKWHGDVAVKMLNVTAPTPQQLQAFKNEVGVLRKTRHVNILLFMGYSTKPQLAIVTQWCEGSSLYHHLHIIETKFEMIKLIDIARQTAQGMDYLHAKSIIHRDLKSNNIFLHEDLTVKIGDFGLATVKSRWSGSHQFEQLSGSILWMAPEVIRMQDKNPYSFQSDVYAFGIVLYELMTGQLPYSNINNRDQVLCPPWECNKCCARAYFP

SEQ ID NO: 119 - DNA, 2319 bp, Bos taurus
ctcagctgcgccgggtctcacaagacggttcccgaggtggcccaggcgccgtcccaccgccgacgccgcccgggccgcccgggccgtccctccccgctgccccccgtcctccgcctccgcctccccccgccctcagcctcccttccccctccccgcccagcagcggtcgctcgggcccggctctcggttataagatggcggcgctgagtggcggcggcggcggcggcggcggtggcgcggagcagggccaggctctgttcaacggggacatggagcccgaggccggcgccgcggcctcttcggctgcggaccccgccattcccgaggaggtgtggaatatcaaacaaatgattaagttgacacaggagcatatagaggccctattggacaaatttggtggggagcataatccaccatcaatatatctggaggcctatgaagaatacaccagcaagctagatgccctccaacaaagagaacaacagttattggaatccctggggaatggaactgatttttctgtttctagctctgcatcaacggacaccgttacatcttcttcctcttctagcctttcagtgctgccttcatctctttcagtttttcaaaatcccacagatgtgtcacggagcaaccccaagtcaccacaaaaacctatcgttagagtcttcctgcccaataaacagaggacagtggtacctgcacggtgtggagtcacagtccgggacagcctgaagaaggcactgatgatgagaggtctaatcccagagtgctgtgctgtttacagaattcaggatggggagaagaaaccaattggctgggacactgatatttcctggcttactggagaggagttgcatgtagaagtgttggagaatgttccacttacaacacacaactttgtacggaaaacttttttcaccttagcattttgtgacttctgtagaaagctgcttttccagggattccgctgtcaaacatgtggttataaatttcaccagcgttgtagtacagaggttccactgatgtgtgttaattatgaccaactagatttgctgtttgtctccaagttctttgaacaccacccaataccacaggaggaggcctccttagcagagactacccttccatgtggctcatccccttctgcacccccctccgattctattgggcccccaattctcaccagtccatctccttcaaaatccattccaattccacagcctttccgaccagcagatgaagatcatcgaaatcagtttggacaacgagaccggtcctcatcagctccaaatgtgcatataaacacaatagaacccgtcaatattgatgacttgattagagaccaagggtttcgtagtgatggaggatcaaccacaggtttatccgccacaccccctgcctcattacctggctcactctctaatgtgaaagcattgcagaaatctccaggacctcagcgagaaagaaagtcctcttcatcctcagaagacaggaatcgaatgaaaacgcttggtagacgggattcaagtgacgattgggagattcctgatggacagatcacagtgggacaaagaattggatcagggtcatttgggacagtctacaagggaaagtggcatggtgatgtggcagtgaaaatgttgaatgtgacagcacccacacctcagcagttacaggccttcaaaaatgaagtaggagtactcaggaaaacgcgacatgtgaatatcctcctcttcatgggttattcaacaaagccacaactggctattgttacccagtggtgtgagggctccagtttatatcatcatctccacatcattgagaccaaattcgagatgatcaaacttatagatattgcacggcagactgcacagggcatggattacttacacgccaagtcaatcatccacagagacctcaagagtaataatatttttcttcatgaagacctcacagtaaaaataggtgattttggtctagccacagtgaaatctcgatggagtgggtcccatcagtttgaacagttgtctggatccattttgtggatggcaccagaagtaatcagaatgcaagataaaaacccatatagctttcagtcagatgtatatgcatttgggattgttctgtatgaattgatgaccggacagttaccttattcaaatatcaacaacagggaccaggtgctttgtcctccatgggagtgtaataaatgctgtgcaagggcttacttcccatgagagaagtgagtgaccaacagaaggtctgtgcaaggaaaagagacaaagccacggatcagaagcacatggccataactga

SEQ ID NO: 120 - protein, 681 aa, Bos taurus; identical to SEQ ID NO: 118

SEQ ID NO: 121 - DNA, 2661 bp, Bos taurus
tcagctgcgccgggtctcacaagacggttcccgaggtggcccaggcgccgtcccaccgccgacgccgcccgggccgcccgggccgtccctccccgctgccccccgtcctccgcctccgcctccccccgccctcagcctcccttccccctccccgcccagcagcggtcgctcgggcccggctctcggttataagatggcggcgctgagtggcggcggcggcggcggcggcggtggcgcggagcagggccaggctctgttcaacggggacatggagcccgaggccggcgccgcggcctcttcggctgcggaccccgccattcccgaggaggtgtggaatatcaaacaaatgattaagttgacacaggagcatatagaggccctattggacaaatttggtggggagcataatccaccatcaatatatctggaggcctatgaagaatacaccagcaagctagatgccctccaacaaagagaacaacagttattggaatccctggggaatggaactgatttttctgtttctagctctgcatcaacggacaccgttacatcttcttcctcttctagcctttcagtgctgccttcatctctttcagtttttcaaaatcccacagatgtgtcacggagcaaccccaagtcaccacaaaaacctatcgttagagtcttcctgcccaataaacagaggacagtggtacctgcacggtgtggagtcacagtccgggacagcctgaagaaggcactgatgatgagaggtctaatcccagagtgctgtgctgtttacagaattcaggatggggagaagaaaccaattggctgggacactgatatttcctggcttactggagaggagttgcatgtagaagtgttggagaatgttccacttacaacacacaactttgtacggaaaacttttttcaccttagcattttgtgacttctgtagaaagctgcttttccagggattccgctgtcaaacatgtggttataaatttcaccagcgttgtagtacagaggttccactgatgtgtgttaattatgaccaactagatttgctgtttgtctccaagttctttgaacaccacccaataccacaggaggaggcctccttagcagagactacccttccatgtggctcatccccttctgcacccccctccgattctattgggcccccaattctcaccagtccatctccttcaaaatccattccaattccacagcctttccgaccagcagatgaagatcatcgaaatcagtttggacaacgagaccggtcctcatcagctccaaatgtgcatataaacacaatagaacccgtcaatattgatgacttgattagagaccaagggtttcgtagtgatggaggatcaaccacaggtttatccgccacaccccctgcctcattacctggctcactctctaatgtgaaagcattgcagaaatctccaggacctcagcgagaaagaaagtcctcttcatcctcagaagacaggaatcgaatgaaaacgcttggtagacgggattcaagtgacgattgggagattcctgatggacagatcacagtgggacaaagaattggatcagggtcatttgggacagtctacaagggaaagtggcatggtgatgtggcagtgaaaatgttgaatgtgacagcacccacacctcagcagttacaggccttcaaaaatgaagtaggagtactcaggaaaacgcgacatgtgaatatcctcctcttcatgggttattcaacaaagccacaactggctattgttacccagtggtgtgagggctccagtttatatcatcatctccacatcattgagaccaaattcgagatgatcaaacttatagatattgcacggcagactgcacagggcatggattacttacacgccaagtcaatcatccacagagacctcaagagtaataatatttttcttcatgaagacctcacagtaaaaataggtgattttggtctagccacagtgaaatctcgatggagtgggtcccatcagtttgaacagttgtctggatccattttgtggatggcaccagaagtaatcagaatgcaagataaaaacccatatagctttcagtcagatgtatatgcatttgggattgttctgtatgaattgatgaccggacagttaccttattcaaatatcaacaacagggaccagtctgtgcaaggaaaagagacaaagccacggatcagaagcacatggccataactgaagattttgtgaactctcacaaggaaaaaatttgctctttgaacaataagaaggaactcactaaaatgtaactgagaactgttcaacaggttgaaagctgaaagatgccattggaactgacaaaatgtttcttaaacataaatgatgaaacagtgaaactacataatatctcctctggctgaaacattcaagaagtttaaaatgcttaagttaaaaataaaatcctagtaaacaatggacttactgtgcaacatagagaatatcttacgataacctgtaatggaaaagaatctgaaaaagaatgtatataactgaatcactttgctgtaaactagaatctgacacaacactgtaaatcactacacttttctgttgcatgccaaagattatttaataacgtcattaaaaaattattttaataatta

SEQ ID NO: 122 - protein, 679 aa, Bos taurus
MAALSGGGGGGGGGAEQGQALFNGDMEPEAGAAASSAADPAIPEEVWNIKQMIKLTQEHIEALLDKFGGEHNPPSIYLEAYEEYTSKLDALQQREQQLLESLGNGTDFSVSSSASTDTVTSSSSSSLSVLPSSLSVFQNPTDVSRSNPKSPQKPIVRVFLPNKQRTVVPARCGVTVRDSLKKALMMRGLIPECCAVYRIQDGEKKPIGWDTDISWLTGEELHVEVLENVPLTTHNFVRKTFFTLAFCDFCRKLLFQGFRCQTCGYKFHQRCSTEVPLMCVNYDQLDLLFVSKFFEHHPIPQEEASLAETTLPCGSSPSAPPSDSIGPPILTSPSPSKSIPIPQPFRPADEDHRNQFGQRDRSSSAPNVHINTIEPVNIDDLIRDQGFRSDGGSTTGLSATPPASLPGSLSNVKALQKSPGPQRERKSSSSSEDRNRMKTLGRRDSSDDWEIPDGQITVGQRIGSGSFGTVYKGKWHGDVAVKMLNVTAPTPQQLQAFKNEVGVLRKTRHVNILLFMGYSTKPQLAIVTQWCEGSSLYHHLHIIETKFEMIKLIDIARQTAQGMDYLHAKSIIHRDLKSNNIFLHEDLTVKIGDFGLATVKSRWSGSHQFEQLSGSILWMAPEVIRMQDKNPYSFQSDVYAFGIVLYELMTGQLPYSNINNRDQSVQGKETKPRIRSTWP

SEQ ID NO: 123 - DNA, 7434 bp, Bos taurus
acaccgttacatcttcttcctcttctagcctttcagtgctgccttcatctctttcagtttttcaaaatcccacagatgtgtcacggagcaaccccaagtcaccacaaaaacctatcgttagagtcttcctgcccaataaacagaggacagtggtacctgcacggtgtggagtcacagtccgggacagcctgaagaaggcactgatgatgagaggtctaatcccagagtgctgtgctgtttacagaattcaggatggggagaagaaaccaattggctgggacactgatatttcctggcttactggagaggagttgcatgtagaagtgttggagaatgttccacttacaacacacaactttgtacggaaaacttttttcaccttagcattttgtgacttctgtagaaagctgcttttccagggattccgctgtcaaacatgtggttataaatttcaccagcgttgtagtacagaggttccactgatgtgtgttaattatgaccaactagatttgctgtttgtctccaagttctttgaacaccacccaataccacaggaggaggcctccttagcagagactacccttccatgtggctcatccccttctgcacccccctccgattctattgggcccccaattctcaccagtccatctccttcaaaatccattccaattccacagcctttccgaccagcagatgaagatcatcgaaatcagtttggacaacgagaccggtcctcatcagctccaaatgtgcatataaacacaatagaacccgtcaatattgatgacttgattagagaccaagggtttcgtagtgatggaggatcaaccacaggtttatccgccacaccccctgcctcattacctggctcactctctaatgtgaaagcattgcagaaatctccaggacctcagcgagaaagaaagtcctcttcatcctcagaagacaggaatcgaatgaaaacgcttggtagacgggattcaagtgacgattgggagattcctgatggacagatcacagtgggacaaagaattggatcagggtcatttgggacagtctacaagggaaagtggcatggtgatgtggcagtgaaaatgttgaatgtgacagcacccacacctcagcagttacaggccttcaaaaatgaagtaggagtactcaggaaaacgcgacatgtgaatatcctcctcttcatgggttattcaacaaagccacaactggctattgttacccagtggtgtgagggctccagtttatatcatcatctccacatcattgagaccaaattcgagatgatcaaacttatagatattgcacggcagactgcacagggcatggattacttacacgccaagtcaatcatccacagagacctcaagagtaataatatttttcttcatgaagacctcacagtaaaaataggtgattttggtctagccacagtgaaatctcgatggagtgggtcccatcagtttgaacagttgtctggatccattttgtggatggcaccagaagtaatcagaatgcaagataaaaacccatatagctttcagtcagatgtatatgcatttgggattgttctgtatgaattgatgaccggacagttaccttattcaaatatcaacaacagggaccagataatttttatggtgggacgaggatatctgtctccagatctcagtaaggtacggagtaactgtccaaaagccatgaagagattaatggcagagtgcctaaaaaagaaaagagatgaaagaccactctttccccaagtaggaaagactctcctaagcaagagacaaaattcagaagttatcagggaaaaagataagcagattctcgcctctattgagctgctggcccgctcattgccaaaaattcaccgcagtgcatcagaaccctccttgaatcgggctggcttccaaacagaggattttagtctatatgcttgtgcttctccaaaaacacccattcaggcagggggatatggagaatttgcagccttcaagtagccacaccatcatgacagcatctactcttatttcttaagtcttgtgttcgtacaatttgttaacatcaaaacacagttctgttcctcaactctttttaaagttaaaatttttcagtgcataagctggtgtggaacagaaggaaatttcccatccaacaaaagagggaagaatgttttaggaaccagaattctctgctgccagtgtttcttcttcaacacaaatatcacaagtctgcccactcccaggaagaaagaggagagaccctgagttctgaccttttgatggtcaggcatgatggaaagaaactgctgctacagcttgggagatttgctctgggaagtctgccagtcaactttgcccttctaaccaccagatcaatatgtggctgatcatctgatggggcagttgcaatcaccaagccttgttctctttcctgttctgggattgtgttgtggaacccttttccctagccaccaccagttcatttctgagggatggaacaaaaatgcagcatgcccttcctgtgtggtgcatgttcagtccttgacaaatttttaccaaaatgaagctactttatttaaaaggagggtgagaggtgaggaggtcactttgggtgtggcggaaagggaatgctgcatctttttcctgggctgctggggctctggccttggcttgccagccggaagcgctggcacgcatcgccttcttttcccattgggtccagcaatgaagacgagtgtttggggttttttttttctccaccatgtagcaagttctcaggaaaatacaattgatatcttcctcctaagctcttccaatcagtcaccaagtacttatgtggttactttgtccagggcacaaaatgcctgtatctaattaaaagcctacaaaactgcttgataacagttttgaatgtgagacatttatgtaatttaaatgtaaggtacaagttttaatttctgagtttcttctattatatttttattaaaaaaagaaaataattttcagattgaattggagtaaaataatattacttcccactagaattatatatcctggaaaattgtatttttgttacataagcagcttttaaagaaagatcattacccttttctctacataaatatatggggagtcttagcctaatgacaaatatttataatttttaaattaatggtacttgctggatccatactaacatctttactaatacctcattgtttcttccaacttactcctacactacatcctacatcttcttcctagtcttttatctagaatatgcaacctcaaataaaaatggtggtgtcctcattcattctcctccttccttttttcccaagcctgatcttcaaaaggttggttaatttggcagctgagttcctccccaggcagagaatagaccaattttaggtgtattgggactgagggaggatgtgtaaagattaacatcagtaaagaaccgctgtggagtaattaagaactttgttctttataactggagaatataacctaaccctaacatccctcagcctttactaaagtgtggcgtaaatcacagtagtagcaaagaaagtgactctggatgtgttcctggccagtacctcccttatcatgaatgtagactctctcatcaagatttaggaatataaatcaaatcaaatgtgcccagccaagctatgtagtaagggacttgaacaatattaggcagaacctataaaataaatcagggaattagaaattatttaaagttttcaaattgtaaattgccccggtgtctttcagcctactgccattatttttgctacaatacctacatttcagaggagggcctactgaaaattccatgcaagtggaaaataatcctcaagttattaatgagtttgaaaagcaatgagttcttaagtctttgtgagtagagcaagatcctacaaaattcagaaatagtaaaaatggattcatgctgatttgaagagcatctgtgtgcataatataatgctgcatctcttttaaaagcagtctatttttctttttaaatttgtccccatagatgcttttgaacatgaacatgcttatgttaccttttccgaggttgggaagagccaggagctctcaggcagggccccctccctcagctgggcaggagctgctcaggaggagctagttatagaggaagcttagcgttggcattttcaaaattcaaggtgataacgctttcttcttcctttctgttttagaatagattgctgtctgatttgaaaaagggaaatagatttgatctcaaatgaatctgtgcccagaagccaggctcagggtattcagagatttgtatagtgccctcaaaaaataacaaaattttagctttccttttttcttcttttctccatcaaattcttttttctctagtttacaaatgacatggaaaaggaatttcccctgagttttgtatgcctttttttttttggcttagactatagataggcgtgttgagctcctaagaaaatacaaggaggaactctttgttgtgcagagcactttatgagtagtttgtgtggataatatgtgactgcttccctgacgagcttgtgaggctgtacttatgtctttcctgtaaggcagcttcagtgccttctgtagtgtatataaggaaagattacgccttctgaaaaatctcagagcaaccataagattattttaaaatatgtagtatgactgatggactttttcatcattaaattagtctagcatctaaacttttaccactgaaataatattgaccaaaaagcaatttataaaaggtatttgtgaatagaaaatacaatgtgatcatttgtacttatgtgcaccttaaaagaggaattctgtctagctgtcaaattctggttccttaacatccagtccttgattgtgattgagatctggtaggacgtgctggggcacgctagcagataaaatcccgtatactttaggatagatgttacatttatgtcagtgttggcaaagagcattgtgtagtaataaagaattcaagacttcagcaatgtcaacctgaaactttgtaaatatttcctagattgttatttgatgcagtcacagctctttatcacacaatgttgtctttccctcatcaggcaattttagaactgctgcacacccctcctcagatctcacctgcccctcctgtacattcacctctccagccttgtgcacacctcatttagctttagtttgaaacacattgcagggttcaggtgacctcttcaaaaactacctcctcagaatgaggtaatgaatagttatttattttaaaatatgaaaagtcaggagctctagaatatgaagatgatctaagattttaacttttatgtatacttgttgagcactctccttttgtcctaaagggcattatacatttaagcagtaatactgaaaaatgtagctcagagtaactgaatgttgttgaaagtggtgccagaatctgttttaggggtacgtatcagaatcttaatcttaaatcggttacatgaaattaaatagttaatggtaacacttgactaacagatataattttaattttcggtaggcttttagcaagacagtaagtacatcttcataatgagttagccacagcttcatcacatgcacagattttcctgttgagagactgcccagttaagagggtagaatgatgaaccatttttcaggattctcttctttgtccaaactggcattgtgagtgctagaatatcagcactttcaaactagtgattccaactattaggctattaaaaagcaaaacaaaccaaacaaaccatagccagacatgggaagtttactatgagtataaacagcaaatagcttacaggtcatacattgaaatggtgtaggtaaggcgttagaaaaataccttgacaatttgccaaatgatcttactgtgccttcatgatgcaataaaaaaaaaaaaaatttagcataaatcagtgatttgtgaagagagcagccaccctggtctaactcagctgtgttaatattttttagcgtgcaatttagactgcaaagataaatgcactaaagagtttatagccaaaatcacatttaaaaaatgagagaaaacacaggtaaattttcagtgaacaaaattatttttttaaagtacataatccctagtatagtcagatatatttatcacatagagcaaataggttgaaatcacaattcagtgacatttctagagaaactttttctactcccataggttcttcaaagcatggaacttttatataacagaaatgtgtgacggtcattttaaattgctgtagtttggggctgaagtactgtgtgctgggcagcaatcacatgtattaactagtgagaaaggagaaattaagatataggacagaatttgattttcttgttcccagattactgctgccaacctagacactgagtttccagaggctgaaacgtaaacttgcagctcagcaactgttttgcaaagttagtgggactgtcctgcttatgctgttcaaaaatgctctgagggccaggtggggcctccaggggctcctctctgaggggacatcagactagctaacgacctggcgggcggatgtgaaccggacacactccatggtgtgcttcttgtatcggtccctcgccaccctcaagaaaggcttcagcgggttctctagacgtctccactaaggtgtgttactaacagccatgggttgttgagcacccgaggagtgcaatagcatctctgcatgattgtatattggcccgaagagaatgaagtggccagtgtactcatgttccatgttgctagctctggtaaactgaaaatactggtaagatttttgttttatcagtacactagagagtaagctttgttttgttgtttttagataatgttttcacttccatttggaaagacatttaaattgagtttcagtcctaaattttgccagtcatggtaattagcagtttctatcaggtatttttaaggtagaagaggatagaaacataagttctaaaagcttaaggtaaccgtggtttattttaaaatgtttaggggtggttagtctctacctcaaaaaaagtgagtgaatcttttatttcagcattcacaagttcggctgttgtttttgtaatacattttttttttaaccttttgacccccctttacctaagtgtcaatgtagttttattaattactaagtcagtttcattaaaatgtttatttagcagttttgactaattgcaatgattaatatagccagttgtgcatgaggacacagccagtgagtatatctgggttttttttgtgatgctttttttcttaagacttctgtagatttatgaagtactcattgaaaacaactaaaatacgtttattcgtgttaatatggaaaaaaaaaaa

SEQ ID NO: 124 - protein, 603 aa, Bos taurus
MMRGLIPECCAVYRIQDGEKKPIGWDTDISWLTGEELHVEVLENVPLTTHNFVRKTFFTLAFCDFCRKLLFQGFRCQTCGYKFHQRCSTEVPLMCVNYDQLDLLFVSKFFEHHPIPQEEASLAETTLPCGSSPSAPPSDSIGPPILTSPSPSKSIPIPQPFRPADEDHRNQFGQRDRSSSAPNVHINTIEPVNIDDLIRDQGFRSDGGSTTGLSATPPASLPGSLSNVKALQKSPGPQRERKSSSSSEDRNRMKTLGRRDSSDDWEIPDGQITVGQRIGSGSFGTVYKGKWHGDVAVKMLNVTAPTPQQLQAFKNEVGVLRKTRHVNILLFMGYSTKPQLAIVTQWCEGSSLYHHLHIIETKFEMIKLIDIARQTAQGMDYLHAKSIIHRDLKSNNIFLHEDLTVKIGDFGLATVKSRWSGSHQFEQLSGSILWMAPEVIRMQDKNPYSFQSDVYAFGIVLYELMTGQLPYSNINNRDQIIFMVGRGYLSPDLSKVRSNCPKAMKRLMAECLKKKRDERPLFPQVGKTLLSKRQNSEVIREKDKQILASIELLARSLPKIHRSASEPSLNRAGFQTEDFSLYACASPKTPIQAGGYGEFAAFK

SEQ ID NO: 125 - DNA, 2295 bp, Equus caballus
  misc_feature (79)..(79): n is a, c, g, or t
atgaagacgctgagcggcggcggcggcggcgcggagcagggccaggctctgttcaacggggacatggaacccggaggcnccgcgccggcgcccgcggcctcgtcggccgcggaccctgccattcccgaggaggtatggaatatcaaacaaatgattaaattgacacaggaacatatagaggccctattggacaaatttggtggggagcataatccaccatcaatatatctggaggcctatgaagaatacaccagcaagctagatgccctccaacaaagagaacaacagttattggaatccctggggaatggaactgatttttctgtttctagttctgcatcaacggacaccgttacatcttcttcctcttctagcctttcagtgctaccttcatctctttcagtttttcaaaatcccacagatgtgtcacggagcaaccctaagtcaccacaaaaacctatcgttagagtcttcctgcccaacaaacagaggacagtggtacctgcaaggtgtggcgttacagtccgggacagtctaaagaaagcactgatgatgagaggtctaatcccagagtgctgtgctgtttacagaattcaggatggagagaagaaaccaattggctgggacactgatatttcctggctcactggagaggaattgcatgtagaagtgttggagaatgttccacttacaacacacaactttgtacggaaaacttttttcaccttagcattttgtgacttttgtcgaaagctgcttttccagggtttccgctgtcaaacatgtggttataaatttcaccagcgttgtagtacagaggttccactgatgtgtgttaattatgaccaacttgatttgctgtttgtctccaagttctttgaacaccacccagtatcacaggaggaggcctccttagcagagactgcccttacatctggatcatccccttctgcacccccctccgattccattgggccccaaattctcaccagtccatctccttcaaaatccattccaattccacagcctttccgaccagcagatgaagatcatcgaaatcagtttggacaacgagaccggtcctcatcagctccaaatgtacatataaacacaatagaacctgtcaatattgatgacttgattagagaccaagggtttcgtagtgatggaggatcaaccacaggtttatctgccaccccccctgcctcattacctggctcactcactaatgtgaaggcattacagaaatctccaggacctcaacgggaaaggaaatcatcttcatcctcagaagacaggaatcgaatgaaaactcttggtagacgggattcaagtgacgattgggagattcctgatgggcagatcacagtgggacaaagaattggatctgggtcatttgggacagtctacaagggaaagtggcatggtgatgtggcagtgaaaatgttgaatgtgacagcacccacacctcagcagttacaggccttcaaaaatgaagtaggagtactcaggaaaactcgacatgtgaatatcctactcttcatgggctattcaacaaagccacaactggctattgttacccagtggtgtgagggctccagcttatatcaccatctccacatcattgagaccaaatttgagatgatcaaacttatagatattgctcggcaaactgcacagggcatggattacttacacgccaagtcaatcatccacagagacctcaagagtaataatatttttcttcatgaagacctcacagtaaaaataggtgattttggtctagccacagtgaaatctcgatggagtgggtcccatcagtttgaacagttgtctggatccattttgtggatggcaccagaagtaatcagaatgcaagataaaaacccgtatagctttcaatcagatgtatatgcctttgggattgttctgtatgaattgatgactggacagttaccttattcaaacatcaacaacagggaccagataatttttatggtgggaagaggatatctatctccagatctcagtaaggtacggagtaactgtccaaaagccatgaagagattaatggcagagtgcctaaaaaagaaaagagacgagagaccactcttcccccaaattctcgcctctattgagctgctggcccgctcattgccaaaaattcaccgcagtgcatcagagccctccttgaatcgggctggcttccagacagaggattttagtctatatgcttgtgcttctccgaaaacacccatccaggcagggggatatggtgcgtttcctgtccactga

SEQ ID NO: 126 - protein, 764 aa, Equus caballus
  misc_feature (27)..(27): Xaa can be any naturally occurring amino acid
MKTLSGGGGGAEQGQALFNGDMEPGGXAPAPAASSAADPAIPEEVWNIKQMIKLTQEHIEALLDKFGGEHNPPSIYLEAYEEYTSKLDALQQREQQLLESLGNGTDFSVSSSASTDTVTSSSSSSLSVLPSSLSVFQNPTDVSRSNPKSPQKPIVRVFLPNKQRTVVPARCGVTVRDSLKKALMMRGLIPECCAVYRIQDGEKKPIGWDTDISWLTGEELHVEVLENVPLTTHNFVRKTFFTLAFCDFCRKLLFQGFRCQTCGYKFHQRCSTEVPLMCVNYDQLDLLFVSKFFEHHPVSQEEASLAETALTSGSSPSAPPSDSIGPQILTSPSPSKSIPIPQPFRPADEDHRNQFGQRDRSSSAPNVHINTIEPVNIDDLIRDQGFRSDGGSTTGLSATPPASLPGSLTNVKALQKSPGPQRERKSSSSSEDRNRMKTLGRRDSSDDWEIPDGQITVGQRIGSGSFGTVYKGKWHGDVAVKMLNVTAPTPQQLQAFKNEVGVLRKTRHVNILLFMGYSTKPQLAIVTQWCEGSSLYHHLHIIETKFEMIKLIDIARQTAQGMDYLHAKSIIHRDLKSNNIFLHEDLTVKIGDFGLATVKSRWSGSHQFEQLSGSILWMAPEVIRMQDKNPYSFQSDVYAFGIVLYELMTGQLPYSNINNRDQIIFMVGRGYLSPDLSKVRSNCPKAMKRLMAECLKKKRDERPLFPQILASIELLARSLPKIHRSASEPSLNRAGFQTEDFSLYACASPKTPIQAGGYGAFPVH

SEQ ID NO: 127 - DNA, 2678 bp, Gallus gallus
tccccctccctcgccccagcgcttcgatccaagatggcggcgctgagcagcggcagcagcgccgagggggcctcgctcttcaacggggacatggagcccgagccgccgccgcccgtgctgggcgcctgctacgccgggagcggcggcggcgacccggccatcccggaggaggtgtggaatatcaaacagatgattaaattaacacaagaacatatagaagcgctgttagacaagtttggaggagagcataacccaccatcaatatatttagaggcctatgaggagtacaccagcaaactagatgctctacagcagagagaacagcagttattggaatccatgggaaatggaactgatttctctgtttccagttcagcttcaacggacacagttgcatcatcttcctcctctagcctctctgtagcaccttcatccctttcagtttatcaaaatcctactgatatgtcgcggaataaccctaagtctccacagaagcctattgttagagtcttcctgcccaacaagcaaaggactgtggttccggcaagatgtggggtgacagtccgagacagcctgaagaaagctctgatgatgagaggtcttattccagaatgctgtgctgtttacagaatacaggatggagagaagaagccaattggctgggacactgacatttcctggctaaccggagaggagttacacgtggaggtcttggagaatgtgccactcacaacacacaattttgtacgaaaaacattcttcacgttagcgttctgcgacttctgtcgaaagctgcttttccagggattccgatgccagacatgtggctacaaatttcaccagcgctgtagcacagaagtgccactgatgtgtgttaactacgaccaactcgatttgctgtttgtctccaagttctttgaacatcaccccatatcgcaggaggagaccaccttaggagagaccaccccggcatcgggatcgtacccctcagtgcccccatcagattctgttggaccaccaattctccctagtccttctccttcaaaatccattccaatcccacagcccttccgaccagcagatgaagaccatcggaatcagtttgggcaacgcgaccgatcctcttcagctcccaatgttcacatcaatacaattgagccagtcaatattgatgacttgattagagaccagggtgtacgaggagagggagcccctttgaaccagctgatgcgctgtcttcggaaataccaatcccggactcccagtcccctccttcattctgtccccagtgaaatagtgtttgattttgagcctggcccagtgttcagaggttcaactgcaggtttgtctgcaacacctcctgcatctttgcctgggtcacttaccaatgtgaaagcattacagaaatcaccaggcccccaacgggaaaggaaatcatcctcatcctcagaagacagaaataggatgaaaacccttggtcgacgagattcaagtgatgattgggaaataccagatgggcagatcacagttggacaaaggataggatctggatcatttggaacagtctacaaaggaaagtggcatggtgacgtggcagtgaaaatgttgaatgttacagcacccacacctcaacagttacaggctttcaaaaatgaagtaggagtgctcaggaaaacacggcatgtgaatatcctactttttatgggttattcaacaaaacctcagttggctattgttacacagtggtgtgaggggtccagcttatatcaccatctgcacataattgagaccaagtttgaaatgatcaaactaattgatattgcacgacagactgcacaaggcatggattatttgcatgccaagtcaatcatccacagagacctcaagagtaataatatttttcttcatgaagacctcacagtaaaaataggtgacttcggtctggctacagtgaaatcacgatggagtggatctcatcaatttgaacagttatctggatcaattctatggatggcaccggaagtgatcaggatgcaagacaaaaacccatatagctttcagtcagatgtgtatgcattcgggattgtgctttatgaactgatgactggacagttaccatactcaaacatcaacaacagggaccagataatttttatggtgggacgaggatatctatctccagacctcagtaaagtaagaagtaactgtccaaaagctatgaagagactaatggcagaatgcttgaaaaagaaaagagatgagagacctctttttccacagattcttgcctccattgagcttctggcccggtcgttgccaaaaattcaccgcagtgcatctgagccgtcactaaaccgggctggcttccagaccgaggatttcagtctgtatgcttgtgcttctccaaaaacgcccatccaagcagggggatacggtgggtttccagtacactgaaaagaaatgtgaaagcgtgtgcctgtttgctcatgtgctggtgtgttcctgtgtgtgcaacgcatacgtacgttctcagttcctaccagcgactttttaaggtttactgagggaatgaagactcatttcctaacatggggcattgaacgtcctgagcacaagtcagtgctggtaaggaatgtcttgggaacagctggcaagaagaattagaaggtacttaaagg

SEQ ID NO: 128 - protein, 806 aa, Gallus gallus
MAALSSGSSAEGASLFNGDMEPEPPPPVLGACYAGSGGGDPAIPEEVWNIKQMIKLTQEHIEALLDKFGGEHNPPSIYLEAYEEYTSKLDALQQREQQLLESMGNGTDFSVSSSASTDTVASSSSSSLSVAPSSLSVYQNPTDMSRNNPKSPQKPIVRVFLPNKQRTVVPARCGVTVRDSLKKALMMRGLIPECCAVYRIQDGEKKPIGWDTDISWLTGEELHVEVLENVPLTTHNFVRKTFFTLAFCDFCRKLLFQGFRCQTCGYKFHQRCSTEVPLMCVNYDQLDLLFVSKFFEHHPISQEETTLGETTPASGSYPSVPPSDSVGPPILPSPSPSKSIPIPQPFRPADEDHRNQFGQRDRSSSAPNVHINTIEPVNIDDLIRDQGVRGEGAPLNQLMRCLRKYQSRTPSPLLHSVPSEIVFDFEPGPVFRGSTAGLSATPPASLPGSLTNVKALQKSPGPQRERKSSSSSEDRNRMKTLGRRDSSDDWEIPDGQITVGQRIGSGSFGTVYKGKWHGDVAVKMLNVTAPTPQQLQAFKNEVGVLRKTRHVNILLFMGYSTKPQLAIVTQWCEGSSLYHHLHIIETKFEMIKLIDIARQTAQGMDYLHAKSIIHRDLKSNNIFLHEDLTVKIGDFGLATVKSRWSGSHQFEQLSGSILWMAPEVIRMQDKNPYSFQSDVYAFGIVLYELMTGQLPYSNINNRDQIIFMVGRGYLSPDLSKVRSNCPKAMKRLMAECLKKKRDERPLFPQILASIELLARSLPKIHRSASEPSLNRAGFQTEDFSLYACASPKTPIQAGGYGGFPVH